European Patent Application EP 4 148 127 A1, published March 15, 2023. Title: COMPOSITIONS AND METHODS FOR RAPID AND DYNAMIC FLUX CONTROL USING SYNTHETIC METABOLIC VALVES. Applicant: Duke University. The sequence listing filed with the application follows.

SEQUENCE LISTING (54 sequences)

SEQ ID NO: 1 - DNA, 3111 bp, Artificial Sequence
  Plasmid pSMART-HC-Kan-yibD-THNS
gtgcgtaattgtgctgatctcttatatagctgctctcattatctctctaccctgaagtgactctctcacctgtaaaaataatatctcacaggcttaatagtttcttaatacaaagcctgtaaaacgtcaggataacttctgtgtaggaggataatctatggcaactctctgccgtccgtccgtgagtgtgccggagcatgttatcacgatggaagaaacccttgaactggcccgtcgtcgtcatacggatcatccacagctgcccctggcgctgcgcttaattgaaaacaccggtgttcgcacgcgtcatattgttcaaccgatcgaggataccctggagcatccagggtttgaagatcgcaataaagtatacgagcgcgaggccaaatcgcgtgtgccggcggtaatccaacgcgccctggacgacgcggagcttctggcgacggacattgacgttattatctatgtctcatgcacgggttttatgatgcctagtcttactgcttggttaatcaacgaaatgggcttcgacagcacgacccgccaaattcctatcgcacagcttggctgtgcggccggtggtgccgcgattaaccgcgctcacgatttttgcacggcatatcctgaagcaaatgcgctgatcgttgcctgcgaattctgcagcctgtgttatcagcccacagatctcggtgtaggttctctcctgtgcaacggtctgttcggtgatggaattgctgcggctgtggtgcgcggacgtggtggtacgggggttcgcttggagcgtaacggcagctacttaattccaaaaaccgaagattggatcatgtatgatgtgaaagcaaccggtttccacttcttactggataagcgcgtcccggccaccatggaacccttggcgccggctctgaaagaactcgcgggcgagcatggttgggacgccagtgatctggatttttatattgttcacgccggtggtccgcgtattttagacgacttgagtactttccttgaggtggatccgcatgcgtttcgtttttcccgtgctaccctgaccgagtatggtaacattgcgtcagcagtcgtgctggatgcgttacgccgcttgttcgatgaaggcggtgtggaggaaggtgcgcgcggtctgctggcggggttcgggccaggtattacagccgaaatgtcactgggctgctggcaaaccgcgtagtaaccggcttatcggtcagtttcacctgatttacgtaaaaacccgcttcggcgggtttttgcttttggaggggcagaaagatgaatgactgtccacgacgctatacccaaaagaaagacgaattctctagatatcgctcaatactgaccatttaaatcatacctgacctccatagcagaaagtcaaaagcctccgaccggaggcttttgacttgatcggcacgtaagaggttccaactttcaccataatgaaataagatcactaccgggcgtattttttgagttatcgagattttcaggagctaaggaagctaaaatgagccatattcaacgggaaacgtcttgctcgaggccgcgattaaattccaacatggatgctgatttatatgggtataaatgggctcgcgataatgtcgggcaatcaggtgcgacaatctatcgattgtatgggaagcccgatgcgccagagttgtttctgaaacatggcaaaggtagcgttgccaatgatgttacagatgagatggtcaggctaaactggctgacggaatttatgcctcttccgaccatcaagcattttatccgtactcctgatgatgcatggttactcaccactgcgatcccagggaaaacagcattccaggtattagaagaatatcctgattcaggtgaaaatattgttgatgcgctggcagtgttcctgcgccggttgcattcgattcctgtttgtaattgtccttttaacggcgatcgcgtatttcgtctcgctcaggcgcaatcacgaatgaataacggtttggttggtgcgagtgattttgatgacgagcgtaatggctggcctgttgaacaagtctggaaagaaatgcataagcttttgccattctcaccggattcagtcgtcactcatggtgatttctcacttgataaccttatttttgacgaggggaaattaataggttgtattgatgttggacgagtcggaatcgcagaccgataccaggatcttgccatcctatggaactgcctcggtgagttttctccttcattacagaaacggctttttcaaaaatatggtattgataatcctgatatgaataaattgcagtttcacttgatgctcgatgagtttttctaatgagggcccaaatgtaatcacctggctcaccttcgggtgggcctttctgcgttgctggcgtttttccataggctccgcccccctgacgagcatcacaaaaatcgatgctcaagtcagaggtggcgaaacccgacaggactataaagataccaggcgtttccccctggaagctccctcgtgcgctctcctgttccgaccctgccgcttaccggatacctgtccgcctttctcccttcgggaagcgtggcgctttctcatagctcacgctgtaggtatctcagttcggtgtaggtcgttcgctccaagctgggctgtgtgcacgaaccccccgttcagcccgaccgctgcgccttatccggtaactatcgtcttgagtccaacccggtaagacacgacttatcgccactggcagcagccactggtaacaggattagcagagcgaggtatgtaggcggtgctacagagttcttgaagtggtggcctaactacggctacactagaagaacagtatttggtatctgcgctctgctgaagccagttacctcggaaaaagagttggtagctcttgatccggcaaacaaaccaccgctggtagcggtggtttttttgtttgcaagcagcagattacgcgcagaaaaaaaggatctcaagaagatcctttgattttctaccgaagaaaggcccacccgtgaaggtgagccagtgagttgattgcagtccagttacgctggagtctgaggctcgtcctgaatgatatcaagcttgaattcgtt

SEQ ID NO: 2 - DNA, 2386 bp, Artificial Sequence
  Plasmid pCDF-T2-fabIsgRNA
gcactgaaatctagagcggttcagtagaaaagatcaaaggatcttcttgagatcctttttttctgcgcgtaatcttttgccctgtaaacgaaaaaaccacctggggaggtggtttgatcgaaggttaagtcagttggggaactgcttaaccgtggtaactggctttcgcagagcacagcaaccaaatctgtccttccagtgtagccggactttggcgcacacttcaagagcaaccgcgtgtttagctaaacaaatcctctgcgaactcccagttaccaatggctgctgccagtggcgttttaccgtgcttttccgggttggactcaagtgaacagttaccggataaggcgcagcagtcgggctgaacggggagttcttgcttacagcccagcttggagcgaacgacctacaccgagccgagataccagtgtgtgagctatgagaaagcgccacacttcccgtaagggagaaaggcggaacaggtatccggtaaacggcagggtcggaacaggagagcgcaagagggagcgacccgccggaaacggtggggatctttaagtcctgtcgggtttcgcccgtactgtcagattcatggttgagcctcacggctcccacagatgcaccggaaaagcgtctgtttatgtgaactctggcaggagggcggagcctatggaaaaacgccaccggcgcggccctgctgttttgcctcacatgttagtcccctgcttatccacggaatctgtgggtaactttgtatgtgtccgcagcgcccgccgcagtctcacgcccggagcgtagcgaccgagtgagctagctatttgtttatttttctaaatacattcaaatatgtatccgctcatgagacaataaccctgataaatgcttcaataatattgaaaaaggaagagtatgagggaagcggtgatcgccgaagtatcgactcaactatcagaggtagttggcgtcatcgagcgccatctcgaaccgacgttgctggccgtacatttgtacggctccgcagtggatggcggcctgaagccacacagtgatattgatttgctggttacggtgaccgtaaggcttgatgaaacaacgcggcgagctttgatcaacgaccttttggaaacttcggcttcccctggagagagcgagattctccgcgctgtagaagtcaccattgttgtgcacgacgacatcattccgtggcgttatccagctaagcgcgaactgcaatttggagaatggcagcgcaatgacattcttgcaggtatcttcgagccagccacgatcgacattgatctggctatcttgctgacaaaagcaagagaacatagcgttgccttggtaggtccagcggcggaggaactctttgatccggttcctgaacaggatctatttgaggcgctaaatgaaaccttaacgctatggaactcgccgcccgactgggctggcgatgagcgaaatgtagtgcttacgttgtcccgcatttggtacagcgcagtaaccggcaaaatcgcgccgaaggatgtcgctgccgactgggcaatggagcgcctgccggcccagtatcagcccgtcatacttgaagctagacaggcttatcttggacaagaagaagatcgcttggcctcgcgcgcagatcagttggaagaatttgtccactacgtgaaaggcgagatcaccaaggtagtcggcaaataatgtctaacaattcgttcaacactatagggcgaattgaaggaaggccgtcaaggccgcattgaggctcgtcctgaatgatatcaagcttgaattcgttgaattctaaagatctttgacagctagctcagtcctaggtataatactagtcagcctgctccggtcggaccgttttagagctagaaatagcaagttaaaataaggctagtccgttatcaacttgaaaaagtggcaccgagtcggtgctttttttgaagcttgggcccgaacaaaaactcatctcagaagaggatctgaatagcgccgtcgaccatcatcatcatcatcattgagtttaaacggtctccagcttggctgttttggcggatgagagaagattttcagcctgatacagattaaatcagaacgcagaagcggtctgataaaacagaatttgcctggcggcagtagcgcggtggtcccacctgaccccatgccgaactcagaagtgaaacgccgtagcgccgatggtagtgtggggtctccccatgcgagagtagggaactgccaggcatcaaataaaacgaaaggctcagtcgaaagactgggcctttcgttttatctgttgtttgtcggtgaactggatccttactcgagtctagactgcagctgggcctcatgggccttcctttcactgcccgctttccag

SEQ ID NO: 3 - DNA, 7413 bp, Artificial Sequence
  Plasmid pdCas9-ptet-sspB
gacgtcttaagacccactttcacatttaagttgtttttctaatccgcatatgatcaattcaaggccgaataagaaggctggctctgcaccttggtgatcaaataattcgatagcttgtcgtaataatggcggcatactatcagtagtaggtgtttccctttcttctttagcgacttgatgctcttgatcttccaatacgcaacctaaagtaaaatgccccacagcgctgagtgcatataatgcattctctagtgaaaaaccttgttggcataaaaaggctaattgattttcgagagtttcatactgtttttctgtaggccgtgtacctaaatgtacttttgctccatcgcgatgacttagtaaagcacatctaaaacttttagcgttattacgtaaaaaatcttgccagctttccccttctaaagggcaaaagtgagtatggtgcctatctaacatctcaatggctaaggcgtcgagcaaagcccgcttattttttacatgccaatacaatgtaggctgctctacacctagcttctgggcgagtttacgggttgttaaaccttcgattccgacctcattaagcagctctaatgcgctgttaatcactttacttttatctaatctagacatcattaattcctaatttttgttgacactctatcgttgatagagttattttaccactccctatcagtgatagagaaaagaattcaaaagatctaaagaggagaaaggatctatggataagaaatactcaataggcttagctatcggcacaaatagcgtcggatgggcggtgatcactgatgaatataaggttccgtctaaaaagttcaaggttctgggaaatacagaccgccacagtatcaaaaaaaatcttataggggctcttttatttgacagtggagagacagcggaagcgactcgtctcaaacggacagctcgtagaaggtatacacgtcggaagaatcgtatttgttatctacaggagattttttcaaatgagatggcgaaagtagatgatagtttctttcatcgacttgaagagtcttttttggtggaagaagacaagaagcatgaacgtcatcctatttttggaaatatagtagatgaagttgcttatcatgagaaatatccaactatctatcatctgcgaaaaaaattggtagattctactgataaagcggatttgcgcttaatctatttggccttagcgcatatgattaagtttcgtggtcattttttgattgagggagatttaaatcctgataatagtgatgtggacaaactatttatccagttggtacaaacctacaatcaattatttgaagaaaaccctattaacgcaagtggagtagatgctaaagcgattctttctgcacgattgagtaaatcaagacgattagaaaatctcattgctcagctccccggtgagaagaaaaatggcttatttgggaatctcattgctttgtcattgggtttgacccctaattttaaatcaaattttgatttggcagaagatgctaaattacagctttcaaaagatacttacgatgatgatttagataatttattggcgcaaattggagatcaatatgctgatttgtttttggcagctaagaatttatcagatgctattttactttcagatatcctaagagtaaatactgaaataactaaggctcccctatcagcttcaatgattaaacgctacgatgaacatcatcaagacttgactcttttaaaagctttagttcgacaacaacttccagaaaagtataaagaaatcttttttgatcaatcaaaaaacggatatgcaggttatattgatgggggagctagccaagaagaattttataaatttatcaaaccaattttagaaaaaatggatggtactgaggaattattggtgaaactaaatcgtgaagatttgctgcgcaagcaacggacctttgacaacggctctattccccatcaaattcacttgggtgagctgcatgctattttgagaagacaagaagacttttatccatttttaaaagacaatcgtgagaagattgaaaaaatcttgacttttcgaattccttattatgttggtccattggcgcgtggcaatagtcgttttgcatggatgactcggaagtctgaagaaacaattaccccatggaattttgaagaagttgtcgataaaggtgcttcagctcaatcatttattgaacgcatgacaaactttgataaaaatcttccaaatgaaaaagtactaccaaaacatagtttgctttatgagtattttacggtttataacgaattgacaaaggtcaaatatgttactgaaggaatgcgaaaaccagcatttctttcaggtgaacagaagaaagccattgttgatttactcttcaaaacaaatcgaaaagtaaccgttaagcaattaaaagaagattatttcaaaaaaatagaatgttttgatagtgttgaaatttcaggagttgaagatagatttaatgcttcattaggtacctaccatgatttgctaaaaattattaaagataaagattttttggataatgaagaaaatgaagatatcttagaggatattgttttaacattgaccttatttgaagatagggagatgattgaggaaagacttaaaacatatgctcacctctttgatgataaggtgatgaaacagcttaaacgtcgccgttatactggttggggacgtttgtctcgaaaattgattaatggtattagggataagcaatctggcaaaacaatattagattttttgaaatcagatggttttgccaatcgcaattttatgcagctgatccatgatgatagtttgacatttaaagaagacattcaaaaagcacaagtgtctggacaaggcgatagtttacatgaacatattgcaaatttagctggtagccctgctattaaaaaaggtattttacagactgtaaaagttgttgatgaattggtcaaagtaatggggcggcataagccagaaaatatcgttattgaaatggcacgtgaaaatcagacaactcaaaagggccagaaaaattcgcgagagcgtatgaaacgaatcgaagaaggtatcaaagaattaggaagtcagattcttaaagagcatcctgttgaaaatactcaattgcaaaatgaaaagctctatctctattatctccaaaatggaagagacatgtatgtggaccaagaattagatattaatcgtttaagtgattatgatgtcgatgccattgttccacaaagtttccttaaagacgattcaatagacaataaggtcttaacgcgttctgataaaaatcgtggtaaatcggataacgttccaagtgaagaagtagtcaaaaagatgaaaaactattggagacaacttctaaacgccaagttaatcactcaacgtaagtttgataatttaacgaaagctgaacgtggaggtttgagtgaacttgataaagctggttttatcaaacgccaattggttgaaactcgccaaatcactaagcatgtggcacaaattttggatagtcgcatgaatactaaatacgatgaaaatgataaacttattcgagaggttaaagtgattaccttaaaatctaaattagtttctgacttccgaaaagatttccaattctataaagtacgtgagattaacaattaccatcatgcccatgatgcgtatctaaatgccgtcgttggaactgctttgattaagaaatatccaaaacttgaatcggagtttgtctatggtgattataaagtttatgatgttcgtaaaatgattgctaagtctgagcaagaaataggcaaagcaaccgcaaaatatttcttttactctaatatcatgaacttcttcaaaacagaaattacacttgcaaatggagagattcgcaaacgccctctaatcgaaactaatggggaaactggagaaattgtctgggataaagggcgagattttgccacagtgcgcaaagtattgtccatgccccaagtcaatattgtcaagaaaacagaagtacagacaggcggattctccaaggagtcaattttaccaaaaagaaattcggacaagcttattgctcgtaaaaaagactgggatccaaaaaaatatggtggttttgatagtccaacggtagcttattcagtcctagtggttgctaaggtggaaaaagggaaatcgaagaagttaaaatccgttaaagagttactagggatcacaattatggaaagaagttcctttgaaaaaaatccgattgactttttagaagctaaaggatataaggaagttaaaaaagacttaatcattaaactacctaaatatagtctttttgagttagaaaacggtcgtaaacggatgctggctagtgccggagaattacaaaaaggaaatgagctggctctgccaagcaaatatgtgaattttttatatttagctagtcattatgaaaagttgaagggtagtccagaagataacgaacaaaaacaattgtttgtggagcagcataagcattatttagatgagattattgagcaaatcagtgaattttctaagcgtgttattttagcagatgccaatttagataaagttcttagtgcatataacaaacatagagacaaaccaatacgtgaacaagcagaaaatattattcatttatttacgttgacgaatcttggagctcccgctgcttttaaatattttgatacaacaattgatcgtaaacgatatacgtctacaaaagaagttttagatgccactcttatccatcaatccatcactggtctttatgaaacacgcattgatttgagtcagctaggaggtgactaactcgagccggcttatcggtcagtttcacctgatttacgtaaaaacccgcttcggcgggtttttgcttttggaggggcagaaagatgaatgactgtccacgacgctatacccaaaagaaatccctatcagtgatagagattgacatccctatcagtgatagagatactgagcacatcagcaggacgcactgaccaagaggagaaaggatctatggatttgtcacagctaacaccacgtcgtccctatctgctgcgtgcattctatgagtggttgctggataaccagctcacgccgcacctggtggtggatgtgacgctccctggcgtgcaggttcctatggaatatgcgcgtgacgggcaaatcgtactcaacattgcgccgcgtgctgtcggcaatctggaactggcgaatgatgaggtgcgctttaacgcgcgctttggtggcattccgcgtcaggtttctgtgccgctggctgccgtgctggctatctacgcccgtgaaaatggcgcaggcacgatgtttgagcctgaagctgcctacgatgaagataccagcatcatgaatgatgaagaggcatcggcagacaacgaaaccgttatgtcggttattgatggcgacaagccagatcacgatgatgacactcatcctgacgatgaacctccgcagccaccacgcggtggtcgaccggcattacgcgttgtgaagtaactcgagtaaggatctccaggcatcaaataaaacgaaaggctcagtcgaaagactgggcctttcgttttatctgttgtttgtcggtgaacgctctctactagagtcacactggctcaccttcgggtgggcctttctgcgtttatacctagggatatattccgcttcctcgctcactgactcgctacgctcggtcgttcgactgcggcgagcggaaatggcttacgaacggggcggagatttcctggaagatgccaggaagatacttaacagggaagtgagagggccgcggcaaagccgtttttccataggctccgcccccctgacaagcatcacgaaatctgacgctcaaatcagtggtggcgaaacccgacaggactataaagataccaggcgtttccccctggcggctccctcgtgcgctctcctgttcctgcctttcggtttaccggtgtcattccgctgttatggccgcgtttgtctcattccacgcctgacactcagttccgggtaggcagttcgctccaagctggactgtatgcacgaaccccccgttcagtccgaccgctgcgccttatccggtaactatcgtcttgagtccaacccggaaagacatgcaaaagcaccactggcagcagccactggtaattgatttagaggagttagtcttgaagtcatgcgccggttaaggctaaactgaaaggacaagttttggtgactgcgctcctccaagccagttacctcggttcaaagagttggtagctcagagaaccttcgaaaaaccgccctgcaaggcggttttttcgttttcagagcaagagattacgcgcagaccaaaacgatctcaagaagatcatcttattaatcagataaaatatttctagatttcagtgcaatttatctcttcaaatgtagcacctgaagtcagccccatacgatataagttgttactagtgcttggattctcaccaataaaaaacgcccggcggcaaccgagcgttctgaacaaatccagatggagttctgaggtcattactggatctatcaacaggagtccaagcgagctcgatatcaaattacgccccgccctgccactcatcgcagtactgttgtaattcattaagcattctgccgacatggaagccatcacaaacggcatgatgaacctgaatcgccagcggcatcagcaccttgtcgccttgcgtataatatttgcccatggtgaaaacgggggcgaagaagttgtccatattggccacgtttaaatcaaaactggtgaaactcacccagggattggctgagacgaaaaacatattctcaataaaccctttagggaaataggccaggttttcaccgtaacacgccacatcttgcgaatatatgtgtagaaactgccggaaatcgtcgtggtattcactccagagcgatgaaaacgtttcagtttgctcatggaaaacggtgtaacaagggtgaacactatcccatatcaccagctcaccgtctttcattgccatacgaaattccggatgagcattcatcaggcgggcaagaatgtgaataaaggccggataaaacttgtgcttatttttctttacggtctttaaaaaggccgtaatatccagctgaacggtctggttataggtacattgagcaactgactgaaatgcctcaaaatgttctttacgatgccattgggatatatcaacggtggtatatccagtgatttttttctccattttagcttccttagctcctgaaaatctcgataactcaaaaaatacgcccggtagtgatcttatttcattatggtgaaagttggaacctcttacgtgccgatcaacgtctcattttcgccagatatc

SEQ ID NO: 4 - DNA, 974 bp, Artificial Sequence
  Synthetic Construct Delta-cas3::ugpBp-sspB-proB
caagacatgtgtatatcactgtaattcgatatttatgagcagcatcgaaaaatagcccgctgatatcatcgataatactaaaaaaacagggaggctattaccaggcatcaaataaaacgaaaggctcagtcgaaagactgggcctttcgttttatctgttgtttgtcggtgaacgctctctactagagtcacactggctcaccttcgggtgggcctttctgcgtttatatctttctgacaccttactatcttacaaatgtaacaaaaaagttatttttctgtaattcgagcatgtcatgttaccccgcgagcataaaacgcgtgtgtaggaggataatctatggatttgtcacagctaacaccacgtcgtccctatctgctgcgtgcattctatgagtggttgctggataaccagctcacgccgcacctggtggtggatgtgacgctccctggcgtgcaggttcctatggaatatgcgcgtgacgggcaaatcgtactcaacattgcgccgcgtgctgtcggcaatctggaactggcgaatgatgaggtgcgctttaacgcgcgctttggtggcattccgcgtcaggtttctgtgccgctggctgccgtgctggctatctacgcccgtgaaaatggcgcaggcacgatgtttgagcctgaagctgcctacgatgaagataccagcatcatgaatgatgaagaggcatcggcagacaacgaaaccgttatgtcggttattgatggcgacaagccagatcacgatgatgacactcatcctgacgatgaacctccgcagccaccacgcggtggtcgaccggcattacgcgttgtgaagtaattgacggctagctcagtcctaggtacagtgctagccatatgaaggagaacaaatgaatttgcttattgataactggatccctgtacgcccgcgaaacggggggaaagtccaaatcataaatctgcaatcgctatac

SEQ ID NO: 5 - DNA, 1500 bp, Artificial Sequence
  Linear DNA Construct Delta-ptsG::proC-glk
ggctgtgttgaaaggtgttgccgttgaagaactggcgcaggtaaccaccgataacttcgcccgtctgtttcacatcgacgcttcccgccttcaatccatccgttgaatgagtttttttaaagctcgtaattaatacttcgctcttcatgccgccgcaaaccccgcccctgacagggcggggtttcgccgcacgtctccatcgcttgcccaagttgtgaagcacagctaacaccacgtcgtccctatctgctgccctaggtctatgagtggttgctggataactttacgggcatgcataaggctcgtatgatatattcagggagaccacaacggtttccctctacaaataattttgtttaactttcgtagaagagcacttccacacttctggaaaaaggagatataccatgaccaagtatgccctggtcggtgacgtaggtggtaccaatgcacgtctcgctctctgtgatatcgcaagcggggaaatttctcaggccaaaacatattccgggttggattaccccagcttagaagccgtgattcgtgtctatttagaagaacataaagtagaagtcaaagacggttgtattgctattgcgtgccccatcactggggattgggtagcaatgaccaaccatacctgggcgttttctattgccgagatgaaaaaaaatctgggtttctcacacctggagatcatcaacgattttaccgcggtgagcatggcgatcccaatgttaaaaaaggaacacttaattcagttcggcggggcagaacctgtggagggcaagccgatcgcggtttatggtgcaggcacaggcttaggtgtcgcgcacttggtacatgttgacaagcgctgggtgagtttgccgggcgaaggcggccacgtggattttgcccccaattctgaagaggaggcgattattctggaaatcttgcgtgcagaaatcggtcatgtgtctgccgaacgtgtgctgagtggtccaggtctggtgaatctgtaccgcgctattgtcaaagcggataaccgcctgccagaaaaccttaaaccgaaagatatcaccgaacgtgccttggccgactcctgtaccgattgccgccgcgcacttagtctgttttgcgttatcatgggtcgttttggcggcaacctcgcgctgaacctggggacctttggcggtgtttttattgcgggaggtattgttccacgctttttagaatttttcaaagccagtggctttcgcgcggccttcgaagacaagggacgttttaaagaatacgtacatgatatcccagtctatttaattgttcacgataacccaggactgttaggctctggtgcccatctgcgtcagacattgggccatattctgtaatccgtaagacgttggggagactaaggcagccagatggctgccttttttacaggtgttattcagaattgatacgtgccggtaatgctgaaattacgcggtgtgccgtagacgatagaaccttccacgt

SEQ ID NO: 6 - DNA, 1332 bp, Artificial Sequence
  Linear DNA Construct proC-galP
tatgtcgcgaaaaacatcgttgctgctggcctggccgatcgttgtgaaattcaggtttcctacgcaatcggcgtggctgaaccgacctccatcatggtagaaactttcggtactgagaaagtgccttctgaacaactgaccctgctggtacgtgagttcttcgacctgcgcccatacggtctgattcagatgctggatctgctgcacccgatctacaaagaaaccgcagcatacggtcactttggtcgtgaacatttcccgtgggaaaaaaccgacaaagcgcagctgctgcgcgatgctgccggtctgaagtaatctttcttcacctgcgttcaaaggacttcgctcttcatgccgccgcaaaccccgcccctgacagggcggggtttcgccgcacgtctccatcgcttgcccaagttgtgaagcacagctaacaccacgtcgtccctatctgctgccctaggtctatgagtggttgctggataactttacgggcatgcataaggctcgtatgatatattcagggagaccacaacggtttccctctacaaataattttgtttaactttcgtagaagagcacttccacacttctggaaaaaggagatataccatgccagatgccaaaaagcaaggccgttctaacaaggcaatgacattcttcgtgtgcttccttgcggcgcttgccggcctcttgttcggcttggacatcggcgtcattgccggtgctttaccatttatcgctgacgaattccagatcacctcgcacacgcaagaatgggtcgtaagctccatgatgttcggtgcggcagtcggtgcggtgggcagcggctggctctcctttaaactcgggcgcaaaaagagcctgatgatcggcgcaattttgtttgttgccggttcgctgttctctgcggctgcgccaaacgttgaagtactgattctttcccgcgttctactggggctggcggtgggtgtggcctcttataccgcaccgctgtacctctctgaaattgcgccggaaaaaattcgtggcagtatgatctcgatgtatcagttgatgatcactatcgggatcctcggtgcttatctttctgataccgccttcagctacaccggtgcatggcgctggatgctgggtgtgattatcatcccggcaattttgctgctgattggtgtcttcttcctgccagacagcccacgttggtttgccgccaaacgccgttttgttgatgccgaacgcgtgctgctacgcctgcgtgacaccagcgcggaagcgaaacgcgaactggatgaaatccgtgaaagtttgcaggttaaacagagtggctgggcg

SEQ ID NO: 7 - DNA, 970 bp, Artificial Sequence
  fabI-DAS+4:gentR
ctattgaagatgtgggtaactctgcggcattcctgtgctccgatctctctgccggtatctccggtgaagtggtccacgttgacggcggtttcagcattgctgcaatgaacgaactcgaactgaaagcggccaacgatgaaaactattctgaaaactatgcggatgcgtcttaataggaagttcctattctctagaaagtataggaacttccgaatccatgtgggagtttattcttgacacagatatttatgatataataactgagtaagcttaacataaggaggaaaaacatatgttacgcagcagcaacgatgttacgcagcagggcagtcgccctaaaacaaagttaggtggctcaagtatgggcatcattcgcacatgtaggctcggccctgaccaagtcaaatccatgcgggctgctcttgatcttttcggtcgtgagttcggagacgtagccacctactcccaacatcagccggactccgattacctcgggaacttgctccgtagtaagacattcatcgcgcttgctgccttcgaccaagaagcggttgttggcgctctcgcggcttacgttctgcccaagtttgagcagccgcgtagtgagatctatatctatgatctcgcagtctccggcgagcaccggaggcagggcattgccaccgcgctcatcaatctcctcaagcatgaggccaacgcgcttggtgcttatgtgatctacgtgcaagcagattacggtgacgatcccgcagtggctctctatacaaagttgggcatacgggaagaagtgatgcactttgatatcgacccaagtaccgccacctaagaagttcctattctctagaaagtataggaacttccgttctgttggtaaagatgggcggcgttctgccgcccgttatctctgttatacctttctgatatttgttatcgccgatccgtctttctccccttcccgccttgcgtcagg

SEQ ID NO: 8 - DNA, 1026 bp, Artificial Sequence
  lpd-DAS+4:gentR
ggtactaacggcggcgagctgctgggtgaaatcggcctggcaatcgaaatgggttgtgatgctgaagacatcgcactgaccatccacgcgcacccgactctgcacgagtctgtgggcctggcggcagaagtgttcgaaggtagcattaccgacctgccgaacccgaaagcgaagaagaaggcggccaacgatgaaaactattctgaaaactatgcggatgcgtcttaatagcgaatccatgtgggagtttattcttgacacagatatttatgatataataactgagtaagcttaacataaggaggaaaaacatatgttacgcagcagcaacgatgttacgcagcagggcagtcgccctaaaacaaagttaggtggctcaagtatgggcatcattcgcacatgtaggctcggccctgaccaagtcaaatccatgcgggctgctcttgatcttttcggtcgtgagttcggagacgtagccacctactcccaacatcagccggactccgattacctcgggaacttgctccgtagtaagacattcatcgcgcttgctgccttcgaccaagaagcggttgttggcgctctcgcggcttacgttctgcccaagtttgagcagccgcgtagtgagatctatatctatgatctcgcagtctccggcgagcaccggaggcagggcattgccaccgcgctcatcaatctcctcaagcatgaggccaacgcgcttggtgcttatgtgatctacgtgcaagcagattacggtgacgatcccgcagtggctctctatacaaagttgggcatacgggaagaagtgatgcactttgatatcgacccaagtaccgccacctaatttttcgtttgccggaacatccggcaattaaaaaagcggctaaccacgccgctttttttacgtctgcaatttacctttccagtcttcttgctccacgttcagagagacgttcgcatactgctgaccgttgctcgttattcagcctgacagtatggttactgtcgtttagacgttgtggg

SEQ ID NO: 9 - DNA, 869 bp, Artificial Sequence
  gltA-DAS+4:zeoR
gtattccgtcttccatgttcaccgtcattttcgcaatggcacgtaccgttggctggatcgcccactggagcgaaatgcacagtgacggtatgaagattgcccgtccgcgtcagctgtatacaggatatgaaaaacgcgactttaaaagcgatatcaagcgtgcggccaacgatgaaaactattctgaaaactatgcggatgcgtcttaatagttgacaattaatcatcggcatagtatatcggcatagtataatacgactcactataggagggccatcatggccaagttgaccagtgccgttccggtgctcaccgcgcgcgacgtcgccggagcggtcgagttctggaccgaccggctcgggttctcccgggacttcgtggaggacgacttcgccggtgtggtccgggacgacgtgaccctgttcatcagcgcggtccaggaccaggtggtgccggacaacaccctggcctgggtgtgggtgcgcggcctggacgagctgtacgccgagtggtcggaggtcgtgtccacgaacttccgggacgcctccgggccggccatgaccgagatcggcgagcagccgtgggggcgggagttcgccctgcgcgacccggccggcaactgcgtgcactttgtggcagaggagcaggactgaggataagtaatggttgattgctaagttgtaaatattttaacccgccgttcatatggcgggttgatttttatatgcctaaacacaaaaaattgtaaaaataaaatccattaacagacctatatagatatttaaaaagaatagaacagctcaaattatcagcaacccaatactttcaattaaaaacttcatggtagtcgcatttataaccctatgaaa

SEQ ID NO: 10 - DNA, 852 bp, Artificial Sequence
  udhA-DAS+4:bsdR
tctgggtattcactgctttggcgagcgcgctgccgaaattattcatatcggtcaggcgattatggaacagaaaggtggcggcaacactattgagtacttcgtcaacaccacctttaactacccgacgatggcggaagcctatcgggtagctgcgttaaacggtttaaaccgcctgtttgcggccaacgatgaaaactattctgaaaactatgcggatgcgtcttaatagttgacaattaatcatcggcatagtatatcggcatagtataatacgactcactataggagggccatcatgaagaccttcaacatctctcagcaggatctggagctggtggaggtcgccactgagaagatcaccatgctctatgaggacaacaagcaccatgtcggggcggccatcaggaccaagactggggagatcatctctgctgtccacattgaggcctacattggcagggtcactgtctgtgctgaagccattgccattgggtctgctgtgagcaacgggcagaaggactttgacaccattgtggctgtcaggcacccctactctgatgaggtggacagatccatcagggtggtcagcccctgtggcatgtgcagagagctcatctctgactatgctcctgactgctttgtgctcattgagatgaatggcaagctggtcaaaaccaccattgaggaactcatccccctcaagtacaccaggaactaaagtaaaactttatcgaaatggccatccattcttgcgcggatggcctctgccagctgctcatagcggctgcgcagcggtgagccaggacgataaaccaggccaatagtgcggcgtggttccggcttaatgcacgg

SEQ ID NO: 11 - DNA, 898 bp, Artificial Sequence
  zwf-DAS+4:bsdR
gaagtggaagaagcctggaaatgggtagactccattactgaggcgtgggcgatggacaatgatgcgccgaaaccgtatcaggccggaacctggggacccgttgcctcggtggcgatgattacccgtgatggtcgttcctggaatgagtttgaggcggccaacgatgaaaactattctgaaaactatgcggatgcgtcttaatagttgacaattaatcatcggcatagtatatcggcatagtataatacgactcactataggagggccatcatgaagaccttcaacatctctcagcaggatctggagctggtggaggtcgccactgagaagatcaccatgctctatgaggacaacaagcaccatgtcggggcggccatcaggaccaagactggggagatcatctctgctgtccacattgaggcctacattggcagggtcactgtctgtgctgaagccattgccattgggtctgctgtgagcaacgggcagaaggactttgacaccattgtggctgtcaggcacccctactctgatgaggtggacagatccatcagggtggtcagcccctgtggcatgtgcagagagctcatctctgactatgctcctgactgctttgtgctcattgagatgaatggcaagctggtcaaaaccaccattgaggaactcatccccctcaagtacaccaggaactaaagtaatatctgcgcttatcctttatggttattttaccggtaacatgatcttgcgcagattgtagaacaatttttacactttcaggcctcgtgcggattcacccacgaggctttttttattacactgactgaaacgtttttgccctatgagctccggttacaggcgtttcagtcataaatcctctgaatgaaacgcgttgtgaatc

SEQ ID NO: 12 - DNA, 3037 bp, Artificial Sequence
  Plasmid pSMART-waaHp-GFPuv
tgcccaggcatcaaataaaacgaaaggctcagtcgaaagactgggcctttcgttttatctgttgtttgtcggtgaacgctctctactagagtcacactggctcaccttcgggtgggcctttctgcgtttatacacagctaacaccacgtcgtccctatctgctgccctaggtctatgagtggttgctggataacgtgcgtaattgtgctgatctcttatatagctgctctcattatctctctaccctgaagtgactctctcacctgtaaaaataatatctcacaggcttaatagtttcttaatacaaagcctgtaaaacgtcaggataacttctatattcagggagaccacaacggtttccctctacaaataattttgtttaactttcgtgtgtaggaggataatctatggctagcaaaggagaagaacttttcactggagttgtcccaattcttgttgaattagatggtgatgttaatgggcacaaattttctgtcagtggagagggtgaaggtgatgctacatacggaaagcttacccttaaatttatttgcactactggaaaactacctgttccatggccaacacttgtcactactttctcttatggtgttcaatgcttttcccgttatccggatcatatgaaacggcatgactttttcaagagtgccatgcccgaaggttatgtacaggaacgcactatatctttcaaagatgacgggaactacaagacgcgtgctgaagtcaagtttgaaggtgatacccttgttaatcgtatcgagttaaaaggtattgattttaaagaagatggaaacattctcggacacaaactcgagtacaactataactcacacaatgtatacatcacggcagacaaacaaaagaatggaatcaaagctaacttcaaaattcgccacaacattgaagatggatccgttcaactagcagaccattatcaacaaaatactccaattggcgatggccctgtccttttaccagacaaccattacctgtcgacacaatctgccctttcgaaagatcccaacgaaaagcgtgaccacatggtccttcttgagtttgtaactgctgctgggattacacatggcatggatgagctctacaaataatgaggatccccggcttatcggtcagtttcacctgatttacgtaaaaacccgcttcggcgggtttttgcttttggaggggcagaaagatgaatgactgtccacgacgctatacccaaaagaaagacgaattctctagatatcgctcaatactgaccatttaaatcatacctgacctccatagcagaaagtcaaaagcctccgaccggaggcttttgacttgatcggcacgtaagaggttccaactttcaccataatgaaataagatcactaccgggcgtattttttgagttatcgagattttcaggagctaaggaagctaaaatgagccatattcaacgggaaacgtcttgctcgaggccgcgattaaattccaacatggatgctgatttatatgggtataaatgggctcgcgataatgtcgggcaatcaggtgcgacaatctatcgattgtatgggaagcccgatgcgccagagttgtttctgaaacatggcaaaggtagcgttgccaatgatgttacagatgagatggtcaggctaaactggctgacggaatttatgcctcttccgaccatcaagcattttatccgtactcctgatgatgcatggttactcaccactgcgatcccagggaaaacagcattccaggtattagaagaatatcctgattcaggtgaaaatattgttgatgcgctggcagtgttcctgcgccggttgcattcgattcctgtttgtaattgtccttttaacggcgatcgcgtatttcgtctcgctcaggcgcaatcacgaatgaataacggtttggttggtgcgagtgattttgatgacgagcgtaatggctggcctgttgaacaagtctggaaagaaatgcataagcttttgccattctcaccggattcagtcgtcactcatggtgatttctcacttgataaccttatttttgacgaggggaaattaataggttgtattgatgttggacgagtcggaatcgcagaccgataccaggatcttgccatcctatggaactgcctcggtgagttttctccttcattacagaaacggctttttcaaaaatatggtattgataatcctgatatgaataaattgcagtttcacttgatgctcgatgagtttttctaatgagggcccaaatgtaatcacctggctcaccttcgggtgggcctttctgcgttgctggcgtttttccataggctccgcccccctgacgagcatcacaaaaatcgatgctcaagtcagaggtggcgaaacccgacaggactataaagataccaggcgtttccccctggaagctccctcgtgcgctctcctgttccgaccctgccgcttaccggatacctgtccgcctttctcccttcgggaagcgtggcgctttctcatagctcacgctgtaggtatctcagttcggtgtaggtcgttcgctccaagctgggctgtgtgcacgaaccccccgttcagcccgaccgctgcgccttatccggtaactatcgtcttgagtccaacccggtaagacacgacttatcgccactggcagcagccactggtaacaggattagcagagcgaggtatgtaggcggtgctacagagttcttgaagtggtggcctaactacggctacactagaagaacagtatttggtatctgcgctctgctgaagccagttacctcggaaaaagagttggtagctcttgatccggcaaacaaaccaccgctggtagcggtggtttttttgtttgcaagcagcagattacgcgcagaaaaaaaggatctcaagaagatcctttgattttctaccgaagaaaggcccacccgtgaaggtgagccagtgagttgattgcagtccagttacgctggagtctgaggctcgtcctgaatgatatcaagcttgaattcgtt

SEQ ID NO: 13 - DNA, 2780 bp, Artificial Sequence
  pCASCADE-Control Plasmid
gacgtcttaagacccactttcacatttaagttgtttttctaatccgcatatgatcaattcaaggccgaataagaaggctggctctgcaccttggtgatcaaataattcgatagcttgtcgtaataatggcggcatactatcagtagtaggtgtttccctttcttctttagcgacttgatgctcttgatcttccaatacgcaacctaaagtaaaatgccccacagcgctgagtgcatataatgcattctctagtgaaaaaccttgttggcataaaaaggctaattgattttcgagagtttcatactgtttttctgtaggccgtgtacctaaatgtacttttgctccatcgcgatgacttagtaaagcacatctaaaacttttagcgttattacgtaaaaaatcttgccagctttccccttctaaagggcaaaagtgagtatggtgcctatctaacatctcaatggctaaggcgtcgagcaaagcccgcttattttttacatgccaatacaatgtaggctgctctacacctagcttctgggcgagtttacgggttgttaaaccttcgattccgacctcattaagcagctctaatgcgctgttaatcactttacttttatctaatctagacatcatccaggcatcaaataaaacgaaaggctcagtcgaaagactgggcctttcgttttatctgttgtttgtcggtgaacgctctctactagagtcacactggctcaccttcgggtgggcctttctgcgtttatacacagctaacaccacgtcgtccctatctgctgccctaggtctatgagtggttgctggataactctttctgacaccttactatcttacaaatgtaacaaaaaagttatttttctgtaattcgagcatgtcatgttaccccgcgagcataaaacgcgtatattcagggagaccacaacggtttccctctacaaataattttgtttaactttgaattcaaaagatctggtaccacctcgagttccccgcgccagcggggataaaccgaaaaaaaaaccccgcccctgacagggcggggttttttttcctagggatatattccgcttcctcgctcactgactcgctacgctcggtcgttcgactgcggcgagcggaaatggcttacgaacggggcggagatttcctggaagatgccaggaagatacttaacagggaagtgagagggccgcggcaaagccgtttttccataggctccgcccccctgacaagcatcacgaaatctgacgctcaaatcagtggtggcgaaacccgacaggactataaagataccaggcgtttccccctggcggctccctcgtgcgctctcctgttcctgcctttcggtttaccggtgtcattccgctgttatggccgcgtttgtctcattccacgcctgacactcagttccgggtaggcagttcgctccaagctggactgtatgcacgaaccccccgttcagtccgaccgctgcgccttatccggtaactatcgtcttgagtccaacccggaaagacatgcaaaagcaccactggcagcagccactggtaattgatttagaggagttagtcttgaagtcatgcgccggttaaggctaaactgaaaggacaagttttggtgactgcgctcctccaagccagttacctcggttcaaagagttggtagctcagagaaccttcgaaaaaccgccctgcaaggcggttttttcgttttcagagcaagagattacgcgcagaccaaaacgatctcaagaagatcatcttattaatcagataaaatatttctagatttcagtgcaatttatctcttcaaatgtagcacctgaagtcagccccatacgatataagttgttactagtgcttggattctcaccaataaaaaacgcccggcggcaaccgagcgttctgaacaaatccagatggagttctgaggtcattactggatctatcaacaggagtccaagcgagctcgatatcaaattacgccccgccctgccactcatcgcagtactgttgtaattcattaagcattctgccgacatggaagccatcacaaacggcatgatgaacctgaatcgccagcggcatcagcaccttgtcgccttgcgtataatatttgcccatggtgaaaacgggggcgaagaagttgtccatattggccacgtttaaatcaaaactggtgaaactcacccagggattggctgagacgaaaaacatattctcaataaaccctttagggaaataggccaggttttcaccgtaacacgccacatcttgcgaatatatgtgtagaaactgccggaaatcgtcgtggtattcactccagagcgatgaaaacgtttcagtttgctcatggaaaacggtgtaacaagggtgaacactatcccatatcaccagctcaccgtctttcattgccatacgaaattccggatgagcattcatcaggcgggcaagaatgtgaataaaggccggataaaacttgtgcttatttttctttacggtctttaaaaaggccgtaatatccagctgaacggtctggttataggtacattgagcaactgactgaaatgcctcaaaatgttctttacgatgccattgggatatatcaacggtggtatatccagtgatttttttctccattttagcttccttagctcctgaaaatctcgataactcaaaaaatacgcccggtagtgatcttatttcattatggtgaaagttggaacctcttacgtgccgatcaacgtctcattttcgccagatatc

SEQ ID NO: 14 - DNA, 2843 bp, Artificial Sequence
  pCASCADE-gltA2 Plasmid
gacgtcttaagacccactttcacatttaagttgtttttctaatccgcatatgatcaattcaaggccgaataagaaggctggctctgcaccttggtgatcaaataattcgatagcttgtcgtaataatggcggcatactatcagtagtaggtgtttccctttcttctttagcgacttgatgctcttgatcttccaatacgcaacctaaagtaaaatgccccacagcgctgagtgcatataatgcattctctagtgaaaaaccttgttggcataaaaaggctaattgattttcgagagtttcatactgtttttctgtaggccgtgtacctaaatgtacttttgctccatcgcgatgacttagtaaagcacatctaaaacttttagcgttattacgtaaaaaatcttgccagctttccccttctaaagggcaaaagtgagtatggtgcctatctaacatctcaatggctaaggcgtcgagcaaagcccgcttattttttacatgccaatacaatgtaggctgctctacacctagcttctgggcgagtttacgggttgttaaaccttcgattccgacctcattaagcagctctaatgcgctgttaatcactttacttttatctaatctagacatcatccaggcatcaaataaaacgaaaggctcagtcgaaagactgggcctttcgttttatctgttgtttgtcggtgaacgctctctactagagtcacactggctcaccttcgggtgggcctttctgcgtttatacacagctaacaccacgtcgtccctatctgctgccctaggtctatgagtggttgctggataactctttctgacaccttactatcttacaaatgtaacaaaaaagttatttttctgtaattcgagcatgtcatgttaccccgcgagcataaaacgcgtatattcagggagaccacaacggtttccctctacaaataattttgtttaactttgaattcaaaagatctggtaccacctcgagttccccgcgccagcggggataaaccgtattgaccaattcattcgggacagttattagttcgagttccccgcgccagcggggataaaccgaaaaaaaaaccccgcccctgacagggcggggttttttttcctagggatatattccgcttcctcgctcactgactcgctacgctcggtcgttcgactgcggcgagcggaaatggcttacgaacggggcggagatttcctggaagatgccaggaagatacttaacagggaagtgagagggccgcggcaaagccgtttttccataggctccgcccccctgacaagcatcacgaaatctgacgctcaaatcagtggtggcgaaacccgacaggactataaagataccaggcgtttccccctggcggctccctcgtgcgctctcctgttcctgcctttcggtttaccggtgtcattccgctgttatggccgcgtttgtctcattccacgcctgacactcagttccgggtaggcagttcgctccaagctggactgtatgcacgaaccccccgttcagtccgaccgctgcgccttatccggtaactatcgtcttgagtccaacccggaaagacatgcaaaagcaccactggcagcagccactggtaattgatttagaggagttagtcttgaagtcatgcgccggttaaggctaaactgaaaggacaagttttggtgactgcgctcctccaagccagttacctcggttcaaagagttggtagctcagagaaccttcgaaaaaccgccctgcaaggcggttttttcgttttcagagcaagagattacgcgcagaccaaaacgatctcaagaagatcatcttattaatcagataaaatatttctagatttcagtgcaatttatctcttcaaatgtagcacctgaagtcagccccatacgatataagttgttactagtgcttggattctcaccaataaaaaacgcccggcggcaaccgagcgttctgaacaaatccagatggagttctgaggtcattactggatctatcaacaggagtccaagcgagctcgatatcaaattacgccccgccctgccactcatcgcagtactgttgtaattcattaagcattctgccgacatggaagccatcacaaacggcatgatgaacctgaatcgccagcggcatcagcaccttgtcgccttgcgtataatatttgcccatggtgaaaacgggggcgaagaagttgtccatattggccacgtttaaatcaaaactggtgaaactcacccagggattggctgagacgaaaaacatattctcaataaaccctttagggaaataggccaggttttcaccgtaacacgccacatcttgcgaatatatgtgtagaaactgccggaaatcgtcgtggtattcactccagagcgatgaaaacgtttcagtttgctcatggaaaacggtgtaacaagggtgaacactatcccatatcaccagctcaccgtctttcattgccatacgaaattccggatgagcattcatcaggcgggcaagaatgtgaataaaggccggataaaacttgtgcttatttttctttacggtctttaaaaaggccgtaatatccagctgaacggtctggttataggtacattgagcaactgactgaaatgcctcaaaatgttctttacgatgccattgggatatatcaacggtggtatatccagtgatttttttctccattttagcttccttagctcctgaaaatctcgataactcaaaaaatacgcccggtagtgatcttatttcattatggtgaaagttggaacctcttacgtgccgatcaacgtctcattttcgccagatatc

SEQ ID NO: 15 - DNA, 2841 bp, Artificial Sequence
  pCASCADE-fabI Plasmid
gacgtcttaagacccactttcacatttaagttgtttttctaatccgcatatgatcaattcaaggccgaataagaaggctggctctgcaccttggtgatcaaataattcgatagcttgtcgtaataatggcggcatactatcagtagtaggtgtttccctttcttctttagcgacttgatgctcttgatcttccaatacgcaacctaaagtaaaatgccccacagcgctgagtgcatataatgcattctctagtgaaaaaccttgttggcataaaaaggctaattgattttcgagagtttcatactgtttttctgtaggccgtgtacctaaatgtacttttgctccatcgcgatgacttagtaaagcacatctaaaacttttagcgttattacgtaaaaaatcttgccagctttccccttctaaagggcaaaagtgagtatggtgcctatctaacatctcaatggctaaggcgtcgagcaaagcccgcttattttttacatgccaatacaatgtaggctgctctacacctagcttctgggcgagtttacgggttgttaaaccttcgattccgacctcattaagcagctctaatgcgctgttaatcactttacttttatctaatctagacatcatccaggcatcaaataaaacgaaaggctcagtcgaaagactgggcctttcgttttatctgttgtttgtcggtgaacgctctctactagagtcacactggctcaccttcgggtgggcctttctgcgtttatacacagctaacaccacgtcgtccctatctgctgccctaggtctatgagtggttgctggataactctttctgacaccttactatcttacaaatgtaacaaaaaagttatttttctgtaattcgagcatgtcatgttaccccgcgagcataaaacgcgtatattcagggagaccacaacggtttccctctacaaataattttgtttaactttgaattcaaaagatctggtaccacctcgagttccccgcgccagcggggataaaccgttgattataataaccgtttatctgttcgtatcgagttccccgcgccagcggggataaaccgaaaaaaaaaccccgcccctgacagggcggggttttttttcctagggatatattccgcttcctcgctcactgactcgctacgctcggtcgttcgactgcggcgagcggaaatggcttacgaacggggcggagatttcctggaagatgccaggaagatacttaacagggaagtgagagggccgcggcaaagccgtttttccataggctccgcccccctgacaagcatcacgaaatctgacgctcaaatcagtggtggcgaaacccgacaggactataaagataccaggcgtttccccctggcggctccctcgtgcgctctcctgttcctgcctttcggtttaccggtgtcattccgctgttatggccgcgtttgtctcattccacgcctgacactcagttccgggtaggcagttcgctccaagctggactgtatgcacgaaccccccgttcagtccgaccgctgcgccttatccggtaactatcgtcttgagtccaacccggaaagacatgcaaaagcaccactggcagcagccactggtaattgatttagaggagttagtcttgaagtcatgcgccggttaaggctaaactgaaaggacaagttttggtgactgcgctcctccaagccagttacctcggttcaaagagttggtagctcagagaaccttcgaaaaaccgccctgcaaggcggttttttcgttttcagagcaagagattacgcgcagaccaaaacgatctcaagaagatcatcttattaatcagataaaatatttctagatttcagtgcaatttatctcttcaaatgtagcacctgaagtcagccccatacgatataagttgttactagtgcttggattctcaccaataaaaaacgcccggcggcaaccgagcgttctgaacaaatccagatggagttctgaggtcattactggatctatcaacaggagtccaagcgagctcgatatcaaattacgccccgccctgccactcatcgcagtactgttgtaattcattaagcattctgccgacatggaagccatcacaaacggcatgatgaacctgaatcgccagcggcatcagcaccttgtcgccttgcgtataatatttgcccatggtgaaaacgggggcgaagaagttgtccatattggccacgtttaaatcaaaactggtgaaactcacccagggattggctgagacgaaaaacatattctcaataaaccctttagggaaataggccaggttttcaccgtaacacgccacatcttgcgaatatatgtgtagaaactgccggaaatcgtcgtggtattcactccagagcgatgaaaacgtttcagtttgctcatggaaaacggtgtaacaagggtgaacactatcccatatcaccagctcaccgtctttcattgccatacgaaattccggatgagcattcatcaggcgggcaagaatgtgaataaaggccggataaaacttgtgcttatttttctttacggtctttaaaaaggccgtaatatccagctgaacggtctggttataggtacattgagcaactgactgaaatgcctcaaaatgttctttacgatgccattgggatatatcaacggtggtatatccagtgatttttttctccattttagcttccttagctcctgaaaatctcgataactcaaaaaatacgcccggtagtgatcttatttcattatggtgaaagttggaacctcttacgtgccgatcaacgtctcattttcgccagatatc

SEQ ID NO: 16 - DNA, 2841 bp, Artificial Sequence
  pCASCADE-udhA Plasmid
gacgtcttaagacccactttcacatttaagttgtttttctaatccgcatatgatcaattcaaggccgaataagaaggctggctctgcaccttggtgatcaaataattcgatagcttgtcgtaataatggcggcatactatcagtagtaggtgtttccctttcttctttagcgacttgatgctcttgatcttccaatacgcaacctaaagtaaaatgccccacagcgctgagtgcatataatgcattctctagtgaaaaaccttgttggcataaaaaggctaattgattttcgagagtttcatactgtttttctgtaggccgtgtacctaaatgtacttttgctccatcgcgatgacttagtaaagcacatctaaaacttttagcgttattacgtaaaaaatcttgccagctttccccttctaaagggcaaaagtgagtatggtgcctatctaacatctcaatggctaaggcgtcgagcaaagcccgcttattttttacatgccaatacaatgtaggctgctctacacctagcttctgggcgagtttacgggttgttaaaccttcgattccgacctcattaagcagctctaatgcgctgttaatcactttacttttatctaatctagacatcatccaggcatcaaataaaacgaaaggctcagtcgaaagactgggcctttcgttttatctgttgtttgtcggtgaacgctctctactagagtcacactggctcaccttcgggtgggcctttctgcgtttatacacagctaacaccacgtcgtccctatctgctgccctaggtctatgagtggttgctggataactctttctgacaccttactatcttacaaatgtaacaaaaaagttatttttctgtaattcgagcatgtcatgttaccccgcgagcataaaacgcgtatattcagggagaccacaacggtttccctctacaaataattttgtttaactttgaattcaaaagatctggtaccacctcgagttccccgcgccagcggggataaaccgttaccattctgttgcttttatgtataagaatcgagttccccgcgccagcggggataaaccgaaaaaaaaaccccgcccctgacagggcggggttttttttcctagggatatattccgcttcctcgctcactgactcgctacgctcggtcgttcgactgcggcgagcggaaatggcttacgaacggggcggagatttcctggaagatgccaggaagatacttaacagggaagtgagagggccgcggcaaagccgtttttccataggctccgcccccctgacaagcatcacgaaatctgacgctcaaatcagtggtggcgaaacccgacaggactataaagataccaggcgtttccccctggcggctccctcgtgcgctctcctgttcctgcctttcggtttaccggtgtcattccgctgttatggccgcgtttgtctcattccacgcctgacactcagttccgggtaggcagttcgctccaagctggactgtatgcacgaaccccccgttcagtccgaccgctgcgccttatccggtaactatcgtcttgagtccaacccggaaagacatgcaaaagcaccactggcagcagccactggtaattgatttagaggagttagtcttgaagtcatgcgccggttaaggctaaactgaaaggacaagttttggtgactgcgctcctccaagccagttacctcggttcaaagagttggtagctcagagaaccttcgaaaaaccgccctgcaaggcggttttttcgttttcagagcaagagattacgcgcagaccaaaacgatctcaagaagatcatcttattaatcagataaaatatttctagatttcagtgcaatttatctcttcaaatgtagcacctgaagtcagccccatacgatataagttgttactagtgcttggattctcaccaataaaaaacgcccggcggcaaccgagcgttctgaacaaatccagatggagttctgaggtcattactggatctatcaacaggagtccaagcgagctcgatatcaaattacgccccgccctgccactcatcgcagtactgttgtaattcattaagcattctgccgacatggaagccatcacaaacggcatgatgaacctgaatcgccagcggcatcagcaccttgtcgccttgcgtataatatttgcccatggtgaaaacgggggcgaagaagttgtccatattggccacgtttaaatcaaaactggtgaaactcacccagggattggctgagacgaaaaacatattctcaataaaccctttagggaaataggccaggttttcaccgtaacacgccacatcttgcgaatatatgtgtagaaactgccggaaatcgtcgtggtattcactccagagcgatgaaaacgtttcagtttgctcatggaaaacggtgtaacaagggtgaacactatcccatatcaccagctcaccgtctttcattgccatacgaaattccggatgagcattcatcaggcgggcaagaatgtgaataaaggccggataaaacttgtgcttatttttctttacggtctttaaaaaggccgtaatatccagctgaacggtctggttataggtacattgagcaactgactgaaatgcctcaaaatgttctttacgatgccattgggatatatcaacggtggtatatccagtgatttttttctccattttagcttccttagctcctgaaaatctcgataactcaaaaaatacgcccggtagtgatcttatttcattatggtgaaagttggaacctcttacgtgccgatcaacgtctcattttcgccagatatc

SEQ ID NO: 17 - DNA, 2841 bp, Artificial Sequence
  pCASCADE-zwf Plasmid
gacgtcttaagacccactttcacatttaagttgtttttctaatccgcatatgatcaattcaaggccgaataagaaggctggctctgcaccttggtgatcaaataattcgatagcttgtcgtaataatggcggcatactatcagtagtaggtgtttccctttcttctttagcgacttgatgctcttgatcttccaatacgcaacctaaagtaaaatgccccacagcgctgagtgcatataatgcattctctagtgaaaaaccttgttggcataaaaaggctaattgattttcgagagtttcatactgtttttctgtaggccgtgtacctaaatgtacttttgctccatcgcgatgacttagtaaagcacatctaaaacttttagcgttattacgtaaaaaatcttgccagctttccccttctaaagggcaaaagtgagtatggtgcctatctaacatctcaatggctaaggcgtcgagcaaagcccgcttattttttacatgccaatacaatgtaggctgctctacacctagcttctgggcgagtttacgggttgttaaaccttcgattccgacctcattaagcagctctaatgcgctgttaatcactttacttttatctaatctagacatcatccaggcatcaaataaaacgaaaggctcagtcgaaagactgggcctttcgttttatctgttgtttgtcggtgaacgctctctactagagtcacactggctcaccttcgggtgggcctttctgcgtttatacacagctaacaccacgtcgtccctatctgctgccctaggtctatgagtggttgctggataactctttctgacaccttactatcttacaaatgtaacaaaaaagttatttttctgtaattcgagcatgtcatgttaccccgcgagcataaaacgcgtatattcagggagaccacaacggtttccctctacaaataattttgtttaactttgaattcaaaagatctggtaccacctcgagttccccgcgccagcggggataaaccgctcgtaaaagcagtacagtgcaccgtaagatcgagttccccgcgccagcggggataaaccgaaaaaaaaaccccgcccctgacagggcggggttttttttcctagggatatattccgcttcctcgctcactgactcgctacgctcggtcgttcgactgcggcgagcggaaatggcttacgaacggggcggagatttcctggaagatgccaggaagatacttaacagggaagtgagagggccgcggcaaagccgtttttccataggctccgcccccctgacaagcatcacgaaatctgacgctcaaatcagtggtggcgaaacccgacaggactataaagataccaggcgtttccccctggcggctccctcgtgcgctctcctgttcctgcctttcggtttaccggtgtcattccgctgttatggccgcgtttgtctcattccacgcctgacactcagttccgggtaggcagttcgctccaagctggactgtatgcacgaaccccccgttcagtccgaccgctgcgccttatccggtaactatcgtcttgagtccaacccggaaagacatgcaaaagcaccactggcagcagccactggtaattgatttagaggagttagtcttgaagtcatgcgccggttaaggctaaactgaaaggacaagttttggtgactgcgctcctccaagccagttacctcggttcaaagagttggtagctcagagaaccttcgaaaaaccgccctgcaaggcggttttttcgttttcagagcaagagattacgcgcagaccaaaacgatctcaagaagatcatcttattaatcagataaaatatttctagatttcagtgcaatttatctcttcaaatgtagcacctgaagtcagccccatacgatataagttgttactagtgcttggattctcaccaataaaaaacgcccggcggcaaccgagcgttctgaacaaatccagatggagttctgaggtcattactggatctatcaacaggagtccaagcgagctcgatatcaaattacgccccgccctgccactcatcgcagtactgttgtaattcattaagcattctgccgacatggaagccatcacaaacggcatgatgaacctgaatcgccagcggcatcagcaccttgtcgccttgcgtataatatttgcccatggtgaaaacgggggcgaagaagttgtccatattggccacgtttaaatcaaaactggtgaaactcacccagggattggctgagacgaaaaacatattctcaataaaccctttagggaaataggccaggttttcaccgtaacacgccacatcttgcgaatatatgtgtagaaactgccggaaatcgtcgtggtattcactccagagcgatgaaaacgtttcagtttgctcatggaaaacggtgtaacaagggtgaacactatcccatatcaccagctcaccgtctttcattgccatacgaaattccggatgagcattcatcaggcgggcaagaatgtgaataaaggccggataaaacttgtgcttatttttctttacggtctttaaaaaggccgtaatatccagctgaacggtctggttataggtacattgagcaactgactgaaatgcctcaaaatgttctttacgatgccattgggatatatcaacggtggtatatccagtgatttttttctccattttagcttccttagctcctgaaaatctcgataactcaaaaaatacgcccggtagtgatcttatttcattatggtgaaagttggaacctcttacgtgccgatcaacgtctcattttcgccagatatc

SEQ ID NO: 18 - DNA, 2842 bp, Artificial Sequence
  pCASCADE-gltA1 Plasmid
gacgtcttaagacccactttcacatttaagttgtttttctaatccgcatatgatcaattcaaggccgaataagaaggctggctctgcaccttggtgatcaaataattcgatagcttgtcgtaataatggcggcatactatcagtagtaggtgtttccctttcttctttagcgacttgatgctcttgatcttccaatacgcaacctaaagtaaaatgccccacagcgctgagtgcatataatgcattctctagtgaaaaaccttgttggcataaaaaggctaattgattttcgagagtttcatactgtttttctgtaggccgtgtacctaaatgtacttttgctccatcgcgatgacttagtaaagcacatctaaaacttttagcgttattacgtaaaaaatcttgccagctttccccttctaaagggcaaaagtgagtatggtgcctatctaacatctcaatggctaaggcgtcgagcaaagcccgcttattttttacatgccaatacaatgtaggctgctctacacctagcttctgggcgagtttacgggttgttaaaccttcgattccgacctcattaagcagctctaatgcgctgttaatcactttacttttatctaatctagacatcatccaggcatcaaataaaacgaaaggctcagtcgaaagactgggcctttcgttttatctgttgtttgtcggtgaacgctctctactagagtcacactggctcaccttcgggtgggcctttctgcgtttatacacagctaacaccacgtcgtccctatctgctgccctaggtctatgagtggttgctggataactctttctgacaccttactatcttacaaatgtaacaaaaaagttatttttctgtaattcgagcatgtcatgttaccccgcgagcataaaacgcgtatattcagggagaccacaacggtttccctctacaaataattttgtttaactttgaattcaaaagatctggtaccacctcgagttccccgcgccagcggggataaaccgaaaagcatataatgcgtaaaagttatgaagttcgagttccccgcgccagcggggataaaccgaaaaaaaaaccccgcccctgacagggcggggttttttttcctagggatatattccgcttcctcgctcactgactcgctacgctcggtcgttcgactgcggcgagcggaaatggcttacgaacggggcggagatttcctggaagatgccaggaagatacttaacagggaagtgagagggccgcggcaaagccgtttttccataggctccgcccccctgacaagcatcacgaaatctgacgctcaaatcagtggtggcgaaacccgacaggactataaagataccaggcgtttccccctggcggctccctcgtgcgctctcctgttcctgcctttcggtttaccggtgtcattccgctgttatggccgcgtttgtctcattccacgcctgacactcagttccgggtaggcagttcgctccaagctggactgtatgcacgaaccccccgttcagtccgaccgctgcgccttatccggtaactatcgtcttgagtccaacccggaaagacatgcaaaagcaccactggcagcagccactggtaattgatttagaggagttagtcttgaagtcatgcgccggttaaggctaaactgaaaggacaagttttggtgactgcgctcctccaagccagttacctcggttcaaagagttggtagctcagagaaccttcgaaaaaccgccctgcaaggcggttttttcgttttcagagcaagagattacgcgcagaccaaaacgatctcaagaagatcatcttattaatcagataaaatatttctagatttcagtgcaatttatctcttcaaatgtagcacctgaagtcagccccatacgatataagttgttactagtgcttggattctcaccaataaaaaacgcccggcggcaaccgagcgttctgaacaaatccagatggagttctgaggtcattactggatctatcaacaggagtccaagcgagctcgatatcaaattacgccccgccctgccactcatcgcagtactgttgtaattcattaagcattctgccgacatggaagccatcacaaacggcatgatgaacctgaatcgccagcggcatcagcaccttgtcgccttgcgtataatatttgcccatggtgaaaacgggggcgaagaagttgtccatattggccacgtttaaatcaaaactggtgaaactcacccagggattggctgagacgaaaaacatattctcaataaaccctttagggaaataggccaggttttcaccgtaacacgccacatcttgcgaatatatgtgtagaaactgccggaaatcgtcgtggtattcactccagagcgatgaaaacgtttcagtttgctcatggaaaacggtgtaacaagggtgaacactatcccatatcaccagctcaccgtctttcattgccatacgaaattccggatgagcattcatcaggcgggcaagaatgtgaataaaggccggataaaacttgtgcttatttttctttacggtctttaaaaaggccgtaatatccagctgaacggtctggttataggtacattgagcaactgactgaaatgcctcaaaatgttctttacgatgccattgggatatatcaacggtggtatatccagtgatttttttctccattttagcttccttagctcctgaaaatctcgataactcaaaaaatacgcccggtagtgatcttatttcattatggtgaaagttggaacctcttacgtgccgatcaacgtctcattttcgccagatatc

SEQ ID NO: 19 - DNA, 2903 bp, Artificial Sequence
  pCASCADE-gltA2-udhA Plasmid
gacgtcttaagacccactttcacatttaagttgtttttctaatccgcatatgatcaattcaaggccgaataagaaggctggctctgcaccttggtgatcaaataattcgatagcttgtcgtaataatggcggcatactatcagtagtaggtgtttccctttcttctttagcgacttgatgctcttgatcttccaatacgcaacctaaagtaaaatgccccacagcgctgagtgcatataatgcattctctagtgaaaaaccttgttggcataaaaaggctaattgattttcgagagtttcatactgtttttctgtaggccgtgtacctaaatgtacttttgctccatcgcgatgacttagtaaagcacatctaaaacttttagcgttattacgtaaaaaatcttgccagctttccccttctaaagggcaaaagtgagtatggtgcctatctaacatctcaatggctaaggcgtcgagcaaagcccgcttattttttacatgccaataaatgtaggctgctctacacctagcttctgggcgagtttacgggttgttaaaccttcgattccgacctcattaagcagctctaatgcgctgttaatcactttacttttatctaatctagacatcatccaggcatcaaataaaacgaaaggctcagtcgaaagactgggcctttcgttttatctgttgtttgtcggtgaacgctctctactagagtcacactggctcaccttcgggtgggcctttctgcgtttatacacagctaacaccacgtcgtccctatctgctgccctaggtctatgagtggttgctggataactctttctgacaccttactatcttacaaatgtaacaaaaaagttatttttctgtaattcgagcatgtcatgttaccccgcgagcataaaacgcgtatattcagggagaccacaacggtttccctctacaaataattttgtttaactttgaattcaaaagatctggtaccacctcgagttccccgcgccagcggggataaaccgtattgaccaattcattcgggacagttattagttcgagttccccgcgccagcggggataaaccgttaccattctgttgcttttatgtataagaatcgagttccccgcgccagcggggataaaccgaaaaaaaaaccccgcccctgacagggcggggttttttttcctagggatatattccgcttcctcgctcactgactcgctacgctcggtcgttcgactgcggcgagcggaaatggcttacgaacggggcggagatttcctggaagatgccaggaagatacttaacagggaagtgagagggccgcggcaaagccgtttttccataggctccgcccccctgacaagcatcacgaaatctgacgctcaaatcagtggtggcgaaacccgacaggactataaagataccaggcgtttccccctggcggctccctcgtgcgctctcctgttcctgcctttcggtttaccggtgtcattccgctgttatggccgcgtttgtctcattccacgcctgacactcagttccgggtaggcagttcgctccaagctggactgtatgcacgaaccccccgttcagtccgaccgctgcgccttatccggtaactatcgtcttgagtccaacccggaaagacatgcaaaagcaccactggcagcagccactggtaattgatttagaggagttagtcttgaagtcatgcgccggttaaggctaaactgaaaggacaagttttggtgactgcgctcctccaagccagttacctcggttcaaagagttggtagctcagagaaccttcgaaaaaccgccctgcaaggcggttttttcgttttcagagcaagagattacgcgcagaccaaaacgatctcaagaagatcatcttattaatcagataaaatatttctagatttcagtgcaatttatctcttcaaatgtagcacctgaagtcagccccatacgatataagttgttactagtgcttggattctcaccaataaaaaacgcccggcggcaaccgagcgttctgaacaaatccagatggagttctgaggtcattactggatctatcaacaggagtccaagcgagctcgatatcaaattacgccccgccctgccactcatcgcagtactgttgtaattcattaagcattctgccgacatggaagccatcacaaacggcatgatgaacctgaatcgccagcggcatcagcaccttgtcgccttgcgtataatatttgcccatggtgaaaacgggggcgaagaagttgtccatattggccacgtttaaatcaaaactggtgaaactcacccagggattggctgagacgaaaaacatattctcaataaaccctttagggaaataggccaggttttcaccgtaacacgccacatcttgcgaatatatgtgtagaaactgccggaaatcgtcgtggtattcactccagagcgatgaaaacgtttcagtttgctcatggaaaacggtgtaacaagggtgaacactatcccatatcaccagctcaccgtctttcattgccatacgaaattccggatgagcattcatcaggcgggcaagaatgtgaataaaggccggataaaacttgtgcttatttttctttacggtctttaaaaaggccgtaatatccagctgaacggtctggttataggtacattgagcaactgactgaaatgcctcaaaatgttctttacgatgccattgggatatatcaacggtggtatatccagtgatttttttctccattttagcttccttagctcctgaaaatctcgataactcaaaaaatacgcccggtagtgatcttatttcattatggtgaaagttggaacctcttacgtgccgatcaacgtctcattttcgccagatatc

SEQ ID NO: 20 - DNA, 2902 bp, Artificial Sequence
  pCASCADE-fabI-udhA Plasmid
gacgtcttaagacccactttcacatttaagttgtttttctaatccgcatatgatcaattcaaggccgaataagaaggctggctctgcaccttggtgatcaaataattcgatagcttgtcgtaataatggcggcatactatcagtagtaggtgtttccctttcttctttagcgacttgatgctcttgatcttccaatacgcaacctaaagtaaaatgccccacagcgctgagtgcatataatgcattctctagtgaaaaaccttgttggcataaaaaggctaattgattttcgagagtttcatactgtttttctgtaggccgtgtacctaaatgtacttttgctccatcgcgatgacttagtaaagcacatctaaaacttttagcgttattacgtaaaaaatcttgccagctttccccttctaaagggcaaaagtgagtatggtgcctatctaacatctcaatggctaaggcgtcgagcaaagcccgcttattttttacatgccaatacaatgtaggctgctctacacctagcttctgggcgagtttacgggttgttaaaccttcgattccgacctcattaagcagctctaatgcgctgttaatcactttacttttatctaatctagacatcatccaggcatcaaataaaacgaaaggctcagtcgaaagactgggcctttcgttttatctgttgtttgtcggtgaacgctctctactagagtcacactggctcaccttcgggtgggcctttctgcgtttatacacagctaacaccacgtcgtccctatctgctgccctaggtctatgagtggttgctggataactctttctgacaccttactatcttacaaatgtaacaaaaaagttatttttctgtaattcgagcatgtcatgttaccccgcgagcataaaacgcgtatattcagggagaccacaacggtttccctctacaaataattttgtttaactttgaattcaaaagatctggtaccacctcgagttccccgcgccagcggggataaaccgttgattataataaccgtttatctgttcgtatcgagttccccgcgccagcggggataaaccgttaccattctgttgcttttatgtataagaatcgagttccccgcgccagcggggataaaccgaaaaaaaaaccccgcccctgacagggcggggttttttttcctagggatatattccgcttcctcgctcactgactcgctacgctcggtcgttcgactgcggcgagcggaaatggcttacgaacggggcggagatttcctggaagatgccaggaagatacttaacagggaagtgagagggccgcggcaaagccgtttttccataggctccgcccccctgacaagcatcacgaaatctgacgctcaaatcagtggtggcgaaacccgacaggactataaagataccaggcgtttccccctggcggctccctcgtgcgctctcctgttcctgcctttcggtttaccggtgtcattccgctgttatggccgcgtttgtctcattccacgcctgacactcagttccgggtaggcagttcgctccaagctggactgtatgcacgaaccccccgttcagtccgaccgctgcgccttatccggtaactatcgtcttgagtccaacccggaaagacatgcaaaagcaccactggcagcagccactggtaattgatttagaggagttagtcttgaagtcatgcgccggttaaggctaaactgaaaggacaagttttggtgactgcgctcctccaagccagttacctcggttcaaagagttggtagctcagagaaccttcgaaaaaccgccctgcaaggcggttttttcgttttcagagcaagagattacgcgcagaccaaaacgatctcaagaagatcatcttattaatcagataaaatatttctagatttcagtgcaatttatctcttcaaatgtagcacctgaagtcagccccatacgatataagttgttactagtgcttggattctcaccaataaaaaacgcccggcggcaaccgagcgttctgaacaaatccagatggagttctgaggtcattactggatctatcaacaggagtccaagcgagctcgatatcaaattacgccccgccctgccactcatcgcagtactgttgtaattcattaagcattctgccgacatggaagccatcacaaacggcatgatgaacctgaatcgccagcggcatcagcaccttgtcgccttgcgtataatatttgcccatggtgaaaacgggggcgaagaagttgtccatattggccacgtttaaatcaaaactggtgaaactcacccagggattggctgagacgaaaaacatattctcaataaaccctttagggaaataggccaggttttcaccgtaacacgccacatcttgcgaatatatgtgtagaaactgccggaaatcgtcgtggtattcactccagagcgatgaaaacgtttcagtttgctcatggaaaacggtgtaacaagggtgaacactatcccatatcaccagctcaccgtctttcattgccatacgaaattccggatgagcattcatcaggcgggcaagaatgtgaataaaggccggataaaacttgtgcttatttttctttacggtctttaaaaaggccgtaatatccagctgaacggtctggttataggtacattgagcaactgactgaaatgcctcaaaatgttctttacgatgccattgggatatatcaacggtggtatatccagtgatttttttctccattttagcttccttagctcctgaaaatctcgataactcaaaaaatacgcccggtagtgatcttatttcattatggtgaaagttggaacctcttacgtgccgatcaacgtctcattttcgccagatatc

SEQ ID NO: 21 - DNA, 2903 bp, Artificial Sequence
  pCASCADE-fabI-gltA1 Plasmid
gacgtcttaagacccactttcacatttaagttgtttttctaatccgcatatgatcaattcaaggccgaataagaaggctggctctgcaccttggtgatcaaataattcgatagcttgtcgtaataatggcggcatactatcagtagtaggtgtttccctttcttctttagcgacttgatgctcttgatcttccaatacgcaacctaaagtaaaatgccccacagcgctgagtgcatataatgcattctctagtgaaaaaccttgttggcataaaaaggctaattgattttcgagagtttcatactgtttttctgtaggccgtgtacctaaatgtacttttgctccatcgcgatgacttagtaaagcacatctaaaacttttagcgttattacgtaaaaaatcttgccagctttccccttctaaagggcaaaagtgagtatggtgcctatctaacatctcaatggctaaggcgtcgagcaaagcccgcttattttttacatgccaatacaatgtaggctgctctacacctagcttctgggcgagtttacgggttgttaaaccttcgattccgacctcattaagcagctctaatgcgctgttaatcactttacttttatctaatctagacatcatccaggcatcaaataaaacgaaaggctcagtcgaaagactgggcctttcgttttatctgttgtttgtcggtgaacgctctctactagagtcacactggctcaccttcgggtgggcctttctgcgtttatacacagctaacaccacgtcgtccctatctgctgccctaggtctatgagtggttgctggataactctttctgacaccttactatcttacaaatgtaacaaaaaagttatttttctgtaattcgagcatgtcatgttaccccgcgagcataaaacgcgtatattcagggagaccacaacggtttccctctacaaataattttgtttaactttgaattcaaaagatctggtaccacctcgagttccccgcgccagcggggataaaccgttgattataataaccgtttatctgttcgtatcgagttccccgcgccagcggggataaaccgaaaagcatataatgcgtaaaagttatgaagttcgagttccccgcgccagcggggataaaccgaaaaaaaaaccccgcccctgacagggcggggttttttttcctagggatatattccgcttcctcgctcactgactcgctacgctcggtcgttcgactgcggcgagcggaaatggcttacgaacggggcggagatttcctggaagatgccaggaagatacttaacagggaagtgagagggccgcggcaaagccgtttttccataggctccgcccccctgacaagcatcacgaaatctgacgctcaaatcagtggtggcgaaacccgacaggactataaagataccaggcgtttccccctggcggctccctcgtgcgctctcctgttcctgcctttcggtttaccggtgtcattccgctgttatggccgcgtttgtctcattccacgcctgacactcagttccgggtaggcagttcgctccaagctggactgtatgcacgaaccccccgttcagtccgaccgctgcgccttatccggtaactatcgtcttgagtccaacccggaaagacatgcaaaagcaccactggcagcagccactggtaattgatttagaggagttagtcttgaagtcatgcgccggttaaggctaaactgaaaggacaagttttggtgactgcgctcctccaagccagttacctcggttcaaagagttggtagctcagagaaccttcgaaaaaccgccctgcaaggcggttttttcgttttcagagcaagagattacgcgcagaccaaaacgatctcaagaagatcatcttattaatcagataaaatatttctagatttcagtgcaatttatctcttcaaatgtagcacctgaagtcagccccatacgatataagttgttactagtgcttggattctcaccaataaaaaacgcccggcggcaaccgagcgttctgaacaaatccagatggagttctgaggtcattactggatctatcaacaggagtccaagcgagctcgatatcaaattacgccccgccctgccactcatcgcagtactgttgtaattcattaagcattctgccgacatggaagccatcacaaacggcatgatgaacctgaatcgccagcggcatcagcaccttgtcgccttgcgtataatatttgcccatggtgaaaacgggggcgaagaagttgtccatattggccacgtttaaatcaaaactggtgaaactcacccagggattggctgagacgaaaaacatattctcaataaaccctttagggaaataggccaggttttcaccgtaacacgccacatcttgcgaatatatgtgtagaaactgccggaaatcgtcgtggtattcactccagagcgatgaaaacgtttcagtttgctcatggaaaacggtgtaacaagggtgaacactatcccatatcaccagctcaccgtctttcattgccatacgaaattccggatgagcattcatcaggcgggcaagaatgtgaataaaggccggataaaacttgtgcttatttttctttacggtctttaaaaaggccgtaatatccagctgaacggtctggttataggtacattgagcaactgactgaaatgcctcaaaatgttctttacgatgccattgggatatatcaacggtggtatatccagtgatttttttctccattttagcttccttagctcctgaaaatctcgataactcaaaaaatacgcccggtagtgatcttatttcattatggtgaaagttggaacctcttacgtgccgatcaacgtctcattttcgccagatatc

SEQ ID NO: 22 - DNA, 2904 bp, Artificial Sequence
  pCASCADE-fabI-gltA2 Plasmid
gacgtcttaagacccactttcacatttaagttgtttttctaatccgcatatgatcaattcaaggccgaataagaaggctggctctgcaccttggtgatcaaataattcgatagcttgtcgtaataatggcggcatactatcagtagtaggtgtttccctttcttctttagcgacttgatgctcttgatcttccaatacgcaacctaaagtaaaatgccccacagcgctgagtgcatataatgcattctctagtgaaaaaccttgttggcataaaaaggctaattgattttcgagagtttcatactgtttttctgtaggccgtgtacctaaatgtacttttgctccatcgcgatgacttagtaaagcacatctaaaacttttagcgttattacgtaaaaaatcttgccagctttccccttctaaagggcaaaagtgagtatggtgcctatctaacatctcaatggctaaggcgtcgagcaaagcccgcttattttttacatgccaatacaatgtaggctgctctacacctagcttctgggcgagtttacgggttgttaaaccttcgattccgacctcattaagcagctctaatgcgctgttaatcactttacttttatctaatctagacatcatccaggcatcaaataaaacgaaaggctcagtcgaaagactgggcctttcgttttatctgttgtttgtcggtgaacgctctctactagagtcacactggctcaccttcgggtgggcctttctgcgtttatacacagctaacaccacgtcgtccctatctgctgccctaggtctatgagtggttgctggataactctttctgacaccttactatcttacaaatgtaacaaaaaagttatttttctgtaattcgagcatgtcatgttaccccgcgagcataaaacgcgtatattcagggagaccacaacggtttccctctacaaataattttgtttaactttgaattcaaaagatctggtaccacctcgagttccccgcgccagcggggataaaccgttgattataataaccgtttatctgttcgtatcgagttccccgcgccagcggggataaaccgtattgaccaattcattcgggacagttattagttcgagttccccgcgccagcggggataaaccgaaaaaaaaaccccgcccctgacagggcggggttttttttcctagggatatattccgcttcctcgctcactgactcgctacgctcggtcgttcgactgcggcgagcggaaatggcttacgaacggggcggagatttcctggaagatgccaggaagatacttaacagggaagtgagagggccgcggcaaagccgtttttccataggctccgcccccctgacaagcatcacgaaatctgacgctcaaatcagtggtggcgaaacccgacaggactataaagataccaggcgtttccccctggcggctccctcgtgcgctctcctgttcctgcctttcggtttaccggtgtcattccgctgttatggccgcgtttgtctcattccacgcctgacactcagttccgggtaggcagttcgctccaagctggactgtatgcacgaaccccccgttcagtccgaccgctgcgccttatccggtaactatcgtcttgagtccaacccggaaagacatgcaaaagcaccactggcagcagccactggtaattgatttagaggagttagtcttgaagtcatgcgccggttaaggctaaactgaaaggacaagttttggtgactgcgctcctccaagccagttacctcggttcaaagagttggtagctcagagaaccttcgaaaaaccgccctgcaaggcggttttttcgttttcagagcaagagattacgcgcagaccaaaacgatctcaagaagatcatcttattaatcagataaaatatttctagatttcagtgcaatttatctcttcaaatgtagcacctgaagtcagccccatacgatataagttgttactagtgcttggattctcaccaataaaaaacgcccggcggcaaccgagcgttctgaacaaatccagatggagttctgaggtcattactggatctatcaacaggagtccaagcgagctcgatatcaaattacgccccgccctgccactcatcgcagtactgttgtaattcattaagcattctgccgacatggaagccatcacaaacggcatgatgaacctgaatcgccagcggcatcagcaccttgtcgccttgcgtataatatttgcccatggtgaaaacgggggcgaagaagttgtccatattggccacgtttaaatcaaaactggtgaaactcacccagggattggctgagacgaaaaacatattctcaataaaccctttagggaaataggccaggttttcaccgtaacacgccacatcttgcgaatatatgtgtagaaactgccggaaatcgtcgtggtattcactccagagcgatgaaaacgtttcagtttgctcatggaaaacggtgtaacaagggtgaacactatcccatatcaccagctcaccgtctttcattgccatacgaaattccggatgagcattcatcaggcgggcaagaatgtgaataaaggccggataaaacttgtgcttatttttctttacggtctttaaaaaggccgtaatatccagctgaacggtctggttataggtacattgagcaactgactgaaatgcctcaaaatgttctttacgatgccattgggatatatcaacggtggtatatccagtgatttttttctccattttagcttccttagctcctgaaaatctcgataactcaaaaaatacgcccggtagtgatcttatttcattatggtgaaagttggaacctcttacgtgccgatcaacgtctcattttcgccagatatc

SEQ ID NO: 23 - DNA, 2902 bp, Artificial Sequence
  pCASCADE-fabI-zwf Plasmid
gacgtcttaagacccactttcacatttaagttgtttttctaatccgcatatgatcaattcaaggccgaataagaaggctggctctgcaccttggtgatcaaataattcgatagcttgtcgtaataatggcggcatactatcagtagtaggtgtttccctttcttctttagcgacttgatgctcttgatcttccaatacgcaacctaaagtaaaatgccccacagcgctgagtgcatataatgcattctctagtgaaaaaccttgttggcataaaaaggctaattgattttcgagagtttcatactgtttttctgtaggccgtgtacctaaatgtacttttgctccatcgcgatgacttagtaaagcacatctaaaacttttagcgttattacgtaaaaaatcttgccagctttccccttctaaagggcaaaagtgagtatggtgcctatctaacatctcaatggctaaggcgtcgagcaaagcccgcttattttttacatgccaatacaatgtaggctgctctacacctagcttctgggcgagtttacgggttgttaaaccttcgattccgacctcattaagcagctctaatgcgctgttaatcactttacttttatctaatctagacatcatccaggcatcaaataaaacgaaaggctcagtcgaaagactgggcctttcgttttatctgttgtttgtcggtgaacgctctctactagagtcacactggctcaccttcgggtgggcctttctgcgtttatacacagctaacaccacgtcgtccctatctgctgccctaggtctatgagtggttgctggataactctttctgacaccttactatcttacaaatgtaacaaaaaagttatttttctgtaattcgagcatgtcatgttaccccgcgagcataaaacgcgtatattcagggagaccacaacggtttccctctacaaataattttgtttaactttgaattcaaaagatctggtaccacctcgagttccccgcgccagcggggataaaccgttgattataataaccgtttatctgttcgtatcgagttccccgcgccagcggggataaaccgctcgtaaaagcagtacagtgcaccgtaagatcgagttccccgcgccagcggggataaaccgaaaaaaaaaccccgcccctgacagggcggggttttttttcctagggatatattccgcttcctcgctcactgactcgctacgctcggtcgttcgactgcggcgagcggaaatggcttacgaacggggcggagatttcctggaagatgccaggaagatacttaacagggaagtgagagggccgcggcaaagccgtttttccataggctccgcccccctgacaagcatcacgaaatctgacgctcaaatcagtggtggcgaaacccgacaggactataaagataccaggcgtttccccctggcggctccctcgtgcgctctcctgttcctgcctttcggtttaccggtgtcattccgctgttatggccgcgtttgtctcattccacgcctgacactcagttccgggtaggcagttcgctccaagctggactgtatgcacgaaccccccgttcagtccgaccgctgcgccttatccggtaactatcgtcttgagtccaacccggaaagacatgcaaaagcaccactggcagcagccactggtaattgatttagaggagttagtcttgaagtcatgcgccggttaaggctaaactgaaaggacaagttttggtgactgcgctcctccaagccagttacctcggttcaaagagttggtagctcagagaaccttcgaaaaaccgccctgcaaggcggttttttcgttttcagagcaagagattacgcgcagaccaaaacgatctcaagaagatcatcttattaatcagataaaatatttctagatttcagtgcaatttatctcttcaaatgtagcacctgaagtcagccccatacgatataagttgttactagtgcttggattctcaccaataaaaaacgcccggcggcaaccgagcgttctgaacaaatccagatggagttctgaggtcattactggatctatcaacaggagtccaagcgagctcgatatcaaattacgccccgccctgccactcatcgcagtactgttgtaattcattaagcattctgccgacatggaagccatcacaaacggcatgatgaacctgaatcgccagcggcatcagcaccttgtcgccttgcgtataatatttgcccatggtgaaaacgggggcgaagaagttgtccatattggccacgtttaaatcaaaactggtgaaactcacccagggattggctgagacgaaaaacatattctcaataaaccctttagggaaataggccaggttttcaccgtaacacgccacatcttgcgaatatatgtgtagaaactgccggaaatcgtcgtggtattcactccagagcgatgaaaacgtttcagtttgctcatggaaaacggtgtaacaagggtgaacactatcccatatcaccagctcaccgtctttcattgccatacgaaattccggatgagcattcatcaggcgggcaagaatgtgaataaaggccggataaaacttgtgcttatttttctttacggtctttaaaaaggccgtaatatccagctgaacggtctggttataggtacattgagcaactgactgaaatgcctcaaaatgttctttacgatgccattgggatatatcaacggtggtatatccagtgatttttttctccattttagcttccttagctcctgaaaatctcgataactcaaaaaatacgcccggtagtgatcttatttcattatggtgaaagttggaacctcttacgtgccgatcaacgtctcattttcgccagatatc

SEQ ID NO: 24 - DNA, 2903 bp, Artificial Sequence
  pCASCADE-gltA1-udhA Plasmid
gacgtcttaagacccactttcacatttaagttgtttttctaatccgcatatgatcaattcaaggccgaataagaaggctggctctgcaccttggtgatcaaataattcgatagcttgtcgtaataatggcggcatactatcagtagtaggtgtttccctttcttctttagcgacttgatgctcttgatcttccaatacgcaacctaaagtaaaatgccccacagcgctgagtgcatataatgcattctctagtgaaaaaccttgttggcataaaaaggctaattgattttcgagagtttcatactgtttttctgtaggccgtgtacctaaatgtacttttgctccatcgcgatgacttagtaaagcacatctaaaacttttagcgttattacgtaaaaaatcttgccagctttccccttctaaagggcaaaagtgagtatggtgcctatctaacatctcaatggctaaggcgtcgagcaaagcccgcttattttttacatgccaatacaatgtaggctgctctacacctagcttctgggcgagtttacgggttgttaaaccttcgattccgacctcattaagcagctctaatgcgctgttaatcactttacttttatctaatctagacatcatccaggcatcaaataaaacgaaaggctcagtcgaaagactgggcctttcgttttatctgttgtttgtcggtgaacgctctctactagagtcacactggctcaccttcgggtgggcctttctgcgtttatacacagctaacaccacgtcgtccctatctgctgccctaggtctatgagtggttgctggataactctttctgacaccttactatcttacaaatgtaacaaaaaagttatttttctgtaattcgagcatgtcatgttaccccgcgagcataaaacgcgtatattcagggagaccacaacggtttccctctacaaataattttgtttaactttgaattcaaaagatctggtaccacctcgagttccccgcgccagcggggataaaccgaaaagcatataatgcgtaaaagttatgaagttcgagttccccgcgccagcggggataaaccgttaccattctgttgcttttatgtataagaatcgagttccccgcgccagcggggataaaccgaaaaaaaaaccccgcccctgacagggcggggttttttttcctagggatatattccgcttcctcgctcactgactcgctacgctcggtcgttcgactgcggcgagcggaaatggcttacgaacggggcggagatttcctggaagatgccaggaagatacttaacagggaagtgagagggccgcggcaaagccgtttttccataggctccgcccccctgacaagcatcacgaaatctgacgctcaaatcagtggtggcgaaacccgacaggactataaagataccaggcgtttccccctggcggctccctcgtgcgctctcctgttcctgcctttcggtttaccggtgtcattccgctgttatggccgcgtttgtctcattccacgcctgacactcagttccgggtaggcagttcgctccaagctggactgtatgcacgaaccccccgttcagtccgaccgctgcgccttatccggtaactatcgtcttgagtccaacccggaaagacatgcaaaagcaccactggcagcagccactggtaattgatttagaggagttagtcttgaagtcatgcgccggttaaggctaaactgaaaggacaagttttggtgactgcgctcctccaagccagttacctcggttcaaagagttggtagctcagagaaccttcgaaaaaccgccctgcaaggcggttttttcgttttcagagcaagagattacgcgcagaccaaaacgatctcaagaagatcatcttattaatcagataaaatatttctagatttcagtgcaatttatctcttcaaatgtagcacctgaagtcagccccatacgatataagttgttactagtgcttggattctcaccaataaaaaacgcccggcggcaaccgagcgttctgaacaaatccagatggagttctgaggtcattactggatctatcaacaggagtccaagcgagctcgatatcaaattacgccccgccctgccactcatcgcagtactgttgtaattcattaagcattctgccgacatggaagccatcacaaacggcatgatgaacctgaatcgccagcggcatcagcaccttgtcgccttgcgtataatatttgcccatggtgaaaacgggggcgaagaagttgtccatattggccacgtttaaatcaaaactggtgaaactcacccagggattggctgagacgaaaaacatattctcaataaaccctttagggaaataggccaggttttcaccgtaacacgccacatcttgcgaatatatgtgtagaaactgccggaaatcgtcgtggtattcactccagagcgatgaaaacgtttcagtttgctcatggaaaacggtgtaacaagggtgaacactatcccatatcaccagctcaccgtctttcattgccatacgaaattccggatgagcattcatcaggcgggcaagaatgtgaataaaggccggataaaacttgtgcttatttttctttacggtctttaaaaaggccgtaatatccagctgaacggtctggttataggtacattgagcaactgactgaaatgcctcaaaatgttctttacgatgccattgggatatatcaacggtggtatatccagtgatttttttctccattttagcttccttagctcctgaaaatctcgataactcaaaaaatacgcccggtagtgatcttatttcattatggtgaaagttggaacctcttacgtgccgatcaacgtctcattttcgccagatatc

SEQ ID NO: 25 - DNA, 2904 bp, Artificial Sequence
  pCASCADE-gltA2-udhA Plasmid
gacgtcttaagacccactttcacatttaagttgtttttctaatccgcatatgatcaattcaaggccgaataagaaggctggctctgcaccttggtgatcaaataattcgatagcttgtcgtaataatggcggcatactatcagtagtaggtgtttccctttcttctttagcgacttgatgctcttgatcttccaatacgcaacctaaagtaaaatgccccacagcgctgagtgcatataatgcattctctagtgaaaaaccttgttggcataaaaaggctaattgattttcgagagtttcatactgtttttctgtaggccgtgtacctaaatgtacttttgctccatcgcgatgacttagtaaagcacatctaaaacttttagcgttattacgtaaaaaatcttgccagctttccccttctaaagggcaaaagtgagtatggtgcctatctaacatctcaatggctaaggcgtcgagcaaagcccgcttattttttacatgccaatacaatgtaggctgctctacacctagcttctgggcgagtttacgggttgttaaaccttcgattccgacctcattaagcagctctaatgcgctgttaatcactttacttttatctaatctagacatcatccaggcatcaaataaaacgaaaggctcagtcgaaagactgggcctttcgttttatctgttgtttgtcggtgaacgctctctactagagtcacactggctcaccttcgggtgggcctttctgcgtttatacacagctaacaccacgtcgtccctatctgctgccctaggtctatgagtggttgctggataactctttctgacaccttactatcttacaaatgtaacaaaaaagttatttttctgtaattcgagcatgtcatgttaccccgcgagcataaaacgcgtatattcagggagaccacaacggtttccctctacaaataattttgtttaactttgaattcaaaagatctggtaccacctcgagttccccgcgccagcggggataaaccgtattgaccaattcattcgggacagttattagttcgagttccccgcgccagcggggataaaccgttaccattctgttgcttttatgtataagaatcgagttccccgcgccagcggggataaaccgaaaaaaaaaccccgcccctgacagggcggggttttttttcctagggatatattccgcttcctcgctcactgactcgctacgctcggtcgttcgactgcggcgagcggaaatggcttacgaacggggcggagatttcctggaagatgccaggaagatacttaacagggaagtgagagggccgcggcaaagccgtttttccataggctccgcccccctgacaagcatcacgaaatctgacgctcaaatcagtggtggcgaaacccgacaggactataaagataccaggcgtttccccctggcggctccctcgtgcgctctcctgttcctgcctttcggtttaccggtgtcattccgctgttatggccgcgtttgtctcattccacgcctgacactcagttccgggtaggcagttcgctccaagctggactgtatgcacgaaccccccgttcagtccgaccgctgcgccttatccggtaactatcgtcttgagtccaacccggaaagacatgcaaaagcaccactggcagcagccactggtaattgatttagaggagttagtcttgaagtcatgcgccggttaaggctaaactgaaaggacaagttttggtgactgcgctcctccaagccagttacctcggttcaaagagttggtagctcagagaaccttcgaaaaaccgccctgcaaggcggttttttcgttttcagagcaagagattacgcgcagaccaaaacgatctcaagaagatcatcttattaatcagataaaatatttctagatttcagtgcaatttatctcttcaaatgtagcacctgaagtcagccccatacgatataagttgttactagtgcttggattctcaccaataaaaaacgcccggcggcaaccgagcgttctgaacaaatccagatggagttctgaggtcattactggatctatcaacaggagtccaagcgagctcgatatcaaattacgccccgccctgccactcatcgcagtactgttgtaattcattaagcattctgccgacatggaagccatcacaaacggcatgatgaacctgaatcgccagcggcatcagcaccttgtcgccttgcgtataatatttgcccatggtgaaaacgggggcgaagaagttgtccatattggccacgtttaaatcaaaactggtgaaactcacccagggattggctgagacgaaaaacatattctcaataaaccctttagggaaataggccaggttttcaccgtaacacgccacatcttgcgaatatatgtgtagaaactgccggaaatcgtcgtggtattcactccagagcgatgaaaacgtttcagtttgctcatggaaaacggtgtaacaagggtgaacactatcccatatcaccagctcaccgtctttcattgccatacgaaattccggatgagcattcatcaggcgggcaagaatgtgaataaaggccggataaaacttgtgcttatttttctttacggtctttaaaaaggccgtaatatccagctgaacggtctggttataggtacattgagcaactgactgaaatgcctcaaaatgttctttacgatgccattgggatatatcaacggtggtatatccagtgatttttttctccattttagcttccttagctcctgaaaatctcgataactcaaaaaatacgcccggtagtgatcttatttcattatggtgaaagttggaacctcttacgtgccgatcaacgtctcattttcgccagatatc

SEQ ID NO: 26 - DNA, 2903 bp, Artificial Sequence
  pCASCADE-gltA1-zwf Plasmid
gacgtcttaagacccactttcacatttaagttgtttttctaatccgcatatgatcaattcaaggccgaataagaaggctggctctgcaccttggtgatcaaataattcgatagcttgtcgtaataatggcggcatactatcagtagtaggtgtttccctttcttctttagcgacttgatgctcttgatcttccaatacgcaacctaaagtaaaatgccccacagcgctgagtgcatataatgcattctctagtgaaaaaccttgttggcataaaaaggctaattgattttcgagagtttcatactgtttttctgtaggccgtgtacctaaatgtacttttgctccatcgcgatgacttagtaaagcacatctaaaacttttagcgttattacgtaaaaaatcttgccagctttccccttctaaagggcaaaagtgagtatggtgcctatctaacatctcaatggctaaggcgtcgagcaaagcccgcttattttttacatgccaatacaatgtaggctgctctacacctagcttctgggcgagtttacgggttgttaaaccttcgattccgacctcattaagcagctctaatgcgctgttaatcactttacttttatctaatctagacatcatccaggcatcaaataaaacgaaaggctcagtcgaaagactgggcctttcgttttatctgttgtttgtcggtgaacgctctctactagagtcacactggctcaccttcgggtgggcctttctgcgtttatacacagctaacaccacgtcgtccctatctgctgccctaggtctatgagtggttgctggataactctttctgacaccttactatcttacaaatgtaacaaaaaagttatttttctgtaattcgagcatgtcatgttaccccgcgagcataaaacgcgtatattcagggagaccacaacggtttccctctacaaataattttgtttaactttgaattcaaaagatctggtaccacctcgagttccccgcgccagcggggataaaccgaaaagcatataatgcgtaaaagttatgaagttcgagttccccgcgccagcggggataaaccgctcgtaaaagcagtacagtgcaccgtaagatcgagttccccgcgccagcggggataaaccgaaaaaaaaaccccgcccctgacagggcggggttttttttcctagggatatattccgcttcctcgctcactgactcgctacgctcggtcgttcgactgcggcgagcggaaatggcttacgaacggggcggagatttcctggaagatgccaggaagatacttaacagggaagtgagagggccgcggcaaagccgtttttccataggctccgcccccctgacaagcatcacgaaatctgacgctcaaatcagtggtggcgaaacccgacaggactataaagataccaggcgtttccccctggcggctccctcgtgcgctctcctgttcctgcctttcggtttaccggtgtcattccgctgttatggccgcgtttgtctcattccacgcctgacactcagttccgggtaggcagttcgctccaagctggactgtatgcacgaaccccccgttcagtccgaccgctgcgccttatccggtaactatcgtcttgagtccaacccggaaagacatgcaaaagcaccactggcagcagccactggtaattgatttagaggagttagtcttgaagtcatgcgccggttaaggctaaactgaaaggacaagttttggtgactgcgctcctccaagccagttacctcggttcaaagagttggtagctcagagaaccttcgaaaaaccgccctgcaaggcggttttttcgttttcagagcaagagattacgcgcagaccaaaacgatctcaagaagatcatcttattaatcagataaaatatttctagatttcagtgcaatttatctcttcaaatgtagcacctgaagtcagccccatacgatataagttgttactagtgcttggattctcaccaataaaaaacgcccggcggcaaccgagcgttctgaacaaatccagatggagttctgaggtcattactggatctatcaacaggagtccaagcgagctcgatatcaaattacgccccgccctgccactcatcgcagtactgttgtaattcattaagcattctgccgacatggaagccatcacaaacggcatgatgaacctgaatcgccagcggcatcagcaccttgtcgccttgcgtataatatttgcccatggtgaaaacgggggcgaagaagttgtccatattggccacgtttaaatcaaaactggtgaaactcacccagggattggctgagacgaaaaacatattctcaataaaccctttagggaaataggccaggttttcaccgtaacacgccacatcttgcgaatatatgtgtagaaactgccggaaatcgtcgtggtattcactccagagcgatgaaaacgtttcagtttgctcatggaaaacggtgtaacaagggtgaacactatcccatatcaccagctcaccgtctttcattgccatacgaaattccggatgagcattcatcaggcgggcaagaatgtgaataaaggccggataaaacttgtgcttatttttctttacggtctttaaaaaggccgtaatatccagctgaacggtctggttataggtacattgagcaactgactgaaatgcctcaaaatgttctttacgatgccattgggatatatcaacggtggtatatccagtgatttttttctccattttagcttccttagctcctgaaaatctcgataactcaaaaaatacgcccggtagtgatcttatttcattatggtgaaagttggaacctcttacgtgccgatcaacgtctcattttcgccagatatc

SEQ ID NO: 27 - DNA, 2904 bp, Artificial Sequence
  pCASCADE-gltA2-zwf Plasmid
gacgtcttaagacccactttcacatttaagttgtttttctaatccgcatatgatcaattcaaggccgaataagaaggctggctctgcaccttggtgatcaaataattcgatagcttgtcgtaataatggcggcatactatcagtagtaggtgtttccctttcttctttagcgacttgatgctcttgatcttccaatacgcaacctaaagtaaaatgccccacagcgctgagtgcatataatgcattctctagtgaaaaaccttgttggcataaaaaggctaattgattttcgagagtttcatactgtttttctgtaggccgtgtacctaaatgtacttttgctccatcgcgatgacttagtaaagcacatctaaaacttttagcgttattacgtaaaaaatcttgccagctttccccttctaaagggcaaaagtgagtatggtgcctatctaacatctcaatggctaaggcgtcgagcaaagcccgcttattttttacatgccaatacaatgtaggctgctctacacctagcttctgggcgagtttacgggttgttaaaccttcgattccgacctcattaagcagctctaatgcgctgttaatcactttacttttatctaatctagacatcatccaggcatcaaataaaacgaaaggctcagtcgaaagactgggcctttcgttttatctgttgtttgtcggtgaacgctctctactagagtcacactggctcaccttcgggtgggcctttctgcgtttatacacagctaacaccacgtcgtccctatctgctgccctaggtctatgagtggttgctggataactctttctgacaccttactatcttacaaatgtaacaaaaaagttatttttctgtaattcgagcatgtcatgttaccccgcgagcataaaacgcgtatattcagggagaccacaacggtttccctctacaaataattttgtttaactttgaattcaaaagatctggtaccacctcgagttccccgcgccagcggggataaaccgtattgaccaattcattcgggacagttattagttcgagttccccgcgccagcggggataaaccgctcgtaaaagcagtacagtgcaccgtaagatcgagttccccgcgccagcggggataaaccgaaaaaaaaaccccgcccctgacagggcggggttttttttcctagggatatattccgcttcctcgctcactgactcgctacgctcggtcgttcgactgcggcgagcggaaatggcttacgaacggggcggagatttcctggaagatgccaggaagatacttaacagggaagtgagagggccgcggcaaagccgtttttccataggctccgcccccctgacaagcatcacgaaatctgacgctcaaatcagtggtggcgaaacccgacaggactataaagataccaggcgtttccccctggcggctccctcgtgcgctctcctgttcctgcctttcggtttaccggtgtcattccgctgttatggccgcgtttgtctcattccacgcctgacactcagttccgggtaggcagttcgctccaagctggactgtatgcacgaaccccccgttcagtccgaccgctgcgccttatccggtaactatcgtcttgagtccaacccggaaagacatgcaaaagcaccactggcagcagccactggtaattgatttagaggagttagtcttgaagtcatgcgccggttaaggctaaactgaaaggacaagttttggtgactgcgctcctccaagccagttacctcggttcaaagagttggtagctcagagaaccttcgaaaaaccgccctgcaaggcggttttttcgttttcagagcaagagattacgcgcagaccaaaacgatctcaagaagatcatcttattaatcagataaaatatttctagatttcagtgcaatttatctcttcaaatgtagcacctgaagtcagccccatacgatataagttgttactagtgcttggattctcaccaataaaaaacgcccggcggcaaccgagcgttctgaacaaatccagatggagttctgaggtcattactggatctatcaacaggagtccaagcgagctcgatatcaaattacgccccgccctgccactcatcgcagtactgttgtaattcattaagcattctgccgacatggaagccatcacaaacggcatgatgaacctgaatcgccagcggcatcagcaccttgtcgccttgcgtataatatttgcccatggtgaaaacgggggcgaagaagttgtccatattggccacgtttaaatcaaaactggtgaaactcacccagggattggctgagacgaaaaacatattctcaataaaccctttagggaaataggccaggttttcaccgtaacacgccacatcttgcgaatatatgtgtagaaactgccggaaatcgtcgtggtattcactccagagcgatgaaaacgtttcagtttgctcatggaaaacggtgtaacaagggtgaacactatcccatatcaccagctcaccgtctttcattgccatacgaaattccggatgagcattcatcaggcgggcaagaatgtgaataaaggccggataaaacttgtgcttatttttctttacggtctttaaaaaggccgtaatatccagctgaacggtctggttataggtacattgagcaactgactgaaatgcctcaaaatgttctttacgatgccattgggatatatcaacggtggtatatccagtgatttttttctccattttagcttccttagctcctgaaaatctcgataactcaaaaaatacgcccggtagtgatcttatttcattatggtgaaagttggaacctcttacgtgccgatcaacgtctcattttcgccagatatc

SEQ ID NO: 28 - DNA, 3505 bp, Artificial Sequence
  pBT1-mCherry-DAS+4 Vector
cgcaaaaaaccccgcttcggcggggttttttcgcacgtctccatcgcttgcccaagttgtgaagcacagctaacaccacgtcgtccctatctgctgccctaggtctatgagtggttgctggataactttacgggcatgcataaggctcgtataatatattcagggagaccacaacggtttccctctacaaataattttgtttaactttgatcgcatggttgctactagagaaagaggagaaatactagatggtgagcaagggcgaggaggataacatggccatcatcaaggagttcatgcgcttcaaggtgcacatggagggctccgtgaacggccacgagttcgagatcgagggcgagggcgagggccgcccctacgagggcacccagaccgccaagctgaaggtgaccaagggtggccccctgcccttcgcctgggacatcctgtcccctcagttcatgtacggctccaaggcctacgtgaagcaccccgccgacatccccgactacttgaagctgtccttccccgagggcttcaagtgggagcgcgtgatgaacttcgaggacggcggcgtggtgaccgtgacccaggactcctccctgcaggacggcgagttcatctacaaggtgaagctgcgcggcaccaacttcccctccgacggccccgtaatgcagaagaagaccatgggctgggaggcctcctccgagcggatgtaccccgaggacggcgccctgaagggcgagatcaagcagaggctgaagctgaaggacggcggccactacgacgctgaggtcaagaccacctacaaggccaagaagcccgtgcagctgcccggcgcctacaacgtcaacatcaagttggacatcacctcccacaacgaggactacaccatcgtggaacagtacgaacgcgccgagggccgccactccaccggcggcatggacgaactgtacaaggcggccaacgatgaaaactattctgaaaactatgcggatgcgtcttaataaggacgagcctcagactccagcgtaactggactgaaaacaaactaaagcgcccttgtggcgctttagttttgttccgcggccaccggctggctcgcttcgctcggcccgtggacaaccctgctggacaagctgatggacaggctgcgcctgcccacgagcttgaccacagggattgcccaccggctacccagccttcgaccacatacccaccggctccaactgcgcggcctgcggccttgccccatcaatttttttaattttctctggggaaaagcctccggcctgcggcctgcgcgcttcgcttgccggttggacaccaagtggaaggcgggtcaaggctcgcgcagcgaccgcgcagcggcttggccttgacgcgcctggaacgacccaagcctatgcgagtgggggcagtcgaaggcgaagcccgcccgcctgccccccgagcctcacggcggcgagtgcgggggttccaagggggcagcgccaccttgggcaaggccgaaggccgcgcagtcgatcaacaagccccggaggggccactttttgccggagggggagccgcgccgaaggcgtgggggaaccccgcaggggtgcccttctttgggcaccaaagaactagatatagggcgaaatgcgaaagacttaaaaatcaacaacttaaaaaaggggggtacgcaacagctcattgcggcaccccccgcaatagctcattgcgtaggttaaagaaaatctgtaattgactgccacttttacgcaacgcataattgttgtcgcgctgccgaaaagttgcagctgattgcgcatggtgccgcaaccgtgcggcaccctaccgcatggagataagcatggccacgcagtccagagaaatcggcattcaagccaagaacaagcccggtcactgggtgcaaacggaacgcaaagcgcatgaggcgtgggccgggcttattgcgaggaaacccacggcggcaatgctgctgcatcacctcgtggcgcagatgggccaccagaacgccgtggtggtcagccagaagacactttccaagctcatcggacgttctttgcggacggtccaatacgcagtcaaggacttggtggccgagcgctggatctccgtcgtgaagctcaacggccccggcaccgtgtcggcctacgtggtcaatgaccgcgtggcgtggggccagccccgcgaccagttgcgcctgtcggtgttcagtgccgccgtggtggttgatcacgacgaccaggacgaatcgctgttggggcatggcgacctgcgccgcatcccgaccctgtatccgggcgagcagcaactaccgaccggccccggcgaggagccgcccagccagcccggcattccgggcatggaaccagacctgccagccttgaccgaaacggaggaatgggaacggcgcgggcagcagcgcctgccgatgcccgatgagccgtgttttctggacgatggcgagccgttggagccgccgacacgggtcacgctgccgcgccggtagtacgtaagaggttccaactttcaccataatgaaataagatcactaccgggcgtattttttgagttatcgagattttcaggagctaaggaagctaaaatgagtattcaacatttccgtgtcgcccttattcccttttttgcggcattttgccttcctgtttttgctcacccagaaacgctggtgaaagtaaaagatgctgaagatcagttgggtgcacgagtgggttacatcgaactggatctcaacagcggtaagatccttgagagtttacgccccgaagaacgttttccaatgatgagcacttttaaagttctgctatgtggcgcggtattatcccgtattgacgccgggcaagagcaactcggtcgccgcatacactattctcagaatgacttggttgagtactcaccagtcacagaaaagcatctcacggatggcatgacagtaagagaattatgcagtgctgccataaccatgagtgataacactgcggccaacttacttctggcaacgatcggaggaccgaaggagctaaccgcttttttgcacaacatgggggatcatgtaactcgccttgatcgttgggaaccggagctgaatgaagccataccaaacgacgagcgtgacaccacgatgcctgtagcaatggcaacaacgttgcgcaaactattaactggcgaactacttactctagcttcccggcaacaattaatagactggatggaggcggataaagttgcaggatcacttctgcgctcggccctcccggctggctggtttattgctgataaatctggagccggtgagcgtgggtctcgcggtatcattgcagcactggggccagatggtaagccctcccgcatcgtagttatctacacgacggggagtcaggcaactatggatgaacgaaatagacagatcgctgagataggtgcctcactgattaagcattggtaatgaggatccccctcaagtcaaaagcctccggtc

SEQ ID NO: 29 - DNA, 2841 bp, Artificial Sequence
  pCASCADE-proD Plasmid
gacgtcttaagacccactttcacatttaagttgtttttctaatccgcatatgatcaattcaaggccgaataagaaggctggctctgcaccttggtgatcaaataattcgatagcttgtcgtaataatggcggcatactatcagtagtaggtgtttccctttcttctttagcgacttgatgctcttgatcttccaatacgcaacctaaagtaaaatgccccacagcgctgagtgcatataatgcattctctagtgaaaaaccttgttggcataaaaaggctaattgattttcgagagtttcatactgtttttctgtaggccgtgtacctaaatgtacttttgctccatcgcgatgacttagtaaagcacatctaaaacttttagcgttattacgtaaaaaatcttgccagctttccccttctaaagggcaaaagtgagtatggtgcctatctaacatctcaatggctaaggcgtcgagcaaagcccgcttattttttacatgccaatacaatgtaggctgctctacacctagcttctgggcgagtttacgggttgttaaaccttcgattccgacctcattaagcagctctaatgcgctgttaatcactttacttttatctaatctagacatcatccaggcatcaaataaaacgaaaggctcagtcgaaagactgggcctttcgttttatctgttgtttgtcggtgaacgctctctactagagtcacactggctcaccttcgggtgggcctttctgcgtttatacacagctaacaccacgtcgtccctatctgctgccctaggtctatgagtggttgctggataactctttctgacaccttactatcttacaaatgtaacaaaaaagttatttttctgtaattcgagcatgtcatgttaccccgcgagcataaaacgcgtatattcagggagaccacaacggtttccctctacaaataattttgtttaactttgaattcaaaagatctggtaccacctcgagttccccgcgccagcggggataaaccgagtggttgctggataactttacgggcatgctcgagttccccgcgccagcggggataaaccgaaaaaaaaaccccgcccctgacagggcggggttttttttcctagggatatattccgcttcctcgctcactgactcgctacgctcggtcgttcgactgcggcgagcggaaatggcttacgaacggggcggagatttcctggaagatgccaggaagatacttaacagggaagtgagagggccgcggcaaagccgtttttccataggctccgcccccctgacaagcatcacgaaatctgacgctcaaatcagtggtggcgaaacccgacaggactataaagataccaggcgtttccccctggcggctccctcgtgcgctctcctgttcctgcctttcggtttaccggtgtcattccgctgttatggccgcgtttgtctcattccacgcctgacactcagttccgggtaggcagttcgctccaagctggactgtatgcacgaaccccccgttcagtccgaccgctgcgccttatccggtaactatcgtcttgagtccaacccggaaagacatgcaaaagcaccactggcagcagccactggtaattgatttagaggagttagtcttgaagtcatgcgccggttaaggctaaactgaaaggacaagttttggtgactgcgctcctccaagccagttacctcggttcaaagagttggtagctcagagaaccttcgaaaaaccgccctgcaaggcggttttttcgttttcagagcaagagattacgcgcagaccaaaacgatctcaagaagatcatcttattaatcagataaaatatttctagatttcagtgcaatttatctcttcaaatgtagcacctgaagtcagccccatacgatataagttgttactagtgcttggattctcaccaataaaaaacgcccggcggcaaccgagcgttctgaacaaatccagatggagttctgaggtcattactggatctatcaacaggagtccaagcgagctcgatatcaaattacgccccgccctgccactcatcgcagtactgttgtaattcattaagcattctgccgacatggaagccatcacaaacggcatgatgaacctgaatcgccagcggcatcagcaccttgtcgccttgcgtataatatttgcccatggtgaaaacgggggcgaagaagttgtccatattggccacgtttaaatcaaaactggtgaaactcacccagggattggctgagacgaaaaacatattctcaataaaccctttagggaaataggccaggttttcaccgtaacacgccacatcttgcgaatatatgtgtagaaactgccggaaatcgtcgtggtattcactccagagcgatgaaaacgtttcagtttgctcatggaaaacggtgtaacaagggtgaacactatcccatatcaccagctcaccgtctttcattgccatacgaaattccggatgagcattcatcaggcgggcaagaatgtgaataaaggccggataaaacttgtgcttatttttctttacggtctttaaaaaggccgtaatatccagctgaacggtctggttataggtacattgagcaactgactgaaatgcctcaaaatgttctttacgatgccattgggatatatcaacggtggtatatccagtgatttttttctccattttagcttccttagctcctgaaaatctcgataactcaaaaaatacgcccggtagtgatcttatttcattatggtgaaagttggaacctcttacgtgccgatcaacgtctcattttcgccagatatc

SEQ ID NO: 30 - DNA, 4866 bp, Artificial Sequence
  pSMART-3HP1 Plasmid
gtgcgtaattgtgctgatctcttatatagctgctctcattatctctctaccctgaagtgactctctcacctgtaaaaataatatctcacaggcttaatagtttcttaatacaaagcctgtaaaacgtcaggataacttcttttctggaaaaaggagatataccatggcgacgacgggggcacgtagcgctagtgttggttgggccgagagcctgatcggtctgcatttgggaaaagtggccttaatcaccggaggctcagccggcatcggcgggcagatcggccgccttttagcgctgtctggcgcgcgtgttatgctggccgctcgcgaccgtcacaaactcgaacaaatgcaggccatgattcaatccgaactggcggaagttggttataccgatgtcgaagaccgcgtgcacatcgcgccggggtgtgacgtttcctctgaagcgcagctggcagatctggttgaacgcactctgtcagcattcggtaccgtggattatctgatcaataacgcgggtattgcgggtgtcgaagagatggttatcgacatgccggtggaaggctggcgtcatacgttatttgccaaccttatctcaaattatagcctgatgcgcaaactggcccctctgatgaagaaacaggggagtggctatatcttgaacgtctcgtcgtactttggtggcgaaaaagatgcggctatcccatacccaaatcgtgccgattatgcggtttcaaaagccggtcaacgtgcaatggctgaagtgttcgcccgtttcctcggcccggagatccagattaacgctatcgccccaggcccggtggaaggtgaccgcctccgcggcacgggcgaacgtcccggcttgtttgcgcgccgcgcgcgtttgattttagaaaataagcgtttaaacgagctgcatgctgcccttattgcggctgcgcgtacagatgagcgctccatgcacgaactggtggaattactgctgccgaatgatgtagcggcactcgagcagaatcccgcagccccaacggcgttgcgcgaactcgcgcgccgttttcgcagcgaaggcgacccggccgcgtcaagctccagtgctctgctcaaccgcagcattgcggcgaagttactggcccgcctgcacaacggcggctatgttctgccggcggatatcttcgccaacctgccgaaccctccagacccgttcttcacgcgcgcgcagattgatcgcgaagcccgtaaagtgcgcgacgggattatgggaatgctgtatctgcagcgcatgcctaccgagtttgacgtagcaatggctaccgtttactatctggcggatcgcaatgtgagtggagagaccttccatccgagtggggggctgcgttacgagcgcacacctaccggcggtgagttatttggcctgccgtctcccgagcgcctggcggagttagttggaagcaccgtatatttgatcggtgaacacttaaccgaacatctgaacttgctcgcacgtgcgtatcttgaacgttacggtgcgcgtcaggttgttatgatcgtggaaacggagacaggcgcggaaaccatgcgccgcttacttcacgaccatgtcgaagcaggtcgccttatgaccattgtggcgggtgaccaaatcgaagccgccatcgaccaggcgattacgcgctacggccgtcctggtccggttgtgtgcacccccttccgcccccttccgaccgtcccgttagttggccgcaaggactccgattggagcaccgtactgagtgaagccgaatttgccgaactgtgtgaacatcaactgacacatcattttcgcgtagcgcgcaaaatcgcactttcggatggtgcctcactggctctggttacccccgaaaccacagcgacaagtaccactgaacagttcgccctggccaactttattaagacaaccctgcacgcttttacggccactatcggagttgaaagtgagcgcacggcgcagcgtatcctgattaatcaggtagacctcacccgtcgtgctcgtgcggaagaaccacgcgatccgcatgaacgtcagcaggaactggaacgtttcatcgaggcggtactgctggttacggccccattaccgccggaagcagatacccgctacgctggccgcatccaccgtgggcgtgccattactgtctagtaagctcttcttctggaaaaaggagatataccatgatcgttttagtaactggagcaacggcaggttttggtgaatgcattactcgtcgttttattcaacaagggcataaagttatcgccactggccgtcgccaggaacggttgcaggagttaaaagacgaactgggagataatctgtatatcgcccaactggacgttcgcaaccgcgccgctattgaagagatgctggcatcgcttcctgccgagtggtgcaatattgatatcctggtaaataatgccggcctggcgttgggcatggagcctgcgcataaagccagcgttgaagactgggaaacgatgattgataccaacaacaaaggcctggtatatatgacgcgcgccgtcttaccgggtatggttgaacgtaatcatggtcatattattaacattggctcaacggcaggtagctggccgtatgccggtggtaacgtttacggtgcgacgaaagcgtttgttcgtcagtttagcctgaatctgcgtacggatctgcatggtacggcggtgcgcgtcaccgacatcgaaccgggtctggtgggtggtaccgagttttccaatgtccgctttaaaggcgatgacggtaaagcagaaaaaacctatcaaaataccgttgcattgacgccagaagatgtcagcgaagccgtctggtgggtgtcaacgctgcctgctcacgtcaatatcaataccctggaaatgatgccggttacccaaagctatgccggactgaatgtccaccgtcagtaataggatcgtcccggcttatcggtcagtttcacctgatttacgtaaaaacccgcttcggcgggtttttgcttttggaggggcagaaagatgaatgactgtccacgacgctatacccaaaagaaagacgaattctctagatatcgctcaatactgaccatttaaatcatacctgacctccatagcagaaagtcaaaagcctccgaccggaggcttttgacttgatcggcacgtaagaggttccaactttcaccataatgaaataagatcactaccgggcgtattttttgagttatcgagattttcaggagctaaggaagctaaaatgagccatattcaacgggaaacgtcttgctcgaggccgcgattaaattccaacatggatgctgatttatatgggtataaatgggctcgcgataatgtcgggcaatcaggtgcgacaatctatcgattgtatgggaagcccgatgcgccagagttgtttctgaaacatggcaaaggtagcgttgccaatgatgttacagatgagatggtcaggctaaactggctgacggaatttatgcctcttccgaccatcaagcattttatccgtactcctgatgatgcatggttactcaccactgcgatcccagggaaaacagcattccaggtattagaagaatatcctgattcaggtgaaaatattgttgatgcgctggcagtgttcctgcgccggttgcattcgattcctgtttgtaattgtccttttaacggcgatcgcgtatttcgtctcgctcaggcgcaatcacgaatgaataacggtttggttggtgcgagtgattttgatgacgagcgtaatggctggcctgttgaacaagtctggaaagaaatgcataagcttttgccattctcaccggattcagtcgtcactcatggtgatttctcacttgataaccttatttttgacgaggggaaattaataggttgtattgatgttggacgagtcggaatcgcagaccgataccaggatcttgccatcctatggaactgcctcggtgagttttctccttcattacagaaacggctttttcaaaaatatggtattgataatcctgatatgaataaattgcagtttcacttgatgctcgatgagtttttctaatgagggcccaaatgtaatcacctggctcaccttcgggtgggcctttctgcgttgctggcgtttttccataggctccgcccccctgacgagcatcacaaaaatcgatgctcaagtcagaggtggcgaaacccgacaggactataaagataccaggcgtttccccctggaagctccctcgtgcgctctcctgttccgaccctgccgcttaccggatacctgtccgcctttctcccttcgggaagcgtggcgctttctcatagctcacgctgtaggtatctcagttcggtgtaggtcgttcgctccaagctgggctgtgtgcacgaaccccccgttcagcccgaccgctgcgccttatccggtaactatcgtcttgagtccaacccggtaagacacgacttatcgccactggcagcagccactggtaacaggattagcagagcgaggtatgtaggcggtgctacagagttcttgaagtggtggcctaactacggctacactagaagaacagtatttggtatctgcgctctgctgaagccagttacctcggaaaaagagttggtagctcttgatccggcaaacaaaccaccgctggtagcggtggtttttttgtttgcaagcagcagattacgcgcagaaaaaaaggatctcaagaagatcctttgattttctaccgaagaaaggcccacccgtgaaggtgagccagtgagttgattgcagtccagttacgctggagtctgaggctcgtcctgaatgatatcaagcttgaattcgtt

SEQ ID NO: 31 - DNA, 3353 bp, Artificial Sequence
  Plasmid pSMART-F6AA82M
ccatggttgaatgactcctataacgaagttcacagctaacaccacgtcgtccctatctgctgccctaggtctatgagtggttgctggataacgtgcgtaattgtgctgatctcttatatagctgctctcattatctctctaccctgaagtgactctctcacctgtaaaaataatatctcacaggcttaatagtttcttaatacaaagcctgtaaaacgtcaggataacttctatattcagggagaccacaacggtttccctctacaaataattttgtttaactttcgacatggcaaaatccccccctcgcgacttgctcttcagctttctggaaaaaggagatataccatgaatgttacgtttgaagaacgtgcgagtctgcacggttaccgtatcggcattgcaagcttggatgccccggcttccttaaacgccttgagcctgcctatgatcgatgcgctccaagatcgtttgcgcgcttgggcggaagatgccgatatcgcttgcgttctgttacgtggtaatggcagcaaggcgttttgcgctggtggcgatgtagttcaattggccaaaaaatgcttagcaagcccaggtgaagccccggaactggccgagcgttttttcgcccgtagctatcgcttggatcattatttgcacacctaccccaaaccgttgatctgttgggcccatggtcacgtgctgggtggtggaatgggacttttacagggcgccggcatccgtattgtgacaccatcgtctcgcttagctatgccggaaatttctatcgggctgttccctgacgtgggtggctcccatttcctgagtcgcctcccgggaaaactggggttgtttttcggtcttaccgcgtctccccttaacgcacgcgacgcgctggacttaaatctggctgaccgtttcctgcttgacacgcagcaggatgcgctgatcgatggtctgattcagttaaattggcgcgagcaacctgatctgcagctgcactctcttctgaaagctctggaacagcaggctcgtagtgagctgccggccgctcagtggttgcctcgtcgtgaacgccttgatgccctcctggaccaagccacgttaccattgtcctggcaggcgctggcgtcgctcgaaaatgatgaggatgctctgttagctaaggcagctaaaacgatgctgggcggtagcccgctcaccggccatctcgtgtggggtcaaattcgtcgtgcacgccacctgtccttggcgcaggtgtttcagatggaatacggtatgtcattgaactgctgccgccatccggagttcgcggaaggcgtccgcgcccgtttgattgacaaggatcacgccccccattggcactggccggacgttaaccaggttccggaacaggtaattgcagcgcatttcgcgccattggatgatcaccctttagccgatctggcatagtaaccggcttatcggtcagtttcacctgatttacgtaaaaacccgcttcggcgggtttttgcttttggaggggcagaaagatgaatgactgtccacgacgctatacccaaaagaaagacgaattctctagatatcgctcaatactgaccatttaaatcatacctgacctccatagcagaaagtcaaaagcctccgaccggaggcttttgacttgatcggcacgtaagaggttccaactttcaccataatgaaataagatcactaccgggcgtattttttgagttatcgagattttcaggagctaaggaagctaaaatgagccatattcaacgggaaacgtcttgctcgaggccgcgattaaattccaacatggatgctgatttatatgggtataaatgggctcgcgataatgtcgggcaatcaggtgcgacaatctatcgattgtatgggaagcccgatgcgccagagttgtttctgaaacatggcaaaggtagcgttgccaatgatgttacagatgagatggtcaggctaaactggctgacggaatttatgcctcttccgaccatcaagcattttatccgtactcctgatgatgcatggttactcaccactgcgatcccagggaaaacagcattccaggtattagaagaatatcctgattcaggtgaaaatattgttgatgcgctggcagtgttcctgcgccggttgcattcgattcctgtttgtaattgtccttttaacggcgatcgcgtatttcgtctcgctcaggcgcaatcacgaatgaataacggtttggttggtgcgagtgattttgatgacgagcgtaatggctggcctgttgaacaagtctggaaagaaatgcataagcttttgccattctcaccggattcagtcgtcactcatggtgatttctcacttgataaccttatttttgacgaggggaaattaataggttgtattgatgttggacgagtcggaatcgcagaccgataccaggatcttgccatcctatggaactgcctcggtgagttttctccttcattacagaaacggctttttcaaaaatatggtattgataatcctgatatgaataaattgcagtttcacttgatgctcgatgagtttttctaatgagggcccaaatgtaatcacctggctcaccttcgggtgggcctttctgcgttgctggcgtttttccataggctccgcccccctgacgagcatcacaaaaatcgatgctcaagtcagaggtggcgaaacccgacaggactataaagataccaggcgtttccccctggaagctccctcgtgcgctctcctgttccgaccctgccgcttaccggatacctgtccgcctttctcccttcgggaagcgtggcgctttctcatagctcacgctgtaggtatctcagttcggtgtaggtcgttcgctccaagctgggctgtgtgcacgaaccccccgttcagcccgaccgctgcgccttatccggtaactatcgtcttgagtccaacccggtaagacacgacttatcgccactggcagcagccactggtaacaggattagcagagcgaggtatgtaggcggtgctacagagttcttgaagtggtggcctaactacggctacactagaagaacagtatttggtatctgcgctctgctgaagccagttacctcggaaaaagagttggtagctcttgatccggcaaacaaaccaccgctggtagcggtggtttttttgtttgcaagcagcagattacgcgcagaaaaaaaggatctcaagaagatcctttgattttctaccgaagaaaggcccacccgtgaaggtgagccagtgagttgattgcagtccagttacgctggagtctgaggctcgtcctgaatgatatcaagcttgaattcgtt

SEQ ID NO: 32 - DNA, 3424 bp, Artificial Sequence
  Plasmid pSMART-Ala1
ccaggcatcaaataaaacgaaaggctcagtcgaaagactgggcctttcgttttatctgttgtttgtcggtgaacgctctctactagagtcacactggctcaccttcgggtgggcctttctgcgtttatacacagctaacaccacgtcgtccctatctgctgccctaggtctatgagtggttgctggataactctttctgacaccttactatcttacaaatgtaacaaaaaagttatttttctgtaattcgagcatgtcatgttaccccgcgagcataaaacgcgtatattcagggagaccacaacggtttccctctacaaataattttgtttaactttggaaaaaggagatataccatgatcattggggtgccgaaggagatcaaaaataatgagaaccgcgtcgcgttgaccccgggaggtgtcagccagctgatctctaatggccatcgtgtcttagttgaaacaggcgctggcctgggttctggcttcgaaaacgaggcctacgaatctgcaggtgcggaaattattgctgatccaaaacaggtctgggatgcagagatggtcatgaaagtgaaagaaccgctcccggaagaatatgtctattttcgtaaaggtctggtgctgtttacatatctgcatctggcagctgaaccggagctcgcacaagcccttaaagataaaggtgtcacggccatcgcatacgaaactgtcagcgaagggcgcacgctgccattactgaccccgatgtcagaagtggcaggccgtatggctgcgcagatcggcgcacagtttcttgaaaaaccaaagggcgggaagggtattctcttagcaggagtgccgggcgtcagtcgtgggaaagtaactattattggtggcggcgtggtaggaacaaatgctgccaaaatggccgtcggtttgggggccgacgtaacaatcattgcgcgtaatgccgatcgccttcgtcaattagacgatatctttggccaccaaatcaaaaccctgatttcgaacccagtcaatatcgcggatgcggtggcggaagctgatttgttgatctgcgccgtgttaattccgggagcgaaagcacctacattggtgacggaagaaatggtgaaacaaatgaaaccgggttcagtcattgttgatgtggctattgatcagggtggcatcgtggaaacggtggaccatattaccactcacgaccagccgacgtatgaaaaacatggtgtcgtacactatgcggtggcgaatatgcctggtgcggtcccacgtacgagtacaatcgcactgacaaatgtcaccgtgccgtatgcgttgcaaatcgcgaacaaaggtgccgtgaaagcgctggccgacaatacggcgttacgtgccggtctgaacaccgctaacggtcacgtgacatatgaagcggtcgcgcgtgatttggggtacgaatatgtaccggcggaaaaagccttacaagacgaatcgagtgtcgctggtgcatagtaagctcttctaatacgactcactatagggccggcttatcggtcagtttcacctgatttacgtaaaaacccgcttcggcgggtttttgcttttggaggggcagaaagatgaatgactgtccacgacgctatacccaaaagaaagacgaattctctagatatcgctcaatactgaccatttaaatcatacctgacctccatagcagaaagtcaaaagcctccgaccggaggcttttgacttgatcggcacgtaagaggttccaactttcaccataatgaaataagatcactaccgggcgtattttttgagttatcgagattttcaggagctaaggaagctaaaatgagccatattcaacgggaaacgtcttgctcgaggccgcgattaaattccaacatggatgctgatttatatgggtataaatgggctcgcgataatgtcgggcaatcaggtgcgacaatctatcgattgtatgggaagcccgatgcgccagagttgtttctgaaacatggcaaaggtagcgttgccaatgatgttacagatgagatggtcaggctaaactggctgacggaatttatgcctcttccgaccatcaagcattttatccgtactcctgatgatgcatggttactcaccactgcgatcccagggaaaacagcattccaggtattagaagaatatcctgattcaggtgaaaatattgttgatgcgctggcagtgttcctgcgccggttgcattcgattcctgtttgtaattgtccttttaacggcgatcgcgtatttcgtctcgctcaggcgcaatcacgaatgaataacggtttggttggtgcgagtgattttgatgacgagcgtaatggctggcctgttgaacaagtctggaaagaaatgcataagcttttgccattctcaccggattcagtcgtcactcatggtgatttctcacttgataaccttatttttgacgaggggaaattaataggttgtattgatgttggacgagtcggaatcgcagaccgataccaggatcttgccatcctatggaactgcctcggtgagttttctccttcattacagaaacggctttttcaaaaatatggtattgataatcctgatatgaataaattgcagtttcacttgatgctcgatgagtttttctaatgagggcccaaatgtaatcacctggctcaccttcgggtgggcctttctgcgttgctggcgtttttccataggctccgcccccctgacgagcatcacaaaaatcgatgctcaagtcagaggtggcgaaacccgacaggactataaagataccaggcgtttccccctggaagctccctcgtgcgctctcctgttccgaccctgccgcttaccggatacctgtccgcctttctcccttcgggaagcgtggcgctttctcatagctcacgctgtaggtatctcagttcggtgtaggtcgttcgctccaagctgggctgtgtgcacgaaccccccgttcagcccgaccgctgcgccttatccggtaactatcgtcttgagtccaacccggtaagacacgacttatcgccactggcagcagccactggtaacaggattagcagagcgaggtatgtaggcggtgctacagagttcttgaagtggtggcctaactacggctacactagaagaacagtatttggtatctgcgctctgctgaagccagttacctcggaaaaagagttggtagctcttgatccggcaaacaaaccaccgctggtagcggtggtttttttgtttgcaagcagcagattacgcgcagaaaaaaaggatctcaagaagatcctttgattttctaccgaagaaaggcccacccgtgaaggtgagccagtgagttgattgcagtccagttacgctggagtctgaggctcgtcctgaatgatatcaagcttgaattcgtt

SEQ ID NO: 33 - DNA, 6275 bp, Artificial Sequence
  Plasmid pSMART-Mev1
tgcccaggcatcaaataaaacgaaaggctcagtcgaaagactgggcctttcgttttatctgttgtttgtcggtgaacgctctctactagagtcacactggctcaccttcgggtgggcctttctgcgtttatacacagctaacaccacgtcgtccctatctgctgccctaggtctatgagtggttgctggataacgtgcgtaattgtgctgatctcttatatagctgctctcattatctctctaccctgaagtgactctctcacctgtaaaaataatatctcacaggcttaatagtttcttaatacaaagcctgtaaaacgtcaggataacttctatattcagggagaccacaacggtttccctctacaaataattttgtttaactttcgtggaaaaaggagatataccatgaagacggtagttattatcgacgcactgcgtacccccattggaaaatacaaaggaagtctgagccaggtaagcgccgtcgacctgggcacacatgtgaccacgcagttgttgaagcgtcacagcactatcagcgaggaaattgatcaggtcatttttggtaatgttctgcaggcgggcaatgggcagaaccctgcacgtcagattgcaatcaactcaggtttaagccatgaaattccagcgatgacggtcaatgaggtctgtggcagtgggatgaaagcggtaatcctggccaaacagttaatccagctgggtgaggcggaggtacttatcgcaggtggtattgaaaacatgtcacaggccccgaaactgcaacgctttaactacgaaacagaaagctacgatgcgcctttttcgtccatgatgtatgatggtcttaccgacgcattcagtggtcaggcgatgggtctgacggccgagaatgttgctgaaaaataccacgttacccgtgaggaacaagaccaattctctgtccatagccaactcaaagcggcacaggctcaggcagaaggcatttttgccgatgagattgcaccactggaagtttccggcaccctggtggaaaaggacgagggcattcgtccgaatagcagtgttgaaaaactcggtactttgaaaaccgtattcaaagaggacggcacggtgactgccggtaatgcctcaactatcaacgacggtgcctcggcactgattattgcgtctcaagaatacgcggaagcgcacggcttgccgtatctcgcgattatccgcgattcagtggaggtcggcatcgatcccgcgtacatgggcatttcgccgatcaaagcaattcagaagcttctggcacgcaaccagttgacgaccgaagagattgatttatacgaaatcaatgaagcgttcgcggcgacctcgattgtggttcagcgtgaacttgccctcccggaagaaaaggtcaacatctatggcggaggcatcagtttgggccatgccatcggagcgaccggtgcccgtctgctcaccagcttatcatatcagttgaaccagaaagaaaaaaagtacggcgttgcatctctgtgtattggcggaggtctgggcctcgccatgttgttagaacgtccgcagcaaaaaaaaaactcccgcttttatcagatgtcgccggaggaacgtctggcgagcttgttgaacgaagggcagatctctgccgacactaaaaaggaattcgaaaacacggcactgagcagtcagattgcgaaccatatgattgaaaatcagatcagcgagaccgaggtgcccatgggcgtgggccttcatctcacggtggacgaaacggattatctggtaccaatggccacagaagaaccgtcggtaatcgccgcgttgtcaaatggcgcgaaaatcgcgcaagggttcaaaacggtcaaccagcagcgtctcatgcgcggccagatcgtgttctatgatgtagcagatgcagagagtctgattgacgagttacaggttcgtgagacggagatttttcagcaagccgagctgtcgtacccgagcattgttaaacgtggcggtggccttcgtgacttgcagtatcgcgccttcgacgaatcgttcgtgagtgtcgactttctggtagacgtgaaggacgccatgggggccaatatcgttaatgccatgctggaaggggttgcagagctgtttcgtgagtggttcgccgaacaaaaaatcctgtttagcatcttaagcaattacgcaacggaaagcgtcgtgaccatgaaaaccgcgatccctgttagccgcctttcaaagggcagtaacggtcgtgaaatcgctgaaaaaattgttctcgcgtcccgctatgcatcgttggatccttatcgcgcggtgacacacaacaaaggcattatgaatggtatcgaagcggtcgttctggcgaccggcaacgatactcgcgccgtgagcgcgtcctgccatgcttttgctgtgaaagagggccgttatcagggcttgacgtcctggaccctggacggtgaacagctgatcggcgaaatctcggtgcccctcgccctggccactgtgggcggcgccacaaaagtgttgccaaaaagccaagcggcggcggatctgctggccgtaactgatgctaaggaactgagtcgcgtggttgccgcagtgggcctggcccaaaacctggcagcactgcgcgcgctggtttctgaaggcatccagaaaggtcatatggccctgcaagcgcgctctctggccatgaccgtaggggcgaccggcaaggaagtcgaagcggtagctcaacagttaaaacgccagaaaactatgaatcaggatcgtgcgctggccatcctcaatgacctgcgcaaacagtaatagtcgcgccgaaaaccccgcttcggcggggttttgccgcacgtctccatcgcttgcccaagttgtgaagcacagctaacaccacgtcgtccctatctgctgccctaggtctatgagtggttgctggataaccatccataaattttgcataattaatgtaaagaccaggctcgccagtaacgctaaattcatttggctgtaagcgcggtgtcatccgcgtcaggaaaattaaacagttactttaaaaaatgaaaacgtaaaaaggttgggtttcgatgtattgacgggtaaactttgtcgcccgctaaacatttgtttatattcagggagaccacaacggtttccctctacaaataattttgtttaactttgctggaaaaaggagatataccatgaccattgggattgataaaatctcgtttttcgtgcctccttattatatcgacatgacggccctggccgaggctcgcaatgtggatcccggcaaatttcacatcggtatcggccaggaccaaatggcggtgaatcccatctcgcaggacattgtcaccttcgccgcaaacgcagcagaagctatcttgactaaagaagataaagaggccatcgacatggtgatcgtgggtacggaaagctctattgacgaaagtaaagccgcggcggtggtattacaccgcctgatgggtatccagccgtttgcgcgctcctttgaaatcaaagaggcctgctacggcgcaacggctggactgcaactcgcgaagaaccatgttgcattacatccggataaaaaagtcctggttgtcgcggcggacatcgcgaaatacggcctgaactccggcggggaaccaacgcagggtgccggcgcagtggcgatgcttgtcgcaagcgagcctcgtatcctggctttaaaggaggacaacgtgatgctgacacaggatatttacgatttttggcgtcccaccggtcatccatatccgatggttgatggtcctctgtccaatgaaacttatattcagagcttcgcgcaagtttgggatgaacataagaaacgtaccggtctggattttgcggattacgacgctctggcttttcacattccatacacgaaaatgggcaaaaaagccctcttagctaaaatctcagaccagaccgaggcagaacaggaacgcattttagcgcgttacgaagagtcaattatctacagccgccgtgtaggtaatttatatacggggtcgctttatctgggattgatttccttactcgaaaacgccacaaccctgacggcgggtaaccaaatcggtttattctcttacggtagcggtgccgttgccgaattcttcacgggtgagctggttgccggttaccagaaccacttacagaaagaaacccacctcgccctgctggacaaccgtactgaactcagcatcgcagaatatgaggccatgttcgccgaaacactcgacacggatatcgatcaaaccttagaggatgaactcaaatattccatttcagcgattaataacaccgtccgctcctatcgcaattagtaagatcgtcccggcttatcggtcagtttcacctgatttacgtaaaaacccgcttcggcgggtttttgcttttggaggggcagaaagatgaatgactgtccacgacgctatacccaaaagaaagacgaattctctagatatcgctcaatactgaccatttaaatcatacctgacctccatagcagaaagtcaaaagcctccgaccggaggcttttgacttgatcggcacgtaagaggttccaactttcaccataatgaaataagatcactaccgggcgtattttttgagttatcgagattttcaggagctaaggaagctaaaatgagccatattcaacgggaaacgtcttgctcgaggccgcgattaaattccaacatggatgctgatttatatgggtataaatgggctcgcgataatgtcgggcaatcaggtgcgacaatctatcgattgtatgggaagcccgatgcgccagagttgtttctgaaacatggcaaaggtagcgttgccaatgatgttacagatgagatggtcaggctaaactggctgacggaatttatgcctcttccgaccatcaagcattttatccgtactcctgatgatgcatggttactcaccactgcgatcccagggaaaacagcattccaggtattagaagaatatcctgattcaggtgaaaatattgttgatgcgctggcagtgttcctgcgccggttgcattcgattcctgtttgtaattgtccttttaacggcgatcgcgtatttcgtctcgctcaggcgcaatcacgaatgaataacggtttggttggtgcgagtgattttgatgacgagcgtaatggctggcctgttgaacaagtctggaaagaaatgcataagcttttgccattctcaccggattcagtcgtcactcatggtgatttctcacttgataaccttatttttgacgaggggaaattaataggttgtattgatgttggacgagtcggaatcgcagaccgataccaggatcttgccatcctatggaactgcctcggtgagttttctccttcattacagaaacggctttttcaaaaatatggtattgataatcctgatatgaataaattgcagtttcacttgatgctcgatgagtttttctaatgagggcccaaatgtaatcacctggctcaccttcgggtgggcctttctgcgttgctggcgtttttccataggctccgcccccctgacgagcatcacaaaaatcgatgctcaagtcagaggtggcgaaacccgacaggactataaagataccaggcgtttccccctggaagctccctcgtgcgctctcctgttccgaccctgccgcttaccggatacctgtccgcctttctcccttcgggaagcgtggcgctttctcatagctcacgctgtaggtatctcagttcggtgtaggtcgttcgctccaagctgggctgtgtgcacgaaccccccgttcagcccgaccgctgcgccttatccggtaactatcgtcttgagtccaacccggtaagacacgacttatcgccactggcagcagccactggtaacaggattagcagagcgaggtatgtaggcggtgctacagagttcttgaagtggtggcctaactacggctacactagaagaacagtatttggtatctgcgctctgctgaagccagttacctcggaaaaagagttggtagctcttgatccggcaaacaaaccaccgctggtagcggtggtttttttgtttgcaagcagcagattacgcgcagaaaaaaaggatctcaagaagatcctttgattttctaccgaagaaaggcccacccgtgaaggtgagccagtgagttgattgcagtccagttacgctggagtctgaggctcgtcctgaatgatatcaagcttgaattcgtt

SEQ ID NO: 34 - DNA, 5364 bp, Artificial Sequence
  Plasmid pSMART-2,3-BDO1
gtgcgtaattgtgctgatctcttatatagctgctctcattatctctctaccctgaagtgactctctcacctgtaaaaataatatctcacaggcttaatagtttcttaatacaaagcctgtaaaacgtcaggataacttcttggaaaaaggagatataccatgatgcacagcagcgcatgtgattgtgaagcgagtttgtgcgagacactccgtggtttttccgcaaaacacccggattccgtaatctaccagacatcactgatgtccgcccttctgtcaggcgtatatgaaggggacacgactattgcggatcttctggcccacggcgattttggcctgggtacgttcaatgaactcgacggcgaaatgatcgcgttttcttcgcaagtttatcagctccgtgcggatgggagcgcccgcgccgcgaagccagaacaaaaaacaccgtttgcagtaatgacatggttccaaccgcagtatcgtaaaactttcgatgccccggtgagtcgtcagcagatccacgatgtaatcgatcaacagattccttcagacaacctgttttgcgcgctgcgtattgacgggaatttccgtcatgctcacacacgtaccgttccgcgccagaccccaccctatcgcgcgatgaccgatgtgctggatgatcaaccggtctttcgttttaaccagcgcgaaggagttctggtgggttttcgtaccccgcaacatatgcagggtattaacgtggcgggctaccatgagcatttcattacagatgatcgccaaggcggtggtcacctgttggattaccagctggaatctggcgtcctgactttcggcgagattcacaaactgatgattgacctgccggcggattctgcattcctgcaggcaaatttgcaccccagcaaccttgatgccgccatccgctccgtcgagaactaataggctcttcacttctggaaaaaggagatataccatgaattccgaaaaacaatcgcgtcagtgggcacatggtgctgatatggttgtgggccagctggaggcgcagggggttaaacaggtctttggtattccgggtgctaagatcgacaaagtgtttgattctttactggatagctcaatcgagattatcccggtgcgtcatgaagcaaacgcagcgttcatggccgcggcagttggtcgccttacgggtaaagctggcgtagccctggtcacaagcggccccgggtgctcgaatctcattaccggcattgcaaccgcaaattctgagggagatcctgtagtggcactggggggcgcggtaaaacgtgctgataaagcgaaattagttcaccagagtatggacaccgtcgcgatgttctctccagtaaccaaatatgcggttgaagtttcttccccagatgcaattgcagaggtagtatcaaacgcttttcgtgccgcggaacatggccgcccaggtggggcgttcgtttcgctgccgcaggatattgtagaccaaccggcgacaggcgccatcctgcctgcatctggcccggcactgatgggcccagcgccagagtcggcgattaacgatgtggcaaaacttatcgacaacgccaaaaaccctgtgattctgttgggcttaatggcatcacagccggctaattcggctgcattgcgtaagctgctggagaagagtcgcatcccggtgacttccacctaccaagccgccggagctgtgaaccaagaacatttcacccgcttcgccggtcgtgttggccttttcaataaccaagcgggagaccgtctgctgcatttggccgatctcattatctgtattggatactctccagtcgagtatgaaccgagcatgtggaactcgggtgacgcaaccctcgttcatattgacgtgctgccagcttatgaagaacgcaactatgtacccgatatcgagttggtaggcgacattgcggcgacactgaacctgctcgcttcccgcattgatcataaactggagctctcgcagcgtgcctccgagatcttagtcgatcgccaacaccagcgcgatctgctggatcgccgtggcgcaagcttaaatcaatttgcgctgcatccattacgtatcgtccgtgccatgcaggacatcgtaaacaatgacgtaacgctgaccgtggacatgggctcatttcatatttggatcgcacgctatctctattcatttcgcgcacgtcaggtcatgattagtaatgggcaacaaactatgggcgtggctctgccttgggctatcggtgcgtggctggtgaaccccggccgcaaagtggtgagcgttagcggtgacggaggatttctgcagagtagcatggagttagaaaccgctgtccgcctgaacgctaatgtgttacacatcatttgggtggataatggttataatatggttgcaatccaggaggagaaaaagtatcagcgtttaagcggtgtggcgtttggaccggtagatttcaaagcctacgccgatgcattcggcgcccgtggcttcgcggtcgaaagcgcggatgccttagagagcaccttacgtgcggcaatggatgtgaatggtccggccgtcgtggcgattccggtggattattcggataatccgctgctgatgggacaactgcacctttcgcagatcctgtagtaagctcttctggaaaaaggagatataccatgcagaaggtggcgctcgttaccggatctggccaaggcattggcaaagcgattgcgcttcgtctggtcaaagacggattcgccgttgcaattgctgattacaacgacgaaacggcgcgtgctgtcgccgatgaaatcatccgtaatggtggcaacgctgtcgcagtgaaagtggacgtctctgatcgcgaccaagtatttgcagcggtcgagaaagcacgtaccgctctgggcggtttcaacgttatcgtgaacaacgcgggcattgcgccgtcgacgcctatcgaaagcatcaccccggagattgtagataaggtgtacaacatcaacgtaaaaggagtaatctggggtatgcaagctgccatcgatgcgttccgcaaagaggggcacggcggtaaaatcattaacgcgtgttcgcaggctggtcatactggtaacccggaactggcggtttatagcagcagcaaattcgccgtgcgtggcctgacccagaccgctgcacgcgatctggcgccgctggggatcaccgtcaatgcatattgtccgggtatcgtaaaaaccccgatgtgggcggaaattgatcgccaggtatcagaggccgctggcaaaccgctgggctatggcacggaaacgtttgccaagcgcatcacgttaggccgtctgtcggaaccggaggatgttgcagcatgcgtctcttacctggcgggcccggattctgattatatgacgggtcagtccctgctgattgatggtggcatggtctttaactagtaagatcgtcccggcttatcggtcagtttcacctgatttacgtaaaaacccgcttcggcgggtttttgcttttggaggggcagaaagatgaatgactgtccacgacgctatacccaaaagaaagacgaattctctagatatcgctcaatactgaccatttaaatcatacctgacctccatagcagaaagtcaaaagcctccgaccggaggcttttgacttgatcggcacgtaagaggttccaactttcaccataatgaaataagatcactaccgggcgtattttttgagttatcgagattttcaggagctaaggaagctaaaatgagccatattcaacgggaaacgtcttgctcgaggccgcgattaaattccaacatggatgctgatttatatgggtataaatgggctcgcgataatgtcgggcaatcaggtgcgacaatctatcgattgtatgggaagcccgatgcgccagagttgtttctgaaacatggcaaaggtagcgttgccaatgatgttacagatgagatggtcaggctaaactggctgacggaatttatgcctcttccgaccatcaagcattttatccgtactcctgatgatgcatggttactcaccactgcgatcccagggaaaacagcattccaggtattagaagaatatcctgattcaggtgaaaatattgttgatgcgctggcagtgttcctgcgccggttgcattcgattcctgtttgtaattgtccttttaacggcgatcgcgtatttcgtctcgctcaggcgcaatcacgaatgaataacggtttggttggtgcgagtgattttgatgacgagcgtaatggctggcctgttgaacaagtctggaaagaaatgcataagcttttgccattctcaccggattcagtcgtcactcatggtgatttctcacttgataaccttatttttgacgaggggaaattaataggttgtattgatgttggacgagtcggaatcgcagaccgataccaggatcttgccatcctatggaactgcctcggtgagttttctccttcattacagaaacggctttttcaaaaatatggtattgataatcctgatatgaataaattgcagtttcacttgatgctcgatgagtttttctaatgagggcccaaatgtaatcacctggctcaccttcgggtgggcctttctgcgttgctggcgtttttccataggctccgcccccctgacgagcatcacaaaaatcgatgctcaagtcagaggtggcgaaacccgacaggactataaagataccaggcgtttccccctggaagctccctcgtgcgctctcctgttccgaccctgccgcttaccggatacctgtccgcctttctcccttcgggaagcgtggcgctttctcatagctcacgctgtaggtatctcagttcggtgtaggtcgttcgctccaagctgggctgtgtgcacgaaccccccgttcagcccgaccgctgcgccttatccggtaactatcgtcttgagtccaacccggtaagacacgacttatcgccactggcagcagccactggtaacaggattagcagagcgaggtatgtaggcggtgctacagagttcttgaagtggtggcctaactacggctacactagaagaacagtatttggtatctgcgctctgctgaagccagttacctcggaaaaagagttggtagctcttgatccggcaaacaaaccaccgctggtagcggtggtttttttgtttgcaagcagcagattacgcgcagaaaaaaaggatctcaagaagatcctttgattttctaccgaagaaaggcccacccgtgaaggtgagccagtgagttgattgcagtccagttacgctggagtctgaggctcgtcctgaatgatatcaagcttgaattcgtt

SEQ ID NO: 35 - DNA, 5748 bp, Artificial Sequence
  Plasmid pSMART-2,3-BDO2
gtgcgtaattgtgctgatctcttatatagctgctctcattatctctctaccctgaagtgactctctcacctgtaaaaataatatctcacaggcttaatagtttcttaatacaaagcctgtaaaacgtcaggataacttcttggaaaaaggagatataccatgatgcacagcagcgcatgtgattgtgaagcgagtttgtgcgagacactccgtggtttttccgcaaaacacccggattccgtaatctaccagacatcactgatgtccgcccttctgtcaggcgtatatgaaggggacacgactattgcggatcttctggcccacggcgattttggcctgggtacgttcaatgaactcgacggcgaaatgatcgcgttttcttcgcaagtttatcagctccgtgcggatgggagcgcccgcgccgcgaagccagaacaaaaaacaccgtttgcagtaatgacatggttccaaccgcagtatcgtaaaactttcgatgccccggtgagtcgtcagcagatccacgatgtaatcgatcaacagattccttcagacaacctgttttgcgcgctgcgtattgacgggaatttccgtcatgctcacacacgtaccgttccgcgccagaccccaccctatcgcgcgatgaccgatgtgctggatgatcaaccggtctttcgttttaaccagcgcgaaggagttctggtgggttttcgtaccccgcaacatatgcagggtattaacgtggcgggctaccatgagcatttcattacagatgatcgccaaggcggtggtcacctgttggattaccagctggaatctggcgtcctgactttcggcgagattcacaaactgatgattgacctgccggcggattctgcattcctgcaggcaaatttgcaccccagcaaccttgatgccgccatccgctccgtcgagaactaataggctcttcacttctggaaaaaggagatataccatgaattccgaaaaacaatcgcgtcagtgggcacatggtgctgatatggttgtgggccagctggaggcgcagggggttaaacaggtctttggtattccgggtgctaagatcgacaaagtgtttgattctttactggatagctcaatcgagattatcccggtgcgtcatgaagcaaacgcagcgttcatggccgcggcagttggtcgccttacgggtaaagctggcgtagccctggtcacaagcggccccgggtgctcgaatctcattaccggcattgcaaccgcaaattctgagggagatcctgtagtggcactggggggcgcggtaaaacgtgctgataaagcgaaattagttcaccagagtatggacaccgtcgcgatgttctctccagtaaccaaatatgcggttgaagtttcttccccagatgcaattgcagaggtagtatcaaacgcttttcgtgccgcggaacatggccgcccaggtggggcgttcgtttcgctgccgcaggatattgtagaccaaccggcgacaggcgccatcctgcctgcatctggcccggcactgatgggcccagcgccagagtcggcgattaacgatgtggcaaaacttatcgacaacgccaaaaaccctgtgattctgttgggcttaatggcatcacagccggctaattcggctgcattgcgtaagctgctggagaagagtcgcatcccggtgacttccacctaccaagccgccggagctgtgaaccaagaacatttcacccgcttcgccggtcgtgttggccttttcaataaccaagcgggagaccgtctgctgcatttggccgatctcattatctgtattggatactctccagtcgagtatgaaccgagcatgtggaactcgggtgacgcaaccctcgttcatattgacgtgctgccagcttatgaagaacgcaactatgtacccgatatcgagttggtaggcgacattgcggcgacactgaacctgctcgcttcccgcattgatcataaactggagctctcgcagcgtgcctccgagatcttagtcgatcgccaacaccagcgcgatctgctggatcgccgtggcgcaagcttaaatcaatttgcgctgcatccattacgtatcgtccgtgccatgcaggacatcgtaaacaatgacgtaacgctgaccgtggacatgggctcatttcatatttggatcgcacgctatctctattcatttcgcgcacgtcaggtcatgattagtaatgggcaacaaactatgggcgtggctctgccttgggctatcggtgcgtggctggtgaaccccggccgcaaagtggtgagcgttagcggtgacggaggatttctgcagagtagcatggagttagaaaccgctgtccgcctgaacgctaatgtgttacacatcatttgggtggataatggttataatatggttgcaatccaggaggagaaaaagtatcagcgtttaagcggtgtggcgtttggaccggtagatttcaaagcctacgccgatgcattcggcgcccgtggcttcgcggtcgaaagcgcggatgccttagagagcaccttacgtgcggcaatggatgtgaatggtccggccgtcgtggcgattccggtggattattcggataatccgctgctgatgggacaactgcacctttcgcagatcctgtagtaagctcttctggaaaaaggagatataccatgcgtgcgttggcatatttcaaaaaaggagacatccactttaccaacgatattccgcgtccggagatccagacggatgatgaagtgattattgatgtgagctggtgtgggatttgcggttcggatttgcatgaatatctggatggtccaatttttatgccgaaggatggcgaatgtcacaaactgagtaacgcggcgctgcccctggcaatgggacacgagatgtcgggaattgtcagtaaagtcggcccgaaagtgaccaaggtcaaagtgggcgatcatgttgttgttgatgctgcatcgtcctgtgccgatctccattgctggccccacagcaaattctataactctaaaccttgtgacgcgtgtcaacgcggatcggagaacctgtgcacgcatgccggttttgtcgggcttggggttatctctggcggttttgcggaacaagtggtggtatctcaacatcacattattcccgtgccgaaggaaatccctctggacgtagcagcactggtggaaccgctctcggtaacctggcacgcagtaaaaatttcgggctttaagaaaggctcgagtgcactggtgttgggggccggcccaatcggtctgtgtacgattctggtgctgaaaggtatgggtgcgagcaaaatcgtagttagttcgcgttccgagcgtcgcatcgaaatggcaaaaaaactcggcgtcgaagtgtttaatccatcgaaacacggccataagagtattgaaattctgcgtggtctgaccaaatcacatgacggtttcgattatagctatgactgcagtggaattcaggttaccttcgaaaccagccttaaagcccttacttttaaaggcaccgccaccaatatcgctgtttggggtcccaaacccgtacctttccagcctatggatgtgacacttcaggaaaaagttatgacgggatccatcggctacgtggtggaggacttcgaagaagtggtccgtgccattcacaacggagatatcgcgatggaagattgtaagcagctgattaccggcaaacagcgcattgaggatgggtgggaaaaaggcttccaggaattaatggaccacaaagagtctaatgtaaaaattctgctgaccccgaataatcatggagaaatgaaatagtaatagtaagatcgtcccggcttatcggtcagtttcacctgatttacgtaaaaacccgcttcggcgggtttttgcttttggaggggcagaaagatgaatgactgtccacgacgctatacccaaaagaaagacgaattctctagatatcgctcaatactgaccatttaaatcatacctgacctccatagcagaaagtcaaaagcctccgaccggaggcttttgacttgatcggcacgtaagaggttccaactttcaccataatgaaataagatcactaccgggcgtattttttgagttatcgagattttcaggagctaaggaagctaaaatgagccatattcaacgggaaacgtcttgctcgaggccgcgattaaattccaacatggatgctgatttatatgggtataaatgggctcgcgataatgtcgggcaatcaggtgcgacaatctatcgattgtatgggaagcccgatgcgccagagttgtttctgaaacatggcaaaggtagcgttgccaatgatgttacagatgagatggtcaggctaaactggctgacggaatttatgcctcttccgaccatcaagcattttatccgtactcctgatgatgcatggttactcaccactgcgatcccagggaaaacagcattccaggtattagaagaatatcctgattcaggtgaaaatattgttgatgcgctggcagtgttcctgcgccggttgcattcgattcctgtttgtaattgtccttttaacggcgatcgcgtatttcgtctcgctcaggcgcaatcacgaatgaataacggtttggttggtgcgagtgattttgatgacgagcgtaatggctggcctgttgaacaagtctggaaagaaatgcataagcttttgccattctcaccggattcagtcgtcactcatggtgatttctcacttgataaccttatttttgacgaggggaaattaataggttgtattgatgttggacgagtcggaatcgcagaccgataccaggatcttgccatcctatggaactgcctcggtgagttttctccttcattacagaaacggctttttcaaaaatatggtattgataatcctgatatgaataaattgcagtttcacttgatgctcgatgagtttttctaatgagggcccaaatgtaatcacctggctcaccttcgggtgggcctttctgcgttgctggcgtttttccataggctccgcccccctgacgagcatcacaaaaatcgatgctcaagtcagaggtggcgaaacccgacaggactataaagataccaggcgtttccccctggaagctccctcgtgcgctctcctgttccgaccctgccgcttaccggatacctgtccgcctttctcccttcgggaagcgtggcgctttctcatagctcacgctgtaggtatctcagttcggtgtaggtcgttcgctccaagctgggctgtgtgcacgaaccccccgttcagcccgaccgctgcgccttatccggtaactatcgtcttgagtccaacccggtaagacacgacttatcgccactggcagcagccactggtaacaggattagcagagcgaggtatgtaggcggtgctacagagttcttgaagtggtggcctaactacggctacactagaagaacagtatttggtatctgcgctctgctgaagccagttacctcggaaaaagagttggtagctcttgatccggcaaacaaaccaccgctggtagcggtggtttttttgtttgcaagcagcagattacgcgcagaaaaaaaggatctcaagaagatcctttgattttctaccgaagaaaggcccacccgtgaaggtgagccagtgagttgattgcagtccagttacgctggagtctgaggctcgtcctgaatgatatcaagcttgaattcgtt

SEQ ID NO: 36 - DNA, 2818 bp, Artificial Sequence
  Plasmid pSMART-amnp-GFPuv
tgaggctcgtcctgaatgatatcaagcttgaattcgttagacagtcaacgcgcttgatagcctggcgaagatcatccgatcttcgccttacacttttgtttcacatttctgtgacatactatcggatgtgcggtaattgtatgtgtaggaggataatctatggctagcaaaggagaagaacttttcacatggctagcaaaggagaagaacttttcactggagttgtcccaattcttgttgaattagatggtgatgttaatgggcacaaattttctgtcagtggagagggtgaaggtgatgctacatacggaaagcttacccttaaatttatttgcactactggaaaactacctgttccatggccaacacttgtcactactttctcttatggtgttcaatgcttttcccgttatccggatcatatgaaacggcatgactttttcaagagtgccatgcccgaaggttatgtacaggaacgcactatatctttcaaagatgacgggaactacaagacgcgtgctgaagtcaagtttgaaggtgatacccttgttaatcgtatcgagttaaaaggtattgattttaaagaagatggaaacattctcggacacaaactcgagtacaactataactcacacaatgtatacatcacggcagacaaacaaaagaatggaatcaaagctaacttcaaaattcgccacaacattgaagatggatccgttcaactagcagaccattatcaacaaaatactccaattggcgatggccctgtccttttaccagacaaccattacctgtcgacacaatctgccctttcgaaagatcccaacgaaaagcgtgaccacatggtccttcttgagtttgtaactgctgctgggattacacatggcatggatgagctctacaaataatgaggatccccggcttatcggtcagtttcacctgatttacgtaaaaacccgcttcggcgggtttttgcttttggaggggcagaaagatgaatgactgtccacgacgctatacccaaaagaaagacgaattctctagatatcgctcaatactgaccatttaaatcatacctgacctccatagcagaaagtcaaaagcctccgaccggaggcttttgacttgatcggcacgtaagaggttccaactttcaccataatgaaataagatcactaccgggcgtattttttgagttatcgagattttcaggagctaaggaagctaaaatgagccatattcaacgggaaacgtcttgctcgaggccgcgattaaattccaacatggatgctgatttatatgggtataaatgggctcgcgataatgtcgggcaatcaggtgcgacaatctatcgattgtatgggaagcccgatgcgccagagttgtttctgaaacatggcaaaggtagcgttgccaatgatgttacagatgagatggtcaggctaaactggctgacggaatttatgcctcttccgaccatcaagcattttatccgtactcctgatgatgcatggttactcaccactgcgatcccagggaaaacagcattccaggtattagaagaatatcctgattcaggtgaaaatattgttgatgcgctggcagtgttcctgcgccggttgcattcgattcctgtttgtaattgtccttttaacggcgatcgcgtatttcgtctcgctcaggcgcaatcacgaatgaataacggtttggttggtgcgagtgattttgatgacgagcgtaatggctggcctgttgaacaagtctggaaagaaatgcataagcttttgccattctcaccggattcagtcgtcactcatggtgatttctcacttgataaccttatttttgacgaggggaaattaataggttgtattgatgttggacgagtcggaatcgcagaccgataccaggatcttgccatcctatggaactgcctcggtgagttttctccttcattacagaaacggctttttcaaaaatatggtattgataatcctgatatgaataaattgcagtttcacttgatgctcgatgagtttttctaatgagggcccaaatgtaatcacctggctcaccttcgggtgggcctttctgcgttgctggcgtttttccataggctccgcccccctgacgagcatcacaaaaatcgatgctcaagtcagaggtggcgaaacccgacaggactataaagataccaggcgtttccccctggaagctccctcgtgcgctctcctgttccgaccctgccgcttaccggatacctgtccgcctttctcccttcgggaagcgtggcgctttctcatagctcacgctgtaggtatctcagttcggtgtaggtcgttcgctccaagctgggctgtgtgcacgaaccccccgttcagcccgaccgctgcgccttatccggtaactatcgtcttgagtccaacccggtaagacacgacttatcgccactggcagcagccactggtaacaggattagcagagcgaggtatgtaggcggtgctacagagttcttgaagtggtggcctaactacggctacactagaagaacagtatttggtatctgcgctctgctgaagccagttacctcggaaaaagagttggtagctcttgatccggcaaacaaaccaccgctggtagcggtggtttttttgtttgcaagcagcagattacgcgcagaaaaaaaggatctcaagaagatcctttgattttctaccgaagaaaggcccacccgtgaaggtgagccagtgagttgattgcagtccagttacgctggagtctgaggctcgtcctgaatgatatcaagcttgaattcgtt

SEQ ID NO: 37 - DNA, 2839 bp, Artificial Sequence
  Plasmid pSMART-phoAp-GFPuv
tgaggctcgtcctgaatgatatcaagcttgaattcgttcgattacgtaaagaagttattgaagcatcctcgtcagtaaaaagttaatcttttcaacagctgtcataaagttgtcacggccgagacttatagtcgctttgtttttattttttaatgtatttgtagtgtaggaggataatctatggctagcaaaggagaagaacttttcacatggctagcaaaggagaagaacttttcactggagttgtcccaattcttgttgaattagatggtgatgttaatgggcacaaattttctgtcagtggagagggtgaaggtgatgctacatacggaaagcttacccttaaatttatttgcactactggaaaactacctgttccatggccaacacttgtcactactttctcttatggtgttcaatgcttttcccgttatccggatcatatgaaacggcatgactttttcaagagtgccatgcccgaaggttatgtacaggaacgcactatatctttcaaagatgacgggaactacaagacgcgtgctgaagtcaagtttgaaggtgatacccttgttaatcgtatcgagttaaaaggtattgattttaaagaagatggaaacattctcggacacaaactcgagtacaactataactcacacaatgtatacatcacggcagacaaacaaaagaatggaatcaaagctaacttcaaaattcgccacaacattgaagatggatccgttcaactagcagaccattatcaacaaaatactccaattggcgatggccctgtccttttaccagacaaccattacctgtcgacacaatctgccctttcgaaagatcccaacgaaaagcgtgaccacatggtccttcttgagtttgtaactgctgctgggattacacatggcatggatgagctctacaaataatgaggatccccggcttatcggtcagtttcacctgatttacgtaaaaacccgcttcggcgggtttttgcttttggaggggcagaaagatgaatgactgtccacgacgctatacccaaaagaaagacgaattctctagatatcgctcaatactgaccatttaaatcatacctgacctccatagcagaaagtcaaaagcctccgaccggaggcttttgacttgatcggcacgtaagaggttccaactttcaccataatgaaataagatcactaccgggcgtattttttgagttatcgagattttcaggagctaaggaagctaaaatgagccatattcaacgggaaacgtcttgctcgaggccgcgattaaattccaacatggatgctgatttatatgggtataaatgggctcgcgataatgtcgggcaatcaggtgcgacaatctatcgattgtatgggaagcccgatgcgccagagttgtttctgaaacatggcaaaggtagcgttgccaatgatgttacagatgagatggtcaggctaaactggctgacggaatttatgcctcttccgaccatcaagcattttatccgtactcctgatgatgcatggttactcaccactgcgatcccagggaaaacagcattccaggtattagaagaatatcctgattcaggtgaaaatattgttgatgcgctggcagtgttcctgcgccggttgcattcgattcctgtttgtaattgtccttttaacggcgatcgcgtatttcgtctcgctcaggcgcaatcacgaatgaataacggtttggttggtgcgagtgattttgatgacgagcgtaatggctggcctgttgaacaagtctggaaagaaatgcataagcttttgccattctcaccggattcagtcgtcactcatggtgatttctcacttgataaccttatttttgacgaggggaaattaataggttgtattgatgttggacgagtcggaatcgcagaccgataccaggatcttgccatcctatggaactgcctcggtgagttttctccttcattacagaaacggctttttcaaaaatatggtattgataatcctgatatgaataaattgcagtttcacttgatgctcgatgagtttttctaatgagggcccaaatgtaatcacctggctcaccttcgggtgggcctttctgcgttgctggcgtttttccataggctccgcccccctgacgagcatcacaaaaatcgatgctcaagtcagaggtggcgaaacccgacaggactataaagataccaggcgtttccccctggaagctccctcgtgcgctctcctgttccgaccctgccgcttaccggatacctgtccgcctttctcccttcgggaagcgtggcgctttctcatagctcacgctgtaggtatctcagttcggtgtaggtcgttcgctccaagctgggctgtgtgcacgaaccccccgttcagcccgaccgctgcgccttatccggtaactatcgtcttgagtccaacccggtaagacacgacttatcgccactggcagcagccactggtaacaggattagcagagcgaggtatgtaggcggtgctacagagttcttgaagtggtggcctaactacggctacactagaagaacagtatttggtatctgcgctctgctgaagccagttacctcggaaaaagagttggtagctcttgatccggcaaacaaaccaccgctggtagcggtggtttttttgtttgcaagcagcagattacgcgcagaaaaaaaggatctcaagaagatcctttgattttctaccgaagaaaggcccacccgtgaaggtgagccagtgagttgattgcagtccagttacgctggagtctgaggctcgtcctgaatgatatcaagcttgaattcgtt

SEQ ID NO: 38 - DNA, 2819 bp, Artificial Sequence
  Plasmid pSMART-phoBp-GFPuv
tgaggctcgtcctgaatgatatcaagcttgaattcgttgccacggaaatcaataacctgaagatatgtgcgacgagcttttcataaatctgtcataaatctgacgcataatgacgtcgcattaatgatcgcaacctatttattgtgtaggaggataatctatggctagcaaaggagaagaacttttcacatggctagcaaaggagaagaacttttcactggagttgtcccaattcttgttgaattagatggtgatgttaatgggcacaaattttctgtcagtggagagggtgaaggtgatgctacatacggaaagcttacccttaaatttatttgcactactggaaaactacctgttccatggccaacacttgtcactactttctcttatggtgttcaatgcttttcccgttatccggatcatatgaaacggcatgactttttcaagagtgccatgcccgaaggttatgtacaggaacgcactatatctttcaaagatgacgggaactacaagacgcgtgctgaagtcaagtttgaaggtgatacccttgttaatcgtatcgagttaaaaggtattgattttaaagaagatggaaacattctcggacacaaactcgagtacaactataactcacacaatgtatacatcacggcagacaaacaaaagaatggaatcaaagctaacttcaaaattcgccacaacattgaagatggatccgttcaactagcagaccattatcaacaaaatactccaattggcgatggccctgtccttttaccagacaaccattacctgtcgacacaatctgccctttcgaaagatcccaacgaaaagcgtgaccacatggtccttcttgagtttgtaactgctgctgggattacacatggcatggatgagctctacaaataatgaggatccccggcttatcggtcagtttcacctgatttacgtaaaaacccgcttcggcgggtttttgcttttggaggggcagaaagatgaatgactgtccacgacgctatacccaaaagaaagacgaattctctagatatcgctcaatactgaccatttaaatcatacctgacctccatagcagaaagtcaaaagcctccgaccggaggcttttgacttgatcggcacgtaagaggttccaactttcaccataatgaaataagatcactaccgggcgtattttttgagttatcgagattttcaggagctaaggaagctaaaatgagccatattcaacgggaaacgtcttgctcgaggccgcgattaaattccaacatggatgctgatttatatgggtataaatgggctcgcgataatgtcgggcaatcaggtgcgacaatctatcgattgtatgggaagcccgatgcgccagagttgtttctgaaacatggcaaaggtagcgttgccaatgatgttacagatgagatggtcaggctaaactggctgacggaatttatgcctcttccgaccatcaagcattttatccgtactcctgatgatgcatggttactcaccactgcgatcccagggaaaacagcattccaggtattagaagaatatcctgattcaggtgaaaatattgttgatgcgctggcagtgttcctgcgccggttgcattcgattcctgtttgtaattgtccttttaacggcgatcgcgtatttcgtctcgctcaggcgcaatcacgaatgaataacggtttggttggtgcgagtgattttgatgacgagcgtaatggctggcctgttgaacaagtctggaaagaaatgcataagcttttgccattctcaccggattcagtcgtcactcatggtgatttctcacttgataaccttatttttgacgaggggaaattaataggttgtattgatgttggacgagtcggaatcgcagaccgataccaggatcttgccatcctatggaactgcctcggtgagttttctccttcattacagaaacggctttttcaaaaatatggtattgataatcctgatatgaataaattgcagtttcacttgatgctcgatgagtttttctaatgagggcccaaatgtaatcacctggctcaccttcgggtgggcctttctgcgttgctggcgtttttccataggctccgcccccctgacgagcatcacaaaaatcgatgctcaagtcagaggtggcgaaacccgacaggactataaagataccaggcgtttccccctggaagctccctcgtgcgctctcctgttccgaccctgccgcttaccggatacctgtccgcctttctcccttcgggaagcgtggcgctttctcatagctcacgctgtaggtatctcagttcggtgtaggtcgttcgctccaagctgggctgtgtgcacgaaccccccgttcagcccgaccgctgcgccttatccggtaactatcgtcttgagtccaacccggtaagacacgacttatcgccactggcagcagccactggtaacaggattagcagagcgaggtatgtaggcggtgctacagagttcttgaagtggtggcctaactacggctacactagaagaacagtatttggtatctgcgctctgctgaagccagttacctcggaaaaagagttggtagctcttgatccggcaaacaaaccaccgctggtagcggtggtttttttgtttgcaagcagcagattacgcgcagaaaaaaaggatctcaagaagatcctttgattttctaccgaagaaaggcccacccgtgaaggtgagccagtgagttgattgcagtccagttacgctggagtctgaggctcgtcctgaatgatatcaagcttgaattcgtt

SEQ ID NO: 39 - DNA, 2880 bp, Artificial Sequence
  Plasmid pSMART-phoEp-GFPuv
tgaggctcgtcctgaatgatatcaagcttgaattcgttagcatggcgttttgttgcgcgggatcagcaagcctagcggcagttgtttacgcttttattacagatttaataaattaccacattttaagaatattattaatctgtaatatatctttaacaatctcaggttaaaaactttcctgttttcaacgggactctcccgctggtgtaggaggataatctatggctagcaaaggagaagaacttttcacatggctagcaaaggagaagaacttttcactggagttgtcccaattcttgttgaattagatggtgatgttaatgggcacaaattttctgtcagtggagagggtgaaggtgatgctacatacggaaagcttacccttaaatttatttgcactactggaaaactacctgttccatggccaacacttgtcactactttctcttatggtgttcaatgcttttcccgttatccggatcatatgaaacggcatgactttttcaagagtgccatgcccgaaggttatgtacaggaacgcactatatctttcaaagatgacgggaactacaagacgcgtgctgaagtcaagtttgaaggtgatacccttgttaatcgtatcgagttaaaaggtattgattttaaagaagatggaaacattctcggacacaaactcgagtacaactataactcacacaatgtatacatcacggcagacaaacaaaagaatggaatcaaagctaacttcaaaattcgccacaacattgaagatggatccgttcaactagcagaccattatcaacaaaatactccaattggcgatggccctgtccttttaccagacaaccattacctgtcgacacaatctgccctttcgaaagatcccaacgaaaagcgtgaccacatggtccttcttgagtttgtaactgctgctgggattacacatggcatggatgagctctacaaataatgaggatccccggcttatcggtcagtttcacctgatttacgtaaaaacccgcttcggcgggtttttgcttttggaggggcagaaagatgaatgactgtccacgacgctatacccaaaagaaagacgaattctctagatatcgctcaatactgaccatttaaatcatacctgacctccatagcagaaagtcaaaagcctccgaccggaggcttttgacttgatcggcacgtaagaggttccaactttcaccataatgaaataagatcactaccgggcgtattttttgagttatcgagattttcaggagctaaggaagctaaaatgagccatattcaacgggaaacgtcttgctcgaggccgcgattaaattccaacatggatgctgatttatatgggtataaatgggctcgcgataatgtcgggcaatcaggtgcgacaatctatcgattgtatgggaagcccgatgcgccagagttgtttctgaaacatggcaaaggtagcgttgccaatgatgttacagatgagatggtcaggctaaactggctgacggaatttatgcctcttccgaccatcaagcattttatccgtactcctgatgatgcatggttactcaccactgcgatcccagggaaaacagcattccaggtattagaagaatatcctgattcaggtgaaaatattgttgatgcgctggcagtgttcctgcgccggttgcattcgattcctgtttgtaattgtccttttaacggcgatcgcgtatttcgtctcgctcaggcgcaatcacgaatgaataacggtttggttggtgcgagtgattttgatgacgagcgtaatggctggcctgttgaacaagtctggaaagaaatgcataagcttttgccattctcaccggattcagtcgtcactcatggtgatttctcacttgataaccttatttttgacgaggggaaattaataggttgtattgatgttggacgagtcggaatcgcagaccgataccaggatcttgccatcctatggaactgcctcggtgagttttctccttcattacagaaacggctttttcaaaaatatggtattgataatcctgatatgaataaattgcagtttcacttgatgctcgatgagtttttctaatgagggcccaaatgtaatcacctggctcaccttcgggtgggcctttctgcgttgctggcgtttttccataggctccgcccccctgacgagcatcacaaaaatcgatgctcaagtcagaggtggcgaaacccgacaggactataaagataccaggcgtttccccctggaagctccctcgtgcgctctcctgttccgaccctgccgcttaccggatacctgtccgcctttctcccttcgggaagcgtggcgctttctcatagctcacgctgtaggtatctcagttcggtgtaggtcgttcgctccaagctgggctgtgtgcacgaaccccccgttcagcccgaccgctgcgccttatccggtaactatcgtcttgagtccaacccggtaagacacgacttatcgccactggcagcagccactggtaacaggattagcagagcgaggtatgtaggcggtgctacagagttcttgaagtggtggcctaactacggctacactagaagaacagtatttggtatctgcgctctgctgaagccagttacctcggaaaaagagttggtagctcttgatccggcaaacaaaccaccgctggtagcggtggtttttttgtttgcaagcagcagattacgcgcagaaaaaaaggatctcaagaagatcctttgattttctaccgaagaaaggcccacccgtgaaggtgagccagtgagttgattgcagtccagttacgctggagtctgaggctcgtcctgaatgatatcaagcttgaattcgtt

SEQ ID NO: 40 - DNA, 2879 bp, Artificial Sequence
  Plasmid pSMART-phoHp-GFPuv
tgaggctcgtcctgaatgatatcaagcttgaattcgttaatcctgctgaaagcacacagcttttttcatcactgtcatcactctgtcatctttccagtagaaactaatgtcactgaaatggtgttttatagttaaatataagtaaatatattgttgcaataaatgcgagatctgttgtacttattaagtagcagcggaagttcgtgtaggaggataatctatggctagcaaaggagaagaacttttcacatggctagcaaaggagaagaacttttcactggagttgtcccaattcttgttgaattagatggtgatgttaatgggcacaaattttctgtcagtggagagggtgaaggtgatgctacatacggaaagcttacccttaaatttatttgcactactggaaaactacctgttccatggccaacacttgtcactactttctcttatggtgttcaatgcttttcccgttatccggatcatatgaaacggcatgactttttcaagagtgccatgcccgaaggttatgtacaggaacgcactatatctttcaaagatgacgggaactacaagacgcgtgctgaagtcaagtttgaaggtgatacccttgttaatcgtatcgagttaaaaggtattgattttaaagaagatggaaacattctcggacacaaactcgagtacaactataactcacacaatgtatacatcacggcagacaaacaaaagaatggaatcaaagctaacttcaaaattcgccacaacattgaagatggatccgttcaactagcagaccattatcaacaaaatactccaattggcgatggccctgtccttttaccagacaaccattacctgtcgacacaatctgccctttcgaaagatcccaacgaaaagcgtgaccacatggtccttcttgagtttgtaactgctgctgggattacacatggcatggatgagctctacaaataatgaggatccccggcttatcggtcagtttcacctgatttacgtaaaaacccgcttcggcgggtttttgcttttggaggggcagaaagatgaatgactgtccacgacgctatacccaaaagaaagacgaattctctagatatcgctcaatactgaccatttaaatcatacctgacctccatagcagaaagtcaaaagcctccgaccggaggcttttgacttgatcggcacgtaagaggttccaactttcaccataatgaaataagatcactaccgggcgtattttttgagttatcgagattttcaggagctaaggaagctaaaatgagccatattcaacgggaaacgtcttgctcgaggccgcgattaaattccaacatggatgctgatttatatgggtataaatgggctcgcgataatgtcgggcaatcaggtgcgacaatctatcgattgtatgggaagcccgatgcgccagagttgtttctgaaacatggcaaaggtagcgttgccaatgatgttacagatgagatggtcaggctaaactggctgacggaatttatgcctcttccgaccatcaagcattttatccgtactcctgatgatgcatggttactcaccactgcgatcccagggaaaacagcattccaggtattagaagaatatcctgattcaggtgaaaatattgttgatgcgctggcagtgttcctgcgccggttgcattcgattcctgtttgtaattgtccttttaacggcgatcgcgtatttcgtctcgctcaggcgcaatcacgaatgaataacggtttggttggtgcgagtgattttgatgacgagcgtaatggctggcctgttgaacaagtctggaaagaaatgcataagcttttgccattctcaccggattcagtcgtcactcatggtgatttctcacttgataaccttatttttgacgaggggaaattaataggttgtattgatgttggacgagtcggaatcgcagaccgataccaggatcttgccatcctatggaactgcctcggtgagttttctccttcattacagaaacggctttttcaaaaatatggtattgataatcctgatatgaataaattgcagtttcacttgatgctcgatgagtttttctaatgagggcccaaatgtaatcacctggctcaccttcgggtgggcctttctgcgttgctggcgtttttccataggctccgcccccctgacgagcatcacaaaaatcgatgctcaagtcagaggtggcgaaacccgacaggactataaagataccaggcgtttccccctggaagctccctcgtgcgctctcctgttccgaccctgccgcttaccggatacctgtccgcctttctcccttcgggaagcgtggcgctttctcatagctcacgctgtaggtatctcagttcggtgtaggtcgttcgctccaagctgggctgtgtgcacgaaccccccgttcagcccgaccgctgcgccttatccggtaactatcgtcttgagtccaacccggtaagacacgacttatcgccactggcagcagccactggtaacaggattagcagagcgaggtatgtaggcggtgctacagagttcttgaagtggtggcctaactacggctacactagaagaacagtatttggtatctgcgctctgctgaagccagttacctcggaaaaagagttggtagctcttgatccggcaaacaaaccaccgctggtagcggtggtttttttgtttgcaagcagcagattacgcgcagaaaaaaaggatctcaagaagatcctttgattttctaccgaagaaaggcccacccgtgaaggtgagccagtgagttgattgcagtccagttacgctggagtctgaggctcgtcctgaatgatatcaagcttgaattcgtt

SEQ ID NO: 41 - DNA, 2850 bp, Artificial Sequence
  Plasmid pSMART-phoUp-GFPuv
tgaggctcgtcctgaatgatatcaagcttgaattcgttaccgaactgaagcaggattacaccgtggtgatcgtcacccacaacatgcagcaggctgcgcgttgttccgaccacacggcgtttatgtacctgggcgaattgattgagttcagcaacacggacgatctgttcaccagtgtaggaggataatctatggctagcaaaggagaagaacttttcacatggctagcaaaggagaagaacttttcactggagttgtcccaattcttgttgaattagatggtgatgttaatgggcacaaattttctgtcagtggagagggtgaaggtgatgctacatacggaaagcttacccttaaatttatttgcactactggaaaactacctgttccatggccaacacttgtcactactttctcttatggtgttcaatgcttttcccgttatccggatcatatgaaacggcatgactttttcaagagtgccatgcccgaaggttatgtacaggaacgcactatatctttcaaagatgacgggaactacaagacgcgtgctgaagtcaagtttgaaggtgatacccttgttaatcgtatcgagttaaaaggtattgattttaaagaagatggaaacattctcggacacaaactcgagtacaactataactcacacaatgtatacatcacggcagacaaacaaaagaatggaatcaaagctaacttcaaaattcgccacaacattgaagatggatccgttcaactagcagaccattatcaacaaaatactccaattggcgatggccctgtccttttaccagacaaccattacctgtcgacacaatctgccctttcgaaagatcccaacgaaaagcgtgaccacatggtccttcttgagtttgtaactgctgctgggattacacatggcatggatgagctctacaaataatgaggatccccggcttatcggtcagtttcacctgatttacgtaaaaacccgcttcggcgggtttttgcttttggaggggcagaaagatgaatgactgtccacgacgctatacccaaaagaaagacgaattctctagatatcgctcaatactgaccatttaaatcatacctgacctccatagcagaaagtcaaaagcctccgaccggaggcttttgacttgatcggcacgtaagaggttccaactttcaccataatgaaataagatcactaccgggcgtattttttgagttatcgagattttcaggagctaaggaagctaaaatgagccatattcaacgggaaacgtcttgctcgaggccgcgattaaattccaacatggatgctgatttatatgggtataaatgggctcgcgataatgtcgggcaatcaggtgcgacaatctatcgattgtatgggaagcccgatgcgccagagttgtttctgaaacatggcaaaggtagcgttgccaatgatgttacagatgagatggtcaggctaaactggctgacggaatttatgcctcttccgaccatcaagcattttatccgtactcctgatgatgcatggttactcaccactgcgatcccagggaaaacagcattccaggtattagaagaatatcctgattcaggtgaaaatattgttgatgcgctggcagtgttcctgcgccggttgcattcgattcctgtttgtaattgtccttttaacggcgatcgcgtatttcgtctcgctcaggcgcaatcacgaatgaataacggtttggttggtgcgagtgattttgatgacgagcgtaatggctggcctgttgaacaagtctggaaagaaatgcataagcttttgccattctcaccggattcagtcgtcactcatggtgatttctcacttgataaccttatttttgacgaggggaaattaataggttgtattgatgttggacgagtcggaatcgcagaccgataccaggatcttgccatcctatggaactgcctcggtgagttttctccttcattacagaaacggctttttcaaaaatatggtattgataatcctgatatgaataaattgcagtttcacttgatgctcgatgagtttttctaatgagggcccaaatgtaatcacctggctcaccttcgggtgggcctttctgcgttgctggcgtttttccataggctccgcccccctgacgagcatcacaaaaatcgatgctcaagtcagaggtggcgaaacccgacaggactataaagataccaggcgtttccccctggaagctccctcgtgcgctctcctgttccgaccctgccgcttaccggatacctgtccgcctttctcccttcgggaagcgtggcgctttctcatagctcacgctgtaggtatctcagttcggtgtaggtcgttcgctccaagctgggctgtgtgcacgaaccccccgttcagcccgaccgctgcgccttatccggtaactatcgtcttgagtccaacccggtaagacacgacttatcgccactggcagcagccactggtaacaggattagcagagcgaggtatgtaggcggtgctacagagttcttgaagtggtggcctaactacggctacactagaagaacagtatttggtatctgcgctctgctgaagccagttacctcggaaaaagagttggtagctcttgatccggcaaacaaaccaccgctggtagcggtggtttttttgtttgcaagcagcagattacgcgcagaaaaaaaggatctcaagaagatcctttgattttctaccgaagaaaggcccacccgtgaaggtgagccagtgagttgattgcagtccagttacgctggagtctgaggctcgtcctgaatgatatcaagcttgaattcgtt

SEQ ID NO: 42 - DNA, 2900 bp, Artificial Sequence
  Plasmid pSMART-mipAp-GFPuv
tgaggctcgtcctgaatgatatcaagcttgaattcgttcatccataaattttgcataattaatgtaaagaccaggctcgccagtaacgctaaattcatttggctgtaagcgcggtgtcatccgcgtcaggaaaattaaacagttactttaaaaaatgaaaacgtaaaaaggttgggtttcgatgtattgacgggtaaactttgtcgcccgctaaacatttgtttgtgtaggaggataatctatggctagcaaaggagaagaacttttcacatggctagcaaaggagaagaacttttcactggagttgtcccaattcttgttgaattagatggtgatgttaatgggcacaaattttctgtcagtggagagggtgaaggtgatgctacatacggaaagcttacccttaaatttatttgcactactggaaaactacctgttccatggccaacacttgtcactactttctcttatggtgttcaatgcttttcccgttatccggatcatatgaaacggcatgactttttcaagagtgccatgcccgaaggttatgtacaggaacgcactatatctttcaaagatgacgggaactacaagacgcgtgctgaagtcaagtttgaaggtgatacccttgttaatcgtatcgagttaaaaggtattgattttaaagaagatggaaacattctcggacacaaactcgagtacaactataactcacacaatgtatacatcacggcagacaaacaaaagaatggaatcaaagctaacttcaaaattcgccacaacattgaagatggatccgttcaactagcagaccattatcaacaaaatactccaattggcgatggccctgtccttttaccagacaaccattacctgtcgacacaatctgccctttcgaaagatcccaacgaaaagcgtgaccacatggtccttcttgagtttgtaactgctgctgggattacacatggcatggatgagctctacaaataatgaggatccccggcttatcggtcagtttcacctgatttacgtaaaaacccgcttcggcgggtttttgcttttggaggggcagaaagatgaatgactgtccacgacgctatacccaaaagaaagacgaattctctagatatcgctcaatactgaccatttaaatcatacctgacctccatagcagaaagtcaaaagcctccgaccggaggcttttgacttgatcggcacgtaagaggttccaactttcaccataatgaaataagatcactaccgggcgtattttttgagttatcgagattttcaggagctaaggaagctaaaatgagccatattcaacgggaaacgtcttgctcgaggccgcgattaaattccaacatggatgctgatttatatgggtataaatgggctcgcgataatgtcgggcaatcaggtgcgacaatctatcgattgtatgggaagcccgatgcgccagagttgtttctgaaacatggcaaaggtagcgttgccaatgatgttacagatgagatggtcaggctaaactggctgacggaatttatgcctcttccgaccatcaagcattttatccgtactcctgatgatgcatggttactcaccactgcgatcccagggaaaacagcattccaggtattagaagaatatcctgattcaggtgaaaatattgttgatgcgctggcagtgttcctgcgccggttgcattcgattcctgtttgtaattgtccttttaacggcgatcgcgtatttcgtctcgctcaggcgcaatcacgaatgaataacggtttggttggtgcgagtgattttgatgacgagcgtaatggctggcctgttgaacaagtctggaaagaaatgcataagcttttgccattctcaccggattcagtcgtcactcatggtgatttctcacttgataaccttatttttgacgaggggaaattaataggttgtattgatgttggacgagtcggaatcgcagaccgataccaggatcttgccatcctatggaactgcctcggtgagttttctccttcattacagaaacggctttttcaaaaatatggtattgataatcctgatatgaataaattgcagtttcacttgatgctcgatgagtttttctaatgagggcccaaatgtaatcacctggctcaccttcgggtgggcctttctgcgttgctggcgtttttccataggctccgcccccctgacgagcatcacaaaaatcgatgctcaagtcagaggtggcgaaacccgacaggactataaagataccaggcgtttccccctggaagctccctcgtgcgctctcctgttccgaccctgccgcttaccggatacctgtccgcctttctcccttcgggaagcgtggcgctttctcatagctcacgctgtaggtatctcagttcggtgtaggtcgttcgctccaagctgggctgtgtgcacgaaccccccgttcagcccgaccgctgcgccttatccggtaactatcgtcttgagtccaacccggtaagacacgacttatcgccactggcagcagccactggtaacaggattagcagagcgaggtatgtaggcggtgctacagagttcttgaagtggtggcctaactacggctacactagaagaacagtatttggtatctgcgctctgctgaagccagttacctcggaaaaagagttggtagctcttgatccggcaaacaaaccaccgctggtagcggtggtttttttgtttgcaagcagcagattacgcgcagaaaaaaaggatctcaagaagatcctttgattttctaccgaagaaaggcccacccgtgaaggtgagccagtgagttgattgcagtccagttacgctggagtctgaggctcgtcctgaatgatatcaagcttgaattcgtt

SEQ ID NO: 43 - DNA, 2816 bp, Artificial Sequence
  Plasmid pSMART-pstSp-GFPuv
tgaggctcgtcctgaatgatatcaagcttgaattcgttaagactttatctctctgtcataaaactgtcatattccttacatataactgtcacctgtttgtcctattttgcttctcgtagccaacaaacaatgctttatgagtgtaggaggataatctatggctagcaaaggagaagaacttttcacatggctagcaaaggagaagaacttttcactggagttgtcccaattcttgttgaattagatggtgatgttaatgggcacaaattttctgtcagtggagagggtgaaggtgatgctacatacggaaagcttacccttaaatttatttgcactactggaaaactacctgttccatggccaacacttgtcactactttctcttatggtgttcaatgcttttcccgttatccggatcatatgaaacggcatgactttttcaagagtgccatgcccgaaggttatgtacaggaacgcactatatctttcaaagatgacgggaactacaagacgcgtgctgaagtcaagtttgaaggtgatacccttgttaatcgtatcgagttaaaaggtattgattttaaagaagatggaaacattctcggacacaaactcgagtacaactataactcacacaatgtatacatcacggcagacaaacaaaagaatggaatcaaagctaacttcaaaattcgccacaacattgaagatggatccgttcaactagcagaccattatcaacaaaatactccaattggcgatggccctgtccttttaccagacaaccattacctgtcgacacaatctgccctttcgaaagatcccaacgaaaagcgtgaccacatggtccttcttgagtttgtaactgctgctgggattacacatggcatggatgagctctacaaataatgaggatccccggcttatcggtcagtttcacctgatttacgtaaaaacccgcttcggcgggtttttgcttttggaggggcagaaagatgaatgactgtccacgacgctatacccaaaagaaagacgaattctctagatatcgctcaatactgaccatttaaatcatacctgacctccatagcagaaagtcaaaagcctccgaccggaggcttttgacttgatcggcacgtaagaggttccaactttcaccataatgaaataagatcactaccgggcgtattttttgagttatcgagattttcaggagctaaggaagctaaaatgagccatattcaacgggaaacgtcttgctcgaggccgcgattaaattccaacatggatgctgatttatatgggtataaatgggctcgcgataatgtcgggcaatcaggtgcgacaatctatcgattgtatgggaagcccgatgcgccagagttgtttctgaaacatggcaaaggtagcgttgccaatgatgttacagatgagatggtcaggctaaactggctgacggaatttatgcctcttccgaccatcaagcattttatccgtactcctgatgatgcatggttactcaccactgcgatcccagggaaaacagcattccaggtattagaagaatatcctgattcaggtgaaaatattgttgatgcgctggcagtgttcctgcgccggttgcattcgattcctgtttgtaattgtccttttaacggcgatcgcgtatttcgtctcgctcaggcgcaatcacgaatgaataacggtttggttggtgcgagtgattttgatgacgagcgtaatggctggcctgttgaacaagtctggaaagaaatgcataagcttttgccattctcaccggattcagtcgtcactcatggtgatttctcacttgataaccttatttttgacgaggggaaattaataggttgtattgatgttggacgagtcggaatcgcagaccgataccaggatcttgccatcctatggaactgcctcggtgagttttctccttcattacagaaacggctttttcaaaaatatggtattgataatcctgatatgaataaattgcagtttcacttgatgctcgatgagtttttctaatgagggcccaaatgtaatcacctggctcaccttcgggtgggcctttctgcgttgctggcgtttttccataggctccgcccccctgacgagcatcacaaaaatcgatgctcaagtcagaggtggcgaaacccgacaggactataaagataccaggcgtttccccctggaagctccctcgtgcgctctcctgttccgaccctgccgcttaccggatacctgtccgcctttctcccttcgggaagcgtggcgctttctcatagctcacgctgtaggtatctcagttcggtgtaggtcgttcgctccaagctgggctgtgtgcacgaaccccccgttcagcccgaccgctgcgccttatccggtaactatcgtcttgagtccaacccggtaagacacgacttatcgccactggcagcagccactggtaacaggattagcagagcgaggtatgtaggcggtgctacagagttcttgaagtggtggcctaactacggctacactagaagaacagtatttggtatctgcgctctgctgaagccagttacctcggaaaaagagttggtagctcttgatccggcaaacaaaccaccgctggtagcggtggtttttttgtttgcaagcagcagattacgcgcagaaaaaaaggatctcaagaagatcctttgattttctaccgaagaaaggcccacccgtgaaggtgagccagtgagttgattgcagtccagttacgctggagtctgaggctcgtcctgaatgatatcaagcttgaattcgtt

SEQ ID NO: 44 - DNA, 2808 bp, Artificial Sequence
  Plasmid pSMART-ugpBp-GFPuv
tgaggctcgtcctgaatgatatcaagcttgaattcgtttctttctgacaccttactatcttacaaatgtaacaaaaaagttatttttctgtaattcgagcatgtcatgttaccccgcgagcataaaacgcgtgtgtaggaggataatctatggctagcaaaggagaagaacttttcacatggctagcaaaggagaagaacttttcactggagttgtcccaattcttgttgaattagatggtgatgttaatgggcacaaattttctgtcagtggagagggtgaaggtgatgctacatacggaaagcttacccttaaatttatttgcactactggaaaactacctgttccatggccaacacttgtcactactttctcttatggtgttcaatgcttttcccgttatccggatcatatgaaacggcatgactttttcaagagtgccatgcccgaaggttatgtacaggaacgcactatatctttcaaagatgacgggaactacaagacgcgtgctgaagtcaagtttgaaggtgatacccttgttaatcgtatcgagttaaaaggtattgattttaaagaagatggaaacattctcggacacaaactcgagtacaactataactcacacaatgtatacatcacggcagacaaacaaaagaatggaatcaaagctaacttcaaaattcgccacaacattgaagatggatccgttcaactagcagaccattatcaacaaaatactccaattggcgatggccctgtccttttaccagacaaccattacctgtcgacacaatctgccctttcgaaagatcccaacgaaaagcgtgaccacatggtccttcttgagtttgtaactgctgctgggattacacatggcatggatgagctctacaaataatgaggatccccggcttatcggtcagtttcacctgatttacgtaaaaacccgcttcggcgggtttttgcttttggaggggcagaaagatgaatgactgtccacgacgctatacccaaaagaaagacgaattctctagatatcgctcaatactgaccatttaaatcatacctgacctccatagcagaaagtcaaaagcctccgaccggaggcttttgacttgatcggcacgtaagaggttccaactttcaccataatgaaataagatcactaccgggcgtattttttgagttatcgagattttcaggagctaaggaagctaaaatgagccatattcaacgggaaacgtcttgctcgaggccgcgattaaattccaacatggatgctgatttatatgggtataaatgggctcgcgataatgtcgggcaatcaggtgcgacaatctatcgattgtatgggaagcccgatgcgccagagttgtttctgaaacatggcaaaggtagcgttgccaatgatgttacagatgagatggtcaggctaaactggctgacggaatttatgcctcttccgaccatcaagcattttatccgtactcctgatgatgcatggttactcaccactgcgatcccagggaaaacagcattccaggtattagaagaatatcctgattcaggtgaaaatattgttgatgcgctggcagtgttcctgcgccggttgcattcgattcctgtttgtaattgtccttttaacggcgatcgcgtatttcgtctcgctcaggcgcaatcacgaatgaataacggtttggttggtgcgagtgattttgatgacgagcgtaatggctggcctgttgaacaagtctggaaagaaatgcataagcttttgccattctcaccggattcagtcgtcactcatggtgatttctcacttgataaccttatttttgacgaggggaaattaataggttgtattgatgttggacgagtcggaatcgcagaccgataccaggatcttgccatcctatggaactgcctcggtgagttttctccttcattacagaaacggctttttcaaaaatatggtattgataatcctgatatgaataaattgcagtttcacttgatgctcgatgagtttttctaatgagggcccaaatgtaatcacctggctcaccttcgggtgggcctttctgcgttgctggcgtttttccataggctccgcccccctgacgagcatcacaaaaatcgatgctcaagtcagaggtggcgaaacccgacaggactataaagataccaggcgtttccccctggaagctccctcgtgcgctctcctgttccgaccctgccgcttaccggatacctgtccgcctttctcccttcgggaagcgtggcgctttctcatagctcacgctgtaggtatctcagttcggtgtaggtcgttcgctccaagctgggctgtgtgcacgaaccccccgttcagcccgaccgctgcgccttatccggtaactatcgtcttgagtccaacccggtaagacacgacttatcgccactggcagcagccactggtaacaggattagcagagcgaggtatgtaggcggtgctacagagttcttgaagtggtggcctaactacggctacactagaagaacagtatttggtatctgcgctctgctgaagccagttacctcggaaaaagagttggtagctcttgatccggcaaacaaaccaccgctggtagcggtggtttttttgtttgcaagcagcagattacgcgcagaaaaaaaggatctcaagaagatcctttgattttctaccgaagaaaggcccacccgtgaaggtgagccagtgagttgattgcagtccagttacgctggagtctgaggctcgtcctgaatgatatcaagcttgaattcgtt

SEQ ID NO: 45 - DNA, 2819 bp, Artificial Sequence
  Plasmid pSMART-ydfHp-GFPuv
tgaggctcgtcctgaatgatatcaagcttgaattcgttgctatgccggactgaatgtccaccgtcagtaatttttatacccggcgtaactgccgggttattgcttgtcacaaaaaagtggtagactcatgcagttaactcactgtgtaggaggataatctatggctagcaaaggagaagaacttttcacatggctagcaaaggagaagaacttttcactggagttgtcccaattcttgttgaattagatggtgatgttaatgggcacaaattttctgtcagtggagagggtgaaggtgatgctacatacggaaagcttacccttaaatttatttgcactactggaaaactacctgttccatggccaacacttgtcactactttctcttatggtgttcaatgcttttcccgttatccggatcatatgaaacggcatgactttttcaagagtgccatgcccgaaggttatgtacaggaacgcactatatctttcaaagatgacgggaactacaagacgcgtgctgaagtcaagtttgaaggtgatacccttgttaatcgtatcgagttaaaaggtattgattttaaagaagatggaaacattctcggacacaaactcgagtacaactataactcacacaatgtatacatcacggcagacaaacaaaagaatggaatcaaagctaacttcaaaattcgccacaacattgaagatggatccgttcaactagcagaccattatcaacaaaatactccaattggcgatggccctgtccttttaccagacaaccattacctgtcgacacaatctgccctttcgaaagatcccaacgaaaagcgtgaccacatggtccttcttgagtttgtaactgctgctgggattacacatggcatggatgagctctacaaataatgaggatccccggcttatcggtcagtttcacctgatttacgtaaaaacccgcttcggcgggtttttgcttttggaggggcagaaagatgaatgactgtccacgacgctatacccaaaagaaagacgaattctctagatatcgctcaatactgaccatttaaatcatacctgacctccatagcagaaagtcaaaagcctccgaccggaggcttttgacttgatcggcacgtaagaggttccaactttcaccataatgaaataagatcactaccgggcgtattttttgagttatcgagattttcaggagctaaggaagctaaaatgagccatattcaacgggaaacgtcttgctcgaggccgcgattaaattccaacatggatgctgatttatatgggtataaatgggctcgcgataatgtcgggcaatcaggtgcgacaatctatcgattgtatgggaagcccgatgcgccagagttgtttctgaaacatggcaaaggtagcgttgccaatgatgttacagatgagatggtcaggctaaactggctgacggaatttatgcctcttccgaccatcaagcattttatccgtactcctgatgatgcatggttactcaccactgcgatcccagggaaaacagcattccaggtattagaagaatatcctgattcaggtgaaaatattgttgatgcgctggcagtgttcctgcgccggttgcattcgattcctgtttgtaattgtccttttaacggcgatcgcgtatttcgtctcgctcaggcgcaatcacgaatgaataacggtttggttggtgcgagtgattttgatgacgagcgtaatggctggcctgttgaacaagtctggaaagaaatgcataagcttttgccattctcaccggattcagtcgtcactcatggtgatttctcacttgataaccttatttttgacgaggggaaattaataggttgtattgatgttggacgagtcggaatcgcagaccgataccaggatcttgccatcctatggaactgcctcggtgagttttctccttcattacagaaacggctttttcaaaaatatggtattgataatcctgatatgaataaattgcagtttcacttgatgctcgatgagtttttctaatgagggcccaaatgtaatcacctggctcaccttcgggtgggcctttctgcgttgctggcgtttttccataggctccgcccccctgacgagcatcacaaaaatcgatgctcaagtcagaggtggcgaaacccgacaggactataaagataccaggcgtttccccctggaagctccctcgtgcgctctcctgttccgaccctgccgcttaccggatacctgtccgcctttctcccttcgggaagcgtggcgctttctcatagctcacgctgtaggtatctcagttcggtgtaggtcgttcgctccaagctgggctgtgtgcacgaaccccccgttcagcccgaccgctgcgccttatccggtaactatcgtcttgagtccaacccggtaagacacgacttatcgccactggcagcagccactggtaacaggattagcagagcgaggtatgtaggcggtgctacagagttcttgaagtggtggcctaactacggctacactagaagaacagtatttggtatctgcgctctgctgaagccagttacctcggaaaaagagttggtagctcttgatccggcaaacaaaccaccgctggtagcggtggtttttttgtttgcaagcagcagattacgcgcagaaaaaaaggatctcaagaagatcctttgattttctaccgaagaaaggcccacccgtgaaggtgagccagtgagttgattgcagtccagttacgctggagtctgaggctcgtcctgaatgatatcaagcttgaattcgtt

SEQ ID NO: 46 - DNA, 3424 bp, Artificial Sequence; identical to SEQ ID NO: 32
  Plasmid pSMART-Ala2

SEQ ID NO: 47 - DNA, 21 bp, Artificial Sequence
  fabI T2 targeting sequence
cagcctgctccggtcggaccg

SEQ ID NO: 48 - DNA, 45 bp, Artificial Sequence
  C-terminal DAS+4 tag
gcggccaacgatgaaaactattctgaaaactatgcggatgcgtct

SEQ ID NO: 49 - DNA, 59 bp, Artificial Sequence
  Primer gltA2-FOR
gggacagttattagttcgagttccccgcgccagcggggataaaccgaaaaaaaaacccc

SEQ ID NO: 50 - DNA, 63 bp, Artificial Sequence
  Primer gltA2-REV
gaatgaattggtcaatacggtttatccccgctggcgcggggaactcgaggtggtaccagatct

SEQ ID NO: 51 - DNA, 28 bp, Artificial Sequence
  Primer G2U-FOR1
ccggatgagcattcatcaggcgggcaag

SEQ ID NO: 52 - DNA, 47 bp, Artificial Sequence
  Primer G2U-REV1
cggtttatccccgctggcgcggggaactcgaacttcataacttttac

SEQ ID NO: 53 - DNA, 34 bp, Artificial Sequence
  Primer G2U-FOR2
gcgccagcggggataaaccgttaccattctgttg

SEQ ID NO: 54 - DNA, 28 bp, Artificial Sequence
  Primer G2U-REV2
cttgcccgcctgatgaatgctcatccgg